European Patent Application EP 4 530 354 A2, published April 2, 2025. Title: TREATMENT OF RETINITIS PIGMENTOSA USING ENGINEERED MEGANUCLEASES. Applicant: Precision BioSciences, Inc. Application EP Not Yet Assigned. The sequence listing filed with the application follows.

SEQUENCE LISTING (281 sequences)

SEQ ID NO: 1 - DNA, 22 bp, synthetic construct
  misc_feature 1..22: note = Synthetic Polynucleotide
  source 1..22: mol_type = other DNA
acgggtgtggtacgcagccact

SEQ ID NO: 2 - DNA, 22 bp, synthetic construct
  misc_feature 1..22: note = Synthetic Polynucleotide
  source 1..22: mol_type = other DNA
ccacttcgagtacccacagtac

SEQ ID NO: 3 - DNA, 22 bp, synthetic construct
  misc_feature 1..22: note = Synthetic Polynucleotide
  source 1..22: mol_type = other DNA
gggtgtggtacgcagccacttc

SEQ ID NO: 4 - DNA, 22 bp, synthetic construct
  misc_feature 1..22: note = Synthetic Polynucleotide
  source 1..22: mol_type = other DNA
gcagccacttcgagtacccaca

SEQ ID NO: 5 - DNA, 22 bp, synthetic construct
  misc_feature 1..22: note = Synthetic Polynucleotide
  source 1..22: mol_type = other DNA
acgggtgtggtacgcagcccct

SEQ ID NO: 6 - protein, 354 aa, synthetic construct
  REGION 1..354: note = Synthetic Polypeptide
MNTKYNKEFLLYLAGFVDGDGSIFARIFKGQHWKFKHYIRLTFTVAQKTQRRWFLDKLVDEIGVGYVTDWGSVSHYYLSEIKPLHNFLTQLQPFLKLKQKQANLVLKIIEQLPSAKESPDKFLEVCTWVDQIAALNDSKTRKTTSETVRAVLDSLPGSVGGLSPSQASSAASSASSSPGSGISEALRAGAGSGTGYNKEFLLYLAGFVDGDGSIWASIIPEQGYKFKHRLRLSFTVAQKTQRRWFLDKLVDEIGVGYVVDQGSVSEYRLSEIKPLHNFLTQLQPFLKLKQKQANLVLKIIEQLPSAKESPDKFLEVCTWVDQIAALNDSKTRKTTSETVRAVLDSLSEKKKSSP

SEQ ID NO: 7 - protein, 354 aa, synthetic construct
  REGION 1..354: note = Synthetic Polypeptide
MNTKYNKEFLLYLAGFVDGDGSIYARIFKGQHWKFKHYIRLTFCVRQKTQRRWFLDKLVDEIGVGYVTDSGSVSAYYLSEIKPLHNFLTQLQPFLKLKQKQANLVLKIIEQLPSAKESPDKFLEVCTWVDQIAALNDSKTRKTTSETVRAVLDSLPGSVGGLSPSQASSAASSASSSPGSGISEALRAGAGSGTGYNKEFLLYLAGFVDGDGSIWASIIPEQGYKFKHRLRLSFTVAQKTQRRWFLDKLVDEIGVGYVVDQGSVSEYRLSEIKPLHNFLTQLQPFLKLKQKQANLVLKIIEQLPSAKESPDKFLEVCTWVDQIAALNDSKTRKTTSETVRAVLDSLSEKKKSSP

SEQ ID NO: 8 - protein, 354 aa, synthetic construct
  REGION 1..354: note = Synthetic Polypeptide
MNTKYNKEFLLYLAGFVDGDGSIYARIFKGQHWKFKHHIRLTFHVSQKTQRRWFLDKLVDEIGVGYVTDWGSVSGYYLSEIKPLHNFLTQLQPFLKLKQKQANLVLKIIEQLPSAKESPDKFLEVCTWVDQIAALNDSKTRKTTSETVRAVLDSLPGSVGGLSPSQASSAASSASSSPGSGISEALRAGAGSGTGYNKEFLLYLAGFVDGDGSIWASIIPEQGYKFKHRLRLSFTVAQKTQRRWFLDKLVDEIGVGYVVDQGSVSEYRLSEIKPLHNFLTQLQPFLKLKQKQANLVLKIIEQLPSAKESPDKFLEVCTWVDQIAALNDSKTRKTTSETVRAVLDSLSEKKKSSP

SEQ ID NO: 9 - protein, 354 aa, synthetic construct
  REGION 1..354: note = Synthetic Polypeptide
MNTKYNKEFLLYLAGFVDGDGSIYARIEPRQTAKFKHYLRLTFHVSQKTQRRWFLDKLVDEIGVGYVTDWGSVSGYYLSEIKPLHNFLTQLQPFLKLKQKQANLVLKIIEQLPSAKESPDKFLEVCTWVDQIAALNDSKTRKTTSETVRAVLDSLPGSVGGLSPSQASSAASSASSSPGSGISEALRAGAGSGTGYNKEFLLYLAGFVDGDGSIWASIIPEQGYKFKHRLRLSFTVAQKTQRRWFLDKLVDEIGVGYVVDQGSVSEYRLSEIKPLHNFLTQLQPFLKLKQKQANLVLKIIEQLPSAKESPDKFLEVCTWVDQIAALNDSKTRKTTSETVRAVLDSLSEKKKSSP

SEQ ID NO: 10 - protein, 354 aa, synthetic construct
  REGION 1..354: note = Synthetic Polypeptide
MNTKYNKEFLLYLAGFVDGDGSIYARIEPRQTAKFKHYLRLTFHVSQKTQRRWFLDKLVDEIGVGYVVDQGSVSQYFLSEIKPLHNFLTQLQPFLKLKQKQANLVLKIIEQLPSAKESPDKFLEVCTWVDQIAALNDSKTRKTTSETVRAVLDSLPGSVGGLSPSQASSAASSASSSPGSGISEALRAGAGSGTGYNKEFLLYLAGFVDGDGSIYATIMPEQRQKFKHRLRLYFEVCQKTQRRWFLDKLVDEIGVGYVYDQGSVSTYRLSQIKPLHNFLTQLQPFLKLKQKQANLVLKIIEQLPSAKESPDKFLEVCTWVDQIAALNDSKTRKTTSETVRAVLDSLSEKKKSSP

SEQ ID NO: 11 - protein, 354 aa, synthetic construct
  REGION 1..354: note = Synthetic Polypeptide
MNTKYNKEFLLYLAGFVDGDGSIYARIEPRQNFKFKHTLRLTFFVSQKTQRRWFLDKLVDEIGVGYVTDWGSVSGYYLSQIKPLHNFLTQLQPFLKLKQKQANLVLKIIEQLPSAKESPDKFLEVCTWVDQIAALNDSKTRKTTSETVRAVLDSLPGSVGGLSPSQASSAASSASSSPGSGISEALRAGAGSGTGYNKEFLLYLAGFVDGDGSIYATIIPSQTDKFKHRLRLYFAVSQKTQRRWFLDKLVDEIGVGYVIDSGSVSEYRLSEIKPLHNFLTQLQPFLKLKQKQANLVLKIIEQLPSAKESPDKFLEVCTWVDQIAALNDSKTRKTTSETVRAVLDSLSEKKKSSP

SEQ ID NO: 12 - protein, 354 aa, synthetic construct
  REGION 1..354: note = Synthetic Polypeptide
MNTKYNKEFLLYLAGFVDGDGSIYARIEPRQGNKFKHYLRLTFNVCQKTQRRWFLDKLVDEIGVGYVIDRGSVSDYYLSEIKPLHNFLTQLQPFLKLKQKQANLVLKIIEQLPSAKESPDKFLEVCTWVDQIAALNDSKTRKTTSETVRAVLDSLPGSVGGLSPSQASSAASSASSSPGSGISEALRAGAGSGTGYNKEFLLYLAGFVDGDGSIYASIQPDQVYKFKHRLRLRFAVFQKTQRRWFLDKLVDEIGVGYVYDHGSVSEYRLSQIKPLHNFLTQLQPFLKLKQKQANLVLKIIEQLPSAKESPDKFLEVCTWVDQIAALNDSKTRKTTSETVRAVLDSLSEKKKSSP

SEQ ID NO: 13 - protein, 354 aa, synthetic construct
  REGION 1..354: note = Synthetic Polypeptide
MNTKYNKEFLLYLAGFVDGDGSIYARIEPRQTAKFKHYLRLTFHVSQKTQRRWFLDKLVDEIGVGYVVDQGSVSQYFLSQIKPLHNFLTQLQPFLKLKQKQANLVLKIIEQLPSAKESPDKFLEVCTWVDQIAALNDSKTRKTTSETVRAVLDSLPGSVGGLSPSQASSAASSASSSPGSGISEALRAGAGSGTGYNKEFLLYLAGFVDGDGSIYASIEPVQTYKFKHRLRLSFAVSQKTQRRWFLDKLVDEIGVGYVCDVGSVSEYRLSEIKPLHNFLTQLQPFLKLKQKQANLVLKIIEQLPSAKESPDKFLEVCTWVDQIAALNDSKTRKTTSETVRAVLDSLSEKKKSSP

SEQ ID NO: 14 - protein, 354 aa, synthetic construct
  REGION 1..354: note = Synthetic Polypeptide
MNTKYNKEFLLYLAGFVDGDGSIYARIEPRQTAKFKHYLRLTFHVSQKTQRRWFLDKLVDEIGVGYVVDQGSVSQYYLSQIKPLHNFLTQLQPFLKLKQKQANLVLKIIEQLPSAKESPDKFLEVCTWVDQIAALNDSKTRKTTSETVRAVLDSLPGSVGGLSPSQASSAASSASSSPGSGISEALRAGAGSGTGYNKEFLLYLAGFVDGDGSIYASITPSQAGKFKHRLRLYFEVSQKTQRRWFLDKLVDEIGVGYVYDQGSVSCYRLSQIKPLHNFLTQLQPFLKLKQKQANLVLKIIEQLPSAKESPDKFLEVCTWVDQIAALNDSKTRKTTSETVRAVLDSLSEKKKSSP

SEQ ID NO: 15 - protein, 354 aa, synthetic construct
  REGION 1..354: note = Synthetic Polypeptide
MNTKYNKEFLLYLAGFVDGDGSIYARIYPKQSSKFKHHLRLTFHVSQKTQRRWFLDKLVDEIGVGYVYDSGSVSQYYLSEIKPLHNFLTQLQPFLKLKQKQANLVLKIIEQLPSAKESPDKFLEVCTWVDQIAALNDSKTRKTTSETVRAVLDSLPGSVGGLSPSQASSAASSASSSPGSGISEALRAGAGSGTGYNKEFLLYLAGFVDGDGSIYATIEPAQRYKFKHRLRLKFAVSQKTQRRWFLDKLVDEIGVGYVADQGSVSEYRLSQIKPLHNFLTQLQPFLKLKQKQANLVLKIIEQLPSAKESPDKFLEVCTWVDQIAALNDSKTRKTTSETVRAVLDSLSEKKKSSP

SEQ ID NO: 16 - protein, 354 aa, synthetic construct
  REGION 1..354: note = Synthetic Polypeptide
MNTKYNKEFLLYLAGFVDGDGSIYARIEPEQTAKFKHMLRLTFRVSQKTQRRWFLDKLVDEIGVGYVNDSGSVSGYYLSQIKPLHNFLTQLQPFLKLKQKQANLVLKIIEQLPSAKESPDKFLEVCTWVDQIAALNDSKTRKTTSETVRAVLDSLPGSVGGLSPSQASSAASSASSSPGSGISEALRAGAGSGTGYNKEFLLYLAGFVDGDGSIYATIEPQQPGKFKHRLSLRFAVYQKTQRRWFLDKLVDEIGVGYVYDPGSVSEYRLSQIKPLHNFLTQLQPFLKLKQKQANLVLKIIEQLPSAKESPDKFLEVCTWVDQIAALNDSKTRKTTSETVRAVLDSLSEKKKSSP

SEQ ID NO: 17 - protein, 354 aa, synthetic construct
  REGION 1..354: note = Synthetic Polypeptide
MNTKYNKEFLLYLAGFVDGDGSIYARIEPRQTAKFKHYLRLTFHVSQKTQRRWFLDKLVDEIGVGYVVDQGSVSQYFLSQIKPLHNFLTQLQPFLKLKQKQANLVLKIIEQLPSAKESPDKFLEVCTWVDQIAALNDSKTRKTTSETVRAVLDSLPGSVGGLSPSQASSAASSASSSPGSGISEALRAGAGSGTGYNKEFLLYLAGFVDGDGSIYASIGPEQSSKFKHRLRLLFAVAQKTQRRWFLDKLVDEIGVGYVVDQGSVSEYRLSQIKPLHNFLTQLQPFLKLKQKQANLVLKIIEQLPSAKESPDKFLEVCTWVDQIAALNDSKTRKTTSETVRAVLDSLSEKKKSSP

SEQ ID NO: 18 - protein, 354 aa, synthetic construct
  REGION 1..354: note = Synthetic Polypeptide
MNTKYNKEFLLYLAGFVDGDGSIYARIEPKQTAKFKHHLCLRFHVSQKTQRRWFLDKLVDEIGVGYVVDHGSVSQYFLSQIKPLHNFLTQLQPFLKLKQKQANLVLKIIEQLPSAKESPDKFLEVCTWVDQIAALNDSKTRKTTSETVRAVLDSLPGSVGGLSPSQASSAASSASSSPGSGISEALRAGAGSGTGYNKEFLLYLAGFVDGDGSIYATIQPDQNQKFKHRLRLYFAVYQKTQRRWFLDKLVDEIGVGYVYDTGSVSRYQLSQIKPLHNFLTQLQPFLKLKQKQANLVLKIIEQLPSAKESPDKFLEVCTWVDQIAALNDSKTRKTTSETVRAVLDSLSEKKKSSP

SEQ ID NO: 19 - protein, 354 aa, synthetic construct; identical to SEQ ID NO: 9
  REGION 1..354: note = Synthetic Polypeptide

SEQ ID NO: 20 - protein, 354 aa, synthetic construct
  REGION 1..354: note = Synthetic Polypeptide
MNTKYNKEFLLYLAGFVDGDGSIYARIEPRQRVKFKHFLRLTFHVSQKTQRRWFLDKLVDEIGVGYVTDWGSVSGYYLSEIKPLHNFLTQLQPFLKLKQKQANLVLKIIEQLPSAKESPDKFLEVCTWVDQIAALNDSKTRKTTSETVRAVLDSLPGSVGGLSPSQASSAASSASSSPGSGISEALRAGAGSGTGYNKEFLLYLAGFVDGDGSIWASIIPEQGYKFKHRLRLSFTVAQKTQRRWFLDKLVDEIGVGYVVDQGSVSEYRLSEIKPLHNFLTQLQPFLKLKQKQANLVLKIIEQLPSAKESPDKFLEVCTWVDQIAALNDSKTRKTTSETVRAVLDSLSEKKKSSP

SEQ ID NO: 21 - protein, 354 aa, synthetic construct
  REGION 1..354: note = Synthetic Polypeptide
MNTKYNKEFLLYLAGFVDGDGSIYARIEPRQGCKFKHVLRLTFHVSQKTQRRWFLDKLVDEIGVGYVTDWGSVSGYYLSEIKPLHNFLTQLQPFLKLKQKQANLVLKIIEQLPSAKESPDKFLEVCTWVDQIAALNDSKTRKTTSETVRAVLDSLPGSVGGLSPSQASSAASSASSSPGSGISEALRAGAGSGTGYNKEFLLYLAGFVDGDGSIWASIIPEQGYKFKHRLRLSFTVAQKTQRRWFLDKLVDEIGVGYVVDQGSVSEYRLSEIKPLHNFLTQLQPFLKLKQKQANLVLKIIEQLPSAKESPDKFLEVCTWVDQIAALNDSKTRKTTSETVRAVLDSLSEKKKSSP

SEQ ID NO: 22 - protein, 354 aa, synthetic construct
  REGION 1..354: note = Synthetic Polypeptide
MNTKYNKEFLLYLAGFVDGDGSIYARIEPRQVCKFKHILRLTFHVSQKTQRRWFLDKLVDEIGVGYVTDWGSVSGYYLSEIKPLHNFLTQLQPFLKLKQKQANLVLKIIEQLPSAKESPDKFLEVCTWVDQIAALNDSKTRKTTSETVRAVLDSLPGSVGGLSPSQASSAASSASSSPGSGISEALRAGAGSGTGYNKEFLLYLAGFVDGDGSIWASIIPEQGYKFKHRLRLSFTVAQKTQRRWFLDKLVDEIGVGYVVDQGSVSEYRLSEIKPLHNFLTQLQPFLKLKQKQANLVLKIIEQLPSAKESPDKFLEVCTWVDQIAALNDSKTRKTTSETVRAVLDSLSEKKKSSP

SEQ ID NO: 23 - protein, 354 aa, synthetic construct
  REGION 1..354: note = Synthetic Polypeptide
MNTKYNKEFLLYLAGFVDGDGSIYARIEPRQCFKFKHCLRLTFHVSQKTQRRWFLDKLVDEIGVGYVTDWGSVSGYYLSEIKPLHNFLTQLQPFLKLKQKQANLVLKIIEQLPSAKESPDKFLEVCTWVDQIAALNDSKTRKTTSETVRAVLDSLPGSVGGLSPSQASSAASSASSSPGSGISEALRAGAGSGTGYNKEFLLYLAGFVDGDGSIWASIIPEQGYKFKHRLRLSFTVAQKTQRRWFLDKLVDEIGVGYVVDQGSVSEYRLSEIKPLHNFLTQLQPFLKLKQKQANLVLKIIEQLPSAKESPDKFLEVCTWVDQIAALNDSKTRKTTSETVRAVLDSLSEKKKSSP

SEQ ID NO: 24 - protein, 354 aa, synthetic construct
  REGION 1..354: note = Synthetic Polypeptide
MNTKYNKEFLLYLAGFVDGDGSIYARIEPRQRFKFKHCLRLTFHVSQKTQRRWFLDKLVDEIGVGYVTDWGSVSGYYLSEIKPLHNFLTQLQPFLKLKQKQANLVLKIIEQLPSAKESPDKFLEVCTWVDQIAALNDSKTRKTTSETVRAVLDSLPGSVGGLSPSQASSAASSASSSPGSGISEALRAGAGSGTGYNKEFLLYLAGFVDGDGSIWASIIPEQGYKFKHRLRLSFTVAQKTQRRWFLDKLVDEIGVGYVVDQGSVSEYRLSEIKPLHNFLTQLQPFLKLKQKQANLVLKIIEQLPSAKESPDKFLEVCTWVDQIAALNDSKTRKTTSETVRAVLDSLSEKKKSSP

SEQ ID NO: 25 - protein, 354 aa, synthetic construct
  REGION 1..354: note = Synthetic Polypeptide
MNTKYNKEFLLYLAGFVDGDGSIYARIEPRQFCKFKHILRLTFHVSQKTQRRWFLDKLVDEIGVGYVTDWGSVSGYYLSEIKPLHNFLTQLQPFLKLKQKQANLVLKIIEQLPSAKESPDKFLEVCTWVDQIAALNDSKTRKTTSETVRAVLDSLPGSVGGLSPSQASSAASSASSSPGSGISEALRAGAGSGTGYNKEFLLYLAGFVDGDGSIWASIIPEQGYKFKHRLRLSFTVAQKTQRRWFLDKLVDEIGVGYVVDQGSVSEYRLSEIKPLHNFLTQLQPFLKLKQKQANLVLKIIEQLPSAKESPDKFLEVCTWVDQIAALNDSKTRKTTSETVRAVLDSLSEKKKSSP

SEQ ID NO: 26 - protein, 354 aa, synthetic construct
  REGION 1..354: note = Synthetic Polypeptide
MNTKYNKEFLLYLAGFVDGDGSIYARIEPRQAFKFKHALRLTFHVSQKTQRRWFLDKLVDEIGVGYVTDWGSVSGYYLSEIKPLHNFLTQLQPFLKLKQKQANLVLKIIEQLPSAKESPDKFLEVCTWVDQIAALNDSKTRKTTSETVRAVLDSLPGSVGGLSPSQASSAASSASSSPGSGISEALRAGAGSGTGYNKEFLLYLAGFVDGDGSIWASIIPEQGYKFKHRLRLSFTVAQKTQRRWFLDKLVDEIGVGYVVDQGSVSEYRLSEIKPLHNFLTQLQPFLKLKQKQANLVLKIIEQLPSAKESPDKFLEVCTWVDQIAALNDSKTRKTTSETVRAVLDSLSEKKKSSP

SEQ ID NO: 27 - protein, 354 aa, synthetic construct
  REGION 1..354: note = Synthetic Polypeptide
MNTKYNKEFLLYLAGFVDGDGSIYARIEPRQTCKFKHILRLTFHVSQKTQRRWFLDKLVDEIGVGYVTDWGSVSGYYLSEIKPLHNFLTQLQPFLKLKQKQANLVLKIIEQLPSAKESPDKFLEVCTWVDQIAALNDSKTRKTTSETVRAVLDSLPGSVGGLSPSQASSAASSASSSPGSGISEALRAGAGSGTGYNKEFLLYLAGFVDGDGSIWASIIPEQGYKFKHRLRLSFTVAQKTQRRWFLDKLVDEIGVGYVVDQGSVSEYRLSEIKPLHNFLTQLQPFLKLKQKQANLVLKIIEQLPSAKESPDKFLEVCTWVDQIAALNDSKTRKTTSETVRAVLDSLSEKKKSSP

SEQ ID NO: 28 - protein, 354 aa, synthetic construct
  REGION 1..354: note = Synthetic Polypeptide
MNTKYNKEFLLYLAGFVDGDGSIYARIEPRQCFKFKHGLRLTFHVSQKTQRRWFLDKLVDEIGVGYVTDWGSVSGYYLSEIKPLHNFLTQLQPFLKLKQKQANLVLKIIEQLPSAKESPDKFLEVCTWVDQIAALNDSKTRKTTSETVRAVLDSLPGSVGGLSPSQASSAASSASSSPGSGISEALRAGAGSGTGYNKEFLLYLAGFVDGDGSIWASIIPEQGYKFKHRLRLSFTVAQKTQRRWFLDKLVDEIGVGYVVDQGSVSEYRLSEIKPLHNFLTQLQPFLKLKQKQANLVLKIIEQLPSAKESPDKFLEVCTWVDQIAALNDSKTRKTTSETVRAVLDSLSEKKKSSP

SEQ ID NO: 29 - protein, 354 aa, synthetic construct
  REGION 1..354: note = Synthetic Polypeptide
MNTKYNKEFLLYLAGFVDGDGSIYARIEPRQSSKFKHLLRLTFHVSQKTQRRWFLDKLVDEIGVGYVTDWGSVSGYYLSEIKPLHNFLTQLQPFLKLKQKQANLVLKIIEQLPSAKESPDKFLEVCTWVDQIAALNDSKTRKTTSETVRAVLDSLPGSVGGLSPSQASSAASSASSSPGSGISEALRAGAGSGTGYNKEFLLYLAGFVDGDGSIWASIIPEQGYKFKHRLRLSFTVAQKTQRRWFLDKLVDEIGVGYVVDQGSVSEYRLSEIKPLHNFLTQLQPFLKLKQKQANLVLKIIEQLPSAKESPDKFLEVCTWVDQIAALNDSKTRKTTSETVRAVLDSLSEKKKSSP

SEQ ID NO: 30 - protein, 354 aa, synthetic construct
  REGION 1..354: note = Synthetic Polypeptide
MNTKYNKEFLLYLAGFVDGDGSIYARIYLGQHWKFKHYVRLTFHVSQKTQRRWFLDKLVDEIGVGYVTDWGSVSGYYLSEIKPLHNFLTQLQPFLKLKQKQANLVLKIIEQLPSAKESPDKFLEVCTWVDQIAALNDSKTRKTTSETVRAVLDSLPGSVGGLSPSQASSAASSASSSPGSGISEALRAGAGSGTGYNKEFLLYLAGFVDGDGSIWASIIPEQGYKFKHRLRLSFTVAQKTQRRWFLDKLVDEIGVGYVVDQGSVSEYRLSEIKPLHNFLTQLQPFLKLKQKQANLVLKIIEQLPSAKESPDKFLEVCTWVDQIAALNDSKTRKTTSETVRAVLDSLSEKKKSSP

SEQ ID NO: 31 - protein, 354 aa, synthetic construct
  REGION 1..354: note = Synthetic Polypeptide
MNTKYNKEFLLYLAGFVDGDGSIYARIYLGQHYKFKHYIRLTFHVSQKTQRRWFLDKLVDEIGVGYVTDWGSVSGYYLSEIKPLHNFLTQLQPFLKLKQKQANLVLKIIEQLPSAKESPDKFLEVCTWVDQIAALNDSKTRKTTSETVRAVLDSLPGSVGGLSPSQASSAASSASSSPGSGISEALRAGAGSGTGYNKEFLLYLAGFVDGDGSIWASIIPEQGYKFKHRLRLSFTVAQKTQRRWFLDKLVDEIGVGYVVDQGSVSEYRLSEIKPLHNFLTQLQPFLKLKQKQANLVLKIIEQLPSAKESPDKFLEVCTWVDQIAALNDSKTRKTTSETVRAVLDSLSEKKKSSP

SEQ ID NO: 32 - protein, 354 aa, synthetic construct
  REGION 1..354: note = Synthetic Polypeptide
MNTKYNKEFLLYLAGFVDGDGSIYARIYNAQYYKFKHYIRLTFHVSQKTQRRWFLDKLVDEIGVGYVTDWGSVSGYYLSEIKPLHNFLTQLQPFLKLKQKQANLVLKIIEQLPSAKESPDKFLEVCTWVDQIAALNDSKTRKTTSETVRAVLDSLPGSVGGLSPSQASSAASSASSSPGSGISEALRAGAGSGTGYNKEFLLYLAGFVDGDGSIWASIIPEQGYKFKHRLRLSFTVAQKTQRRWFLDKLVDEIGVGYVVDQGSVSEYRLSEIKPLHNFLTQLQPFLKLKQKQANLVLKIIEQLPSAKESPDKFLEVCTWVDQIAALNDSKTRKTTSETVRAVLDSLSEKKKSSP

SEQ ID NO: 33 - protein, 354 aa, synthetic construct
  REGION 1..354: note = Synthetic Polypeptide
MNTKYNKEFLLYLAGFVDGDGSIYARIERRQNFKFKHHIRLTFHVSQKTQRRWFLDKLVDEIGVGYVTDWGSVSGYYLSEIKPLHNFLTQLQPFLKLKQKQANLVLKIIEQLPSAKESPDKFLEVCTWVDQIAALNDSKTRKTTSETVRAVLDSLPGSVGGLSPSQASSAASSASSSPGSGISEALRAGAGSGTGYNKEFLLYLAGFVDGDGSIWASIIPEQGYKFKHRLRLSFTVAQKTQRRWFLDKLVDEIGVGYVVDQGSVSEYRLSEIKPLHNFLTQLQPFLKLKQKQANLVLKIIEQLPSAKESPDKFLEVCTWVDQIAALNDSKTRKTTSETVRAVLDSLSEKKKSSP

SEQ ID NO: 34 - protein, 354 aa, synthetic construct
  REGION 1..354: note = Synthetic Polypeptide
MNTKYNKEFLLYLAGFVDGDGSIYARIERRQCVKFKHYLRLTFHVSQKTQRRWFLDKLVDEIGVGYVTDWGSVSGYYLSEIKPLHNFLTQLQPFLKLKQKQANLVLKIIEQLPSAKESPDKFLEVCTWVDQIAALNDSKTRKTTSETVRAVLDSLPGSVGGLSPSQASSAASSASSSPGSGISEALRAGAGSGTGYNKEFLLYLAGFVDGDGSIWASIIPEQGYKFKHRLRLSFTVAQKTQRRWFLDKLVDEIGVGYVVDQGSVSEYRLSEIKPLHNFLTQLQPFLKLKQKQANLVLKIIEQLPSAKESPDKFLEVCTWVDQIAALNDSKTRKTTSETVRAVLDSLSEKKKSSP

SEQ ID NO: 35 - protein, 354 aa, synthetic construct
  REGION 1..354: note = Synthetic Polypeptide
MNTKYNKEFLLYLAGFVDGDGSIYARIEYRQGAKFKHYLRLTFHVSQKTQRRWFLDKLVDEIGVGYVTDWGSVSGYYLSEIKPLHNFLTQLQPFLKLKQKQANLVLKIIEQLPSAKESPDKFLEVCTWVDQIAALNDSKTRKTTSETVRAVLDSLPGSVGGLSPSQASSAASSASSSPGSGISEALRAGAGSGTGYNKEFLLYLAGFVDGDGSIWASIIPEQGYKFKHRLRLSFTVAQKTQRRWFLDKLVDEIGVGYVVDQGSVSEYRLSEIKPLHNFLTQLQPFLKLKQKQANLVLKIIEQLPSAKESPDKFLEVCTWVDQIAALNDSKTRKTTSETVRAVLDSLSEKKKSSP

SEQ ID NO: 36 - protein, 354 aa, synthetic construct
  REGION 1..354: note = Synthetic Polypeptide
MNTKYNKEFLLYLAGFVDGDGSIYARIEPRQSGKFKHYIRLTFHVSQKTQRRWFLDKLVDEIGVGYVTDWGSVSGYYLSEIKPLHNFLTQLQPFLKLKQKQANLVLKIIEQLPSAKESPDKFLEVCTWVDQIAALNDSKTRKTTSETVRAVLDSLPGSVGGLSPSQASSAASSASSSPGSGISEALRAGAGSGTGYNKEFLLYLAGFVDGDGSIWASIIPEQGYKFKHRLRLSFTVAQKTQRRWFLDKLVDEIGVGYVVDQGSVSEYRLSEIKPLHNFLTQLQPFLKLKQKQANLVLKIIEQLPSAKESPDKFLEVCTWVDQIAALNDSKTRKTTSETVRAVLDSLSEKKKSSP

SEQ ID NO: 37 - protein, 354 aa, synthetic construct
  REGION 1..354: note = Synthetic Polypeptide
MNTKYNKEFLLYLAGFVDGDGSIYARIFKGQHWKFKHHIRLTFNVSQKTQRRWFLDKLVDEIGVGYVSDTGSQSNYYLSEIKPLHNFLTQLQPFLKLKQKQANLVLKIIEQLPSAKESPDKFLEVCTWVDQIAALNDSKTRKTTSETVRAVLDSLPGSVGGLSPSQASSAASSASSSPGSGISEALRAGAGSGTGYNKEFLLYLAGFVDGDGSIWASIIPEQGYKFKHRLRLSFTVAQKTQRRWFLDKLVDEIGVGYVVDQGSVSEYRLSEIKPLHNFLTQLQPFLKLKQKQANLVLKIIEQLPSAKESPDKFLEVCTWVDQIAALNDSKTRKTTSETVRAVLDSLSEKKKSSP

SEQ ID NO: 38 - protein, 354 aa, synthetic construct
  REGION 1..354: note = Synthetic Polypeptide
MNTKYNKEFLLYLAGFVDGDGSIFARIFKGQHWKFKHHIRLTFNVSQKTQRRWFLDKLVDEIGVGYVNDYGSTSNYYLSEIKPLHNFLTQLQPFLKLKQKQANLVLKIIEQLPSAKESPDKFLEVCTWVDQIAALNDSKTRKTTSETVRAVLDSLPGSVGGLSPSQASSAASSASSSPGSGISEALRAGAGSGTGYNKEFLLYLAGFVDGDGSIWASIIPEQGYKFKHRLRLSFTVAQKTQRRWFLDKLVDEIGVGYVVDQGSVSEYRLSEIKPLHNFLTQLQPFLKLKQKQANLVLKIIEQLPSAKESPDKFLEVCTWVDQIAALNDSKTRKTTSETVRAVLDSLSEKKKSSP

SEQ ID NO: 39 - protein, 354 aa, synthetic construct
  REGION 1..354: note = Synthetic Polypeptide
MNTKYNKEFLLYLAGFVDGDGSIFARIFKGQHWKFKHHIRLTFNVAQKTQRRWFLDKLVDEIGVGYVTDHGSNSNYYLSEIKPLHNFLTQLQPFLKLKQKQANLVLKIIEQLPSAKESPDKFLEVCTWVDQIAALNDSKTRKTTSETVRAVLDSLPGSVGGLSPSQASSAASSASSSPGSGISEALRAGAGSGTGYNKEFLLYLAGFVDGDGSIWASIIPEQGYKFKHRLRLSFTVAQKTQRRWFLDKLVDEIGVGYVVDQGSVSEYRLSEIKPLHNFLTQLQPFLKLKQKQANLVLKIIEQLPSAKESPDKFLEVCTWVDQIAALNDSKTRKTTSETVRAVLDSLSEKKKSSP

SEQ ID NO: 40 - protein, 354 aa, synthetic construct
  REGION 1..354: note = Synthetic Polypeptide
MNTKYNKEFLLYLAGFVDGDGSIYARIFKGQHWKFKHHIRLTFNVTQKTQRRWFLDKLVDEIGVGYVSDYGSMSNYYLSEIKPLHNFLTQLQPFLKLKQKQANLVLKIIEQLPSAKESPDKFLEVCTWVDQIAALNDSKTRKTTSETVRAVLDSLPGSVGGLSPSQASSAASSASSSPGSGISEALRAGAGSGTGYNKEFLLYLAGFVDGDGSIWASIIPEQGYKFKHRLRLSFTVAQKTQRRWFLDKLVDEIGVGYVVDQGSVSEYRLSEIKPLHNFLTQLQPFLKLKQKQANLVLKIIEQLPSAKESPDKFLEVCTWVDQIAALNDSKTRKTTSETVRAVLDSLSEKKKSSP

SEQ ID NO: 41 - protein, 354 aa, synthetic construct
  REGION 1..354: note = Synthetic Polypeptide
MNTKYNKEFLLYLAGFVDGDGSIYARIFKGQHWKFKHHIRLTFAVTQKTQRRWFLDKLVDEIGVGYVTDHGSCSNYYLSEIKPLHNFLTQLQPFLKLKQKQANLVLKIIEQLPSAKESPDKFLEVCTWVDQIAALNDSKTRKTTSETVRAVLDSLPGSVGGLSPSQASSAASSASSSPGSGISEALRAGAGSGTGYNKEFLLYLAGFVDGDGSIWASIIPEQGYKFKHRLRLSFTVAQKTQRRWFLDKLVDEIGVGYVVDQGSVSEYRLSEIKPLHNFLTQLQPFLKLKQKQANLVLKIIEQLPSAKESPDKFLEVCTWVDQIAALNDSKTRKTTSETVRAVLDSLSEKKKSSP

SEQ ID NO: 42 - protein, 354 aa, synthetic construct
  REGION 1..354: note = Synthetic Polypeptide
MNTKYNKEFLLYLAGFVDGDGSIYARIFKGQHWKFKHHIRLTFNVSQKTQRRWFLDKLVDEIGVGYVGDYGSMSHYYLSEIKPLHNFLTQLQPFLKLKQKQANLVLKIIEQLPSAKESPDKFLEVCTWVDQIAALNDSKTRKTTSETVRAVLDSLPGSVGGLSPSQASSAASSASSSPGSGISEALRAGAGSGTGYNKEFLLYLAGFVDGDGSIWASIIPEQGYKFKHRLRLSFTVAQKTQRRWFLDKLVDEIGVGYVVDQGSVSEYRLSEIKPLHNFLTQLQPFLKLKQKQANLVLKIIEQLPSAKESPDKFLEVCTWVDQIAALNDSKTRKTTSETVRAVLDSLSEKKKSSP

SEQ ID NO: 43 - protein, 354 aa, synthetic construct
  REGION 1..354: note = Synthetic Polypeptide
MNTKYNKEFLLYLAGFVDGDGSIYARIFKGQHWKFKHHIRLTFNVSQKTQRRWFLDKLVDEIGVGYVTDFGSQSQYYLSEIKPLHNFLTQLQPFLKLKQKQANLVLKIIEQLPSAKESPDKFLEVCTWVDQIAALNDSKTRKTTSETVRAVLDSLPGSVGGLSPSQASSAASSASSSPGSGISEALRAGAGSGTGYNKEFLLYLAGFVDGDGSIWASIIPEQGYKFKHRLRLSFTVAQKTQRRWFLDKLVDEIGVGYVVDQGSVSEYRLSEIKPLHNFLTQLQPFLKLKQKQANLVLKIIEQLPSAKESPDKFLEVCTWVDQIAALNDSKTRKTTSETVRAVLDSLSEKKKSSP

SEQ ID NO: 44 - protein, 354 aa, synthetic construct
  REGION 1..354: note = Synthetic Polypeptide
MNTKYNKEFLLYLAGFVDGDGSIFARIFKGQHWKFKHHIRLTFNVTQKTQRRWFLDKLVDEIGVGYVSDYGSISNYYLSEIKPLHNFLTQLQPFLKLKQKQANLVLKIIEQLPSAKESPDKFLEVCTWVDQIAALNDSKTRKTTSETVRAVLDSLPGSVGGLSPSQASSAASSASSSPGSGISEALRAGAGSGTGYNKEFLLYLAGFVDGDGSIWASIIPEQGYKFKHRLRLSFTVAQKTQRRWFLDKLVDEIGVGYVVDQGSVSEYRLSEIKPLHNFLTQLQPFLKLKQKQANLVLKIIEQLPSAKESPDKFLEVCTWVDQIAALNDSKTRKTTSETVRAVLDSLSEKKKSSP

SEQ ID NO: 45 - protein, 354 aa, synthetic construct
  REGION 1..354: note = Synthetic Polypeptide
MNTKYNKEFLLYLAGFVDGDGSIYARIFKGQHWKFKHHIRLTFNVTQKTQRRWFLDKLVDEIGVGYVIDYGSISNYYLSEIKPLHNFLTQLQPFLKLKQKQANLVLKIIEQLPSAKESPDKFLEVCTWVDQIAALNDSKTRKTTSETVRAVLDSLPGSVGGLSPSQASSAASSASSSPGSGISEALRAGAGSGTGYNKEFLLYLAGFVDGDGSIWASIIPEQGYKFKHRLRLSFTVAQKTQRRWFLDKLVDEIGVGYVVDQGSVSEYRLSEIKPLHNFLTQLQPFLKLKQKQANLVLKIIEQLPSAKESPDKFLEVCTWVDQIAALNDSKTRKTTSETVRAVLDSLSEKKKSSP

SEQ ID NO: 46 - protein, 354 aa, synthetic construct
  REGION 1..354: note = Synthetic Polypeptide
MNTKYNKEFLLYLAGFVDGDGSIYARIFKGQHWKFKHHIRLTFNVTQKTQRRWFLDKLVDEIGVGYVTDYGSSSNYYLSEIKPLHNFLTQLQPFLKLKQKQANLVLKIIEQLPSAKESPDKFLEVCTWVDQIAALNDSKTRKTTSETVRAVLDSLPGSVGGLSPSQASSAASSASSSPGSGISEALRAGAGSGTGYNKEFLLYLAGFVDGDGSIWASIIPEQGYKFKHRLRLSFTVAQKTQRRWFLDKLVDEIGVGYVVDQGSVSEYRLSEIKPLHNFLTQLQPFLKLKQKQANLVLKIIEQLPSAKESPDKFLEVCTWVDQIAALNDSKTRKTTSETVRAVLDSLSEKKKSSP

SEQ ID NO: 47 - protein, 354 aa, synthetic construct
  REGION 1..354: note = Synthetic Polypeptide
MNTKYNKEFLLYLAGFVDGDGSIFARIFKGQHWKFKHHIRLTFNVSQKTQRRWFLDKLVDEIGVGYVTDGGSSSNYYLSEIKPLHNFLTQLQPFLKLKQKQANLVLKIIEQLPSAKESPDKFLEVCTWVDQIAALNDSKTRKTTSETVRAVLDSLPGSVGGLSPSQASSAASSASSSPGSGISEALRAGAGSGTGYNKEFLLYLAGFVDGDGSIWASIIPEQGYKFKHRLRLSFTVAQKTQRRWFLDKLVDEIGVGYVVDQGSVSEYRLSEIKPLHNFLTQLQPFLKLKQKQANLVLKIIEQLPSAKESPDKFLEVCTWVDQIAALNDSKTRKTTSETVRAVLDSLSEKKKSSP

SEQ ID NO: 48 - protein, 354 aa, synthetic construct
  REGION 1..354: note = Synthetic Polypeptide
MNTKYNKEFLLYLAGFVDGDGSIFARIFKGQHWKFKHHIRLTFNVSQKTQRRWFLDKLVDEIGVGYVYDHGSQSNYYLSEIKPLHNFLTQLQPFLKLKQKQANLVLKIIEQLPSAKESPDKFLEVCTWVDQIAALNDSKTRKTTSETVRAVLDSLPGSVGGLSPSQASSAASSASSSPGSGISEALRAGAGSGTGYNKEFLLYLAGFVDGDGSIWASIIPEQGYKFKHRLRLSFTVAQKTQRRWFLDKLVDEIGVGYVVDQGSVSEYRLSEIKPLHNFLTQLQPFLKLKQKQANLVLKIIEQLPSAKESPDKFLEVCTWVDQIAALNDSKTRKTTSETVRAVLDSLSEKKKSSP

SEQ ID NO: 49 - protein, 354 aa, synthetic construct
  REGION 1..354: note = Synthetic Polypeptide
MNTKYNKEFLLYLAGFVDGDGSIYARIFKGQHWKFKHHIRLTFNVSQKTQRRWFLDKLVDEIGVGYVCDNGSNSNYYLSEIKPLHNFLTQLQPFLKLKQKQANLVLKIIEQLPSAKESPDKFLEVCTWVDQIAALNDSKTRKTTSETVRAVLDSLPGSVGGLSPSQASSAASSASSSPGSGISEALRAGAGSGTGYNKEFLLYLAGFVDGDGSIWASIIPEQGYKFKHRLRLSFTVAQKTQRRWFLDKLVDEIGVGYVVDQGSVSEYRLSEIKPLHNFLTQLQPFLKLKQKQANLVLKIIEQLPSAKESPDKFLEVCTWVDQIAALNDSKTRKTTSETVRAVLDSLSEKKKSSP

SEQ ID NO: 50 - protein, 354 aa, synthetic construct
  REGION 1..354: note = Synthetic Polypeptide
MNTKYNKEFLLYLAGFVDGDGSIFARIFKGQHWKFKHHIRLTFNVSQKTQRRWFLDKLVDEIGVGYVADYGSTSNYYLSEIKPLHNFLTQLQPFLKLKQKQANLVLKIIEQLPSAKESPDKFLEVCTWVDQIAALNDSKTRKTTSETVRAVLDSLPGSVGGLSPSQASSAASSASSSPGSGISEALRAGAGSGTGYNKEFLLYLAGFVDGDGSIWASIIPEQGYKFKHRLRLSFTVAQKTQRRWFLDKLVDEIGVGYVVDQGSVSEYRLSEIKPLHNFLTQLQPFLKLKQKQANLVLKIIEQLPSAKESPDKFLEVCTWVDQIAALNDSKTRKTTSETVRAVLDSLSEKKKSSP

SEQ ID NO: 51 - protein, 354 aa, synthetic construct
  REGION 1..354: note = Synthetic Polypeptide
MNTKYNKEFLLYLAGFVDGDGSIYARIFKGQHWKFKHHIRLTFCVSQKTQRRWFLDKLVDEIGVGYVADYGSMSNYYLSEIKPLHNFLTQLQPFLKLKQKQANLVLKIIEQLPSAKESPDKFLEVCTWVDQIAALNDSKTRKTTSETVRAVLDSLPGSVGGLSPSQASSAASSASSSPGSGISEALRAGAGSGTGYNKEFLLYLAGFVDGDGSIWASIIPEQGYKFKHRLRLSFTVAQKTQRRWFLDKLVDEIGVGYVVDQGSVSEYRLSEIKPLHNFLTQLQPFLKLKQKQANLVLKIIEQLPSAKESPDKFLEVCTWVDQIAALNDSKTRKTTSETVRAVLDSLSEKKKSSP

SEQ ID NO: 52 - protein, 354 aa, synthetic construct
  REGION 1..354: note = Synthetic Polypeptide
MNTKYNKEFLLYLAGFVDGDGSIMARIFKGQHWKFKHYIRLTLCVRQKTQRRWFLDKLVDEIGVGYVCDSGSMSAYYLSEIKPLHNFLTQLQPFLKLKQKQANLVLKIIEQLPSAKESPDKFLEVCTWVDQIAALNDSKTRKTTSETVRAVLDSLPGSVGGLSPSQASSAASSASSSPGSGISEALRAGAGSGTGYNKEFLLYLAGFVDGDGSIWASIIPEQGYKFKHRLRLSFTVAQKTQRRWFLDKLVDEIGVGYVVDQGSVSEYRLSEIKPLHNFLTQLQPFLKLKQKQANLVLKIIEQLPSAKESPDKFLEVCTWVDQIAALNDSKTRKTTSETVRAVLDSLSEKKKSSP

SEQ ID NO: 53 - protein, 354 aa, synthetic construct; identical to SEQ ID NO: 47
  REGION 1..354: note = Synthetic Polypeptide

SEQ ID NO: 54 - protein, 354 aa, synthetic construct
  REGION 1..354: note = Synthetic Polypeptide
MNTKYNKEFLLYLAGFVDGDGSIYARIFKGQHWKFKHHIRLTFHVSQKTQRRWFLDKLVDEIGVGYVTDWGSVSGYYLSEIKPLHNFLTQLQPFLKLKQKQANLVLKIIEQLPSAKESPDKFLEVCTWVDQIAALNDSKTRKTTSETVRAVLDSLPGSVGGLSPSQASSAASSASSSPGSGISEALRAGAGSGTGYNKEFLLYLAGFVDGDGSIWASILPESRMKFKHRLRLGFTVAQKTQRRWFLDKLVDEIGVGYVVDQGSVSEYRLSEIKPLHNFLTQLQPFLKLKQKQANLVLKIIEQLPSAKESPDKFLEVCTWVDQIAALNDSKTRKTTSETVRAVLDSLSEKKKSSP

SEQ ID NO: 55 - protein, 354 aa, synthetic construct
  REGION 1..354: note = Synthetic Polypeptide
MNTKYNKEFLLYLAGFVDGDGSIYARIFKGQHWKFKHHIRLTFHVSQKTQRRWFLDKLVDEIGVGYVTDWGSVSGYYLSEIKPLHNFLTQLQPFLKLKQKQANLVLKIIEQLPSAKESPDKFLEVCTWVDQIAALNDSKTRKTTSETVRAVLDSLPGSVGGLSPSQASSAASSASSSPGSGISEALRAGAGSGTGYNKEFLLYLAGFVDGDGSIWAQILPEKKCAFKHRLRLWFTVAQKTQRRWFLDKLVDEIGVGYVVDQGSVSEYRLSEIKPLHNFLTQLQPFLKLKQKQANLVLKIIEQLPSAKESPDKFLEVCTWVDQIAALNDSKTRKTTSETVRAVLDSLSEKKKSSP

SEQ ID NO: 56 - protein, 354 aa, synthetic construct
  REGION 1..354: note = Synthetic Polypeptide
MNTKYNKEFLLYLAGFVDGDGSIYARIFKGQHWKFKHHIRLTFHVSQKTQRRWFLDKLVDEIGVGYVTDWGSVSGYYLSEIKPLHNFLTQLQPFLKLKQKQANLVLKIIEQLPSAKESPDKFLEVCTWVDQIAALNDSKTRKTTSETVRAVLDSLPGSVGGLSPSQASSAASSASSSPGSGISEALRAGAGSGTGYNKEFLLYLAGFVDGDGSIWACIVPEKASRFKHRLRLAFTVAQKTQRRWFLDKLVDEIGVGYVVDQGSVSEYRLSEIKPLHNFLTQLQPFLKLKQKQANLVLKIIEQLPSAKESPDKFLEVCTWVDQIAALNDSKTRKTTSETVRAVLDSLSEKKKSSP

SEQ ID NO: 57 - protein, 354 aa, synthetic construct
  REGION 1..354: note = Synthetic Polypeptide
MNTKYNKEFLLYLAGFVDGDGSIYARIFKGQHWKFKHHIRLTFHVSQKTQRRWFLDKLVDEIGVGYVTDWGSVSGYYLSEIKPLHNFLTQLQPFLKLKQKQANLVLKIIEQLPSAKESPDKFLEVCTWVDQIAALNDSKTRKTTSETVRAVLDSLPGSVGGLSPSQASSAASSASSSPGSGISEALRAGAGSGTGYNKEFLLYLAGFVDGDGSIWATIVPEKSSIFKHRLRLYFTVAQKTQRRWFLDKLVDEIGVGYVVDQGSVSEYRLSEIKPLHNFLTQLQPFLKLKQKQANLVLKIIEQLPSAKESPDKFLEVCTWVDQIAALNDSKTRKTTSETVRAVLDSLSEKKKSSP

SEQ ID NO: 58 - protein, 354 aa, synthetic construct
  REGION 1..354: note = Synthetic Polypeptide
MNTKYNKEFLLYLAGFVDGDGSIYARIFKGQHWKFKHHIRLTFHVSQKTQRRWFLDKLVDEIGVGYVTDWGSVSGYYLSEIKPLHNFLTQLQPFLKLKQKQANLVLKIIEQLPSAKESPDKFLEVCTWVDQIAALNDSKTRKTTSETVRAVLDSLPGSVGGLSPSQASSAASSASSSPGSGISEALRAGAGSGTGYNKEFLLYLAGFVDGDGSIWASIVPEERTRFKHRLRLYFTVAQKTQRRWFLDKLVDEIGVGYVVDQGSVSEYRLSEIKPLHNFLTQLQPFLKLKQKQANLVLKIIEQLPSAKESPDKFLEVCTWVDQIAALNDSKTRKTTSETVRAVLDSLSEKKKSSP

SEQ ID NO: 59 - protein, 354 aa, synthetic construct
  REGION 1..354: note = Synthetic Polypeptide
MNTKYNKEFLLYLAGFVDGDGSIYARIFKGQHWKFKHHIRLTFHVSQKTQRRWFLDKLVDEIGVGYVTDWGSVSGYYLSEIKPLHNFLTQLQPFLKLKQKQANLVLKIIEQLPSAKESPDKFLEVCTWVDQIAALNDSKTRKTTSETVRAVLDSLPGSVGGLSPSQASSAASSASSSPGSGISEALRAGAGSGTGYNKEFLLYLAGFVDGDGSIWARIEPEKGGRFKHRLRLYFTVAQKTQRRWFLDKLVDEIGVGYVVDQGSVSEYRLSEIKPLHNFLTQLQPFLKLKQKQANLVLKIIEQLPSAKESPDKFLEVCTWVDQIAALNDSKTRKTTSETVRAVLDSLSEKKKSSP

SEQ ID NO: 60 - protein, 354 aa, synthetic construct
  REGION 1..354: note = Synthetic Polypeptide
MNTKYNKEFLLYLAGFVDGDGSIYARIFKGQHWKFKHHIRLTFHVSQKTQRRWFLDKLVDEIGVGYVTDWGSVSGYYLSEIKPLHNFLTQLQPFLKLKQKQANLVLKIIEQLPSAKESPDKFLEVCTWVDQIAALNDSKTRKTTSETVRAVLDSLPGSVGGLSPSQASSAASSASSSPGSGISEALRAGAGSGTGYNKEFLLYLAGFVDGDGSIWASISPEVRAPFKHRLRLYFTVAQKTQRRWFLDKLVDEIGVGYVVDQGSVSEYRLSEIKPLHNFLTQLQPFLKLKQKQANLVLKIIEQLPSAKESPDKFLEVCTWVDQIAALNDSKTRKTTSETVRAVLDSLSEKKKSSP

SEQ ID NO: 61 - protein, 354 aa, synthetic construct
  REGION 1..354: note = Synthetic Polypeptide
MNTKYNKEFLLYLAGFVDGDGSIYARIFKGQHWKFKHHIRLTFHVSQKTQRRWFLDKLVDEIGVGYVTDWGSVSGYYLSEIKPLHNFLTQLQPFLKLKQKQANLVLKIIEQLPSAKESPDKFLEVCTWVDQIAALNDSKTRKTTSETVRAVLDSLPGSVGGLSPSQASSAASSASSSPGSGISEALRAGAGSGTGYNKEFLLYLAGFVDGDGSIWASILPETSARFKHRLRLFFTVAQKTQRRWFLDKLVDEIGVGYVVDQGSVSEYRLSEIKPLHNFLTQLQPFLKLKQKQANLVLKIIEQLPSAKESPDKFLEVCTWVDQIAALNDSKTRKTTSETVRAVLDSLSEKKKSSP

SEQ ID NO: 62 - protein, 354 aa, synthetic construct
  REGION 1..354: note = Synthetic Polypeptide
MNTKYNKEFLLYLAGFVDGDGSIYARIFKGQHWKFKHHIRLTFHVSQKTQRRWFLDKLVDEIGVGYVTDWGSVSGYYLSEIKPLHNFLTQLQPFLKLKQKQANLVLKIIEQLPSAKESPDKFLEVCTWVDQIAALNDSKTRKTTSETVRAVLDSLPGSVGGLSPSQASSAASSASSSPGSGISEALRAGAGSGTGYNKEFLLYLAGFVDGDGSIWAAILPEQSYRFKHRLRLAFTVAQKTQRRWFLDKLVDEIGVGYVVDQGSVSEYRLSEIKPLHNFLTQLQPFLKLKQKQANLVLKIIEQLPSAKESPDKFLEVCTWVDQIAALNDSKTRKTTSETVRAVLDSLSEKKKSSP

SEQ ID NO: 63 - protein, 354 aa, synthetic construct
  REGION 1..354: note = Synthetic Polypeptide
MNTKYNKEFLLYLAGFVDGDGSIYARIFKGQHWKFKHHIRLTFHVSQKTQRRWFLDKLVDEIGVGYVTDWGSVSGYYLSEIKPLHNFLTQLQPFLKLKQKQANLVLKIIEQLPSAKESPDKFLEVCTWVDQIAALNDSKTRKTTSETVRAVLDSLPGSVGGLSPSQASSAASSASSSPGSGISEALRAGAGSGTGYNKEFLLYLAGFVDGDGSIWASILPERKTKFKHRLRLAFTVAQKTQRRWFLDKLVDEIGVGYVVDQGSVSEYRLSEIKPLHNFLTQLQPFLKLKQKQANLVLKIIEQLPSAKESPDKFLEVCTWVDQIAALNDSKTRKTTSETVRAVLDSLSEKKKSSP

SEQ ID NO: 64 - protein, 354 aa, synthetic construct
  REGION 1..354: note = Synthetic Polypeptide
MNTKYNKEFLLYLAGFVDGDGSIYARIFKGQHWKFKHHIRLTFHVSQKTQRRWFLDKLVDEIGVGYVTDWGSVSGYYLSEIKPLHNFLTQLQPFLKLKQKQANLVLKIIEQLPSAKESPDKFLEVCTWVDQIAALNDSKTRKTTSETVRAVLDSLPGSVGGLSPSQASSAASSASSSPGSGISEALRAGAGSGTGYNKEFLLYLAGFVDGDGSIWACIEPERGYRFKHRLRLAFTVAQKTQRRWFLDKLVDEIGVGYVVDQGSVSEYRLSEIKPLHNFLTQLQPFLKLKQKQANLVLKIIEQLPSAKESPDKFLEVCTWVDQIAALNDSKTRKTTSETVRAVLDSLSEKKKSSP

SEQ ID NO: 65 - protein, 354 aa, synthetic construct
  REGION 1..354: note = Synthetic Polypeptide
MNTKYNKEFLLYLAGFVDGDGSIYARIFKGQHWKFKHYIRLTFCVSQKTQRRWFLDKLVDEIGVGYVNDSGSCSNYYLSEIKPLHNFLTQLQPFLKLKQKQANLVLKIIEQLPSAKESPDKFLEVCTWVDQIAALNDSKTRKTTSETVRAVLDSLPGSVGGLSPSQASSAASSASSSPGSGISEALRAGAGSGTGYNKEFLLYLAGFVDGDGSIWARIEPELRLRFKHRLRLFFTVAQKTQRRWFLDKLVDEIGVGYVVDQGSVSEYRLSEIKPLHNFLTQLQPFLKLKQKQANLVLKIIEQLPSAKESPDKFLEVCTWVDQIAALNDSKTRKTTSETVRAVLDSLSEKKKSSP

SEQ ID NO: 66 - protein, 354 aa, synthetic construct
  REGION 1..354: note = Synthetic Polypeptide
MNTKYNKEFLLYLAGFVDGDGSIYARIFKGQHWKFKHYIRLTFCVSQKTQRRWFLDKLVDEIGVGYVNDSGSCSNYYLSEIKPLHNFLTQLQPFLKLKQKQANLVLKIIEQLPSAKESPDKFLEVCTWVDQIAALNDSKTRKTTSETVRAVLDSLPGSVGGLSPSQASSAASSASSSPGSGISEALRAGAGSGTGYNKEFLLYLAGFVDGDGSIWAQIVPERAGRFKHRLRLYFTVAQKTQRRWFLDKLVDEIGVGYVVDQGSVSEYRLSEIKPLHNFLTQLQPFLKLKQKQANLVLKIIEQLPSAKESPDKFLEVCTWVDQIAALNDSKTRKTTSETVRAVLDSLSEKKKSSP

SEQ ID NO: 67 - protein, 354 aa, synthetic construct
  REGION 1..354: note = Synthetic Polypeptide
MNTKYNKEFLLYLAGFVDGDGSIYARIFKGQHWKFKHHIRLTFNVSQKTQRRWFLDKLVDEIGVGYVCDSGSQSNYYLSEIKPLHNFLTQLQPFLKLKQKQANLVLKIIEQLPSAKESPDKFLEVCTWVDQIAALNDSKTRKTTSETVRAVLDSLPGSVGGLSPSQASSAASSASSSPGSGISEALRAGAGSGTGYNKEFLLYLAGFVDGDGSIWASITPEPTASFKHRLRLYFTVAQKTQRRWFLDKLVDEIGVGYVVDQGSVSEYRLSEIKPLHNFLTQLQPFLKLKQKQANLVLKIIEQLPSAKESPDKFLEVCTWVDQIAALNDSKTRKTTSETVRAVLDSLSEKKKSSP

SEQ ID NO: 68 - protein, 354 aa, synthetic construct
  REGION 1..354: note = Synthetic Polypeptide
MNTKYNKEFLLYLAGFVDGDGSIFARIFKGQHWKFKHHIRLTFCVSQKTQRRWFLDKLVDEIGVGYVVDNGSMSNYYLSEIKPLHNFLTQLQPFLKLKQKQANLVLKIIEQLPSAKESPDKFLEVCTWVDQIAALNDSKTRKTTSETVRAVLDSLPGSVGGLSPSQASSAASSASSSPGSGISEALRAGAGSGTGYNKEFLLYLAGFVDGDGSIWASINPEPSYRFKHRLRLSFTVAQKTQRRWFLDKLVDEIGVGYVVDQGSVSEYRLSEIKPLHNFLTQLQPFLKLKQKQANLVLKIIEQLPSAKESPDKFLEVCTWVDQIAALNDSKTRKTTSETVRAVLDSLSEKKKSSP

SEQ ID NO: 69 - protein, 354 aa, synthetic construct
  REGION 1..354: note = Synthetic Polypeptide
MNTKYNKEFLLYLAGFVDGDGSIYARIFKGQHWKFKHHIRLTFCVTQKTQRRWFLDKLVDEIGVGYVHDYGSCSNYYLSEIKPLHNFLTQLQPFLKLKQKQANLVLKIIEQLPSAKESPDKFLEVCTWVDQIAALNDSKTRKTTSETVRAVLDSLPGSVGGLSPSQASSAASSASSSPGSGISEALRAGAGSGTGYNKEFLLYLAGFVDGDGSIWASILPEHQYRFKHRLRLGFTVAQKTQRRWFLDKLVDEIGVGYVVDQGSVSEYRLSEIKPLHNFLTQLQPFLKLKQKQANLVLKIIEQLPSAKESPDKFLEVCTWVDQIAALNDSKTRKTTSETVRAVLDSLSEKKKSSP

SEQ ID NO: 70 - protein, 354 aa, synthetic construct
  REGION 1..354: note = Synthetic Polypeptide
MNTKYNKEFLLYLAGFVDGDGSIYAAIDPDQKYKFKHRLRLIFAVCQKTQRRWFLDKLVDEIGVGYVVDHGSVSEYRLSQIKPLHNFLTQLQPFLKLKQKQANLVLKIIEQLPSAKESPDKFLEVCTWVDQIAALNDSKTRKTTSETVRAVLDSLPGSVGGLSPSQASSAASSASSSPGSGISEALRAGAGSGTGYNKEFLLYLAGFVDGDGSIYARIEPRQTAKFKHYLRLTFHVSQKTQRRWFLDKLVDEIGVGYVVDQGSVSQYFLSEIKPLHNFLTQLQPFLKLKQKQANLVLKIIEQLPSAKESPDKFLEVCTWVDQIAALNDSKTRKTTSETVRAVLDSLSEKKKSSP

SEQ ID NO: 71 - protein, 354 aa, synthetic construct
  REGION 1..354: note = Synthetic Polypeptide
MNTKYNKEFLLYLAGFVDGDGSIYATIEPAQRYKFKHRLRLKFAVSQKTQRRWFLDKLVDEIGVGYVADQGSVSEYRLSEIKPLHNFLTQLQPFLKLKQKQANLVLKIIEQLPSAKESPDKFLEVCTWVDQIAALNDSKTRKTTSETVRAVLDSLPGSVGGLSPSQASSAASSASSSPGSGISEALRAGAGSGTGYNKEFLLYLAGFVDGDGSIYARIEPRQTAKFKHYLRLTFHVSQKTQRRWFLDKLVDEIGVGYVVDQGSVSQYFLSEIKPLHNFLTQLQPFLKLKQKQANLVLKIIEQLPSAKESPDKFLEVCTWVDQIAALNDSKTRKTTSETVRAVLDSLSEKKKSSP

SEQ ID NO: 72 - protein, 354 aa, synthetic construct
  REGION 1..354: note = Synthetic Polypeptide
MNTKYNKEFLLYLAGFVDGDGSIYATINPDQTNKFKHRLRLWFAVCQKTQRRWFLDKLVDEIGVGYVADTGSVSEYRLSQIKPLHNFLTQLQPFLKLKQKQANLVLKIIEQLPSAKESPDKFLEVCTWVDQIAALNDSKTRKTTSETVRAVLDSLPGSVGGLSPSQASSAASSASSSPGSGISEALRAGAGSGTGYNKEFLLYLAGFVDGDGSIYARIEPRQTAKFKHYLRLTFHVSQKTQRRWFLDKLVDEIGVGYVVDQGSVSQYFLSEIKPLHNFLTQLQPFLKLKQKQANLVLKIIEQLPSAKESPDKFLEVCTWVDQIAALNDSKTRKTTSETVRAVLDSLSEKKKSSP

SEQ ID NO: 73 - protein, 354 aa, synthetic construct
  REGION 1..354: note = Synthetic Polypeptide
MNTKYNKEFLLYLAGFVDGDGSIYACIEPAQNSKFKHYLRLRFEVSQKTQRRWFLDKLVDEIGVGYVYDQGSVSSYRLSQIKPLHNFLTQLQPFLKLKQKQANLVLKIIEQLPSAKESPDKFLEVCTWVDQIAALNDSKTRKTTSETVRAVLDSLPGSVGGLSPSQASSAASSASSSPGSGISEALRAGAGSGTGYNKEFLLYLAGFVDGDGSIYARIEPRQTAKFKHYLRLTFHVSQKTQRRWFLDKLVDEIGVGYVVDQGSVSQYFLSEIKPLHNFLTQLQPFLKLKQKQANLVLKIIEQLPSAKESPDKFLEVCTWVDQIAALNDSKTRKTTSETVRAVLDSLSEKKKSSP

SEQ ID NO: 74 - protein, 354 aa, synthetic construct
  REGION 1..354: note = Synthetic Polypeptide
MNTKYNKEFLLYLAGFVDGDGSIYASITPCQSYKFKHRLLLKFSVAQKTQRRWFLDKLVDEIGVGYVTDSGSVSEYRLSQIKPLHNFLTQLQPFLKLKQKQANLVLKIIEQLPSAKESPDKFLEVCTWVDQIAALNDSKTRKTTSETVRAVLDSLPGSVGGLSPSQASSAASSASSSPGSGISEALRAGAGSGTGYNKEFLLYLAGFVDGDGSIYARIEPRQTAKFKHYLRLTFHVSQKTQRRWFLDKLVDEIGVGYVVDQGSVSQYFLSQIKPLHNFLTQLQPFLKLKQKQANLVLKIIEQLPSAKESPDKFLEVCTWVDQIAALNDSKTRKTTSETVRAVLDSLSEKKKSSP

SEQ ID NO: 75 - protein, 354 aa, synthetic construct
  REGION 1..354: note = Synthetic Polypeptide
MNTKYNKEFLLYLAGFVDGDGSIYATIMPEQTVKFKHRLRLFFEVAQKTQRRWFLDKLVDEIGVGYVYDQGSVSSYRLSQIKPLHNFLTQLQPFLKLKQKQANLVLKIIEQLPSAKESPDKFLEVCTWVDQIAALNDSKTRKTTSETVRAVLDSLPGSVGGLSPSQASSAASSASSSPGSGISEALRAGAGSGTGYNKEFLLYLAGFVDGDGSIYARIEPRQTAKFKHYLRLTFHVSQKTQRRWFLDKLVDEIGVGYVVDQGSVSQYFLSQIKPLHNFLTQLQPFLKLKQKQANLVLKIIEQLPSAKESPDKFLEVCTWVDQIAALNDSKTRKTTSETVRAVLDSLSEKKKSSP

SEQ ID NO: 76 - protein, 354 aa, synthetic construct
  REGION 1..354: note = Synthetic Polypeptide
MNTKYNKEFLLYLAGFVDGDGSIYATIQPEQAPKFKHRLRLHFTVHQKTQRRWFLDKLVDEIGVGYVYDQGSVSEYRLSQIKPLHNFLTQLQPFLKLKQKQANLVLKIIEQLPSAKESPDKFLEVCTWVDQIAALNDSKTRKTTSETVRAVLDSLPGSVGGLSPSQASSAASSASSSPGSGISEALRAGAGSGTGYNKEFLLYLAGFVDGDGSIYARIEPRQTAKFKHYLRLTFHVSQKTQRRWFLDKLVDEIGVGYVVDQGSVSQYFLSQIKPLHNFLTQLQPFLKLKQKQANLVLKIIEQLPSAKESPDKFLEVCTWVDQIAALNDSKTRKTTSETVRAVLDSLSEKKKSSP

SEQ ID NO: 77 - protein, 354 aa, synthetic construct
  REGION 1..354: note = Synthetic Polypeptide
MNTKYNKEFLLYLAGFVDGDGSIWATIEPSQTLKFKHRLRLHFSVYQKTQRRWFLDKLVDEIGVGYVYDDGSVSRYQLSQIKPLHNFLTQLQPFLKLKQKQANLVLKIIEQLPSAKESPDKFLEVCTWVDQIAALNDSKTRKTTSETVRAVLDSLPGSVGGLSPSQASSAASSASSSPGSGISEALRAGAGSGTGYNKEFLLYLAGFVDGDGSIYARIEPRQTAKFKHYLRLTFHVSQKTQRRWFLDKLVDEIGVGYVVDQGSVSQYFLSQIKPLHNFLTQLQPFLKLKQKQANLVLKIIEQLPSAKESPDKFLEVCTWVDQIAALNDSKTRKTTSETVRAVLDSLSEKKKSSP

SEQ ID NO: 78 - protein, 354 aa, synthetic construct
  REGION 1..354: note = Synthetic Polypeptide
MNTKYNKEFLLYLAGFVDGDGSIYASITPCQSYKFKHRLLLKFSVAQKTQRRWFLDKLVDEIGVGYVTDSGSVSEYRLSEIKPLHNFLTQLQPFLKLKQKQANLVLKIIEQLPSAKESPDKFLEVCTWVDQIAALNDSKTRKTTSETVRAVLDSLPGSVGGLSPSQASSAASSASSSPGSGISEALRAGAGSGTGYNKEFLLYLAGFVDGDGSIYARIEPRQTAKFKHYLRLTFHVSQKTQRRWFLDKLVDEIGVGYVVDQGSVSQYFLSQIKPLHNFLTQLQPFLKLKQKQANLVLKIIEQLPSAKESPDKFLEVCTWVDQIAALNDSKTRKTTSETVRAVLDSLSEKKKSSP

SEQ ID NO: 79 - protein, 354 aa, synthetic construct
  REGION 1..354: note = Synthetic Polypeptide
MNTKYNKEFLLYLAGFVDGDGSIYATIIPSQNLKFKHRLRLYFEVCQKTQRRWFLDKLVDEIGVGYVYDQGSVSSYRLSEIKPLHNFLTQLQPFLKLKQKQANLVLKIIEQLPSAKESPDKFLEVCTWVDQIAALNDSKTRKTTSETVRAVLDSLPGSVGGLSPSQASSAASSASSSPGSGISEALRAGAGSGTGYNKEFLLYLAGFVDGDGSIYARIEPRQTAKFKHYLRLTFHVSQKTQRRWFLDKLVDEIGVGYVVDQGSVSQYFLSQIKPLHNFLTQLQPFLKLKQKQANLVLKIIEQLPSAKESPDKFLEVCTWVDQIAALNDSKTRKTTSETVRAVLDSLSEKKKSSP

SEQ ID NO: 80 - protein, 354 aa, synthetic construct
  REGION 1..354: note = Synthetic Polypeptide
MNTKYNKEFLLYLAGFVDGDGSIYASICPTQAAKFKHRLRLHFAVFQKTQRRWFLDKLVDEIGVGYVTDCGSVSEYRLSQIKPLHNFLTQLQPFLKLKQKQANLVLKIIEQLPSAKESPDKFLEVCTWVDQIAALNDSKTRKTTSETVRAVLDSLPGSVGGLSPSQASSAASSASSSPGSGISEALRAGAGSGTGYNKEFLLYLAGFVDGDGSIYARIEPRQTAKFKHYLRLTFHVSQKTQRRWFLDKLVDEIGVGYVVDQGSVSQYFLSQIKPLHNFLTQLQPFLKLKQKQANLVLKIIEQLPSAKESPDKFLEVCTWVDQIAALNDSKTRKTTSETVRAVLDSLSEKKKSSP

SEQ ID NO: 81 - protein, 354 aa, synthetic construct
  REGION 1..354: note = Synthetic Polypeptide
MNTKYNKEFLLYLAGFVDGDGSIYASIEPAQSYKFKHRLQLKFAVAQKTQRRWFLDKLVDEIGVGYVCDIGSVSEYRLSQIKPLHNFLTQLQPFLKLKQKQANLVLKIIEQLPSAKESPDKFLEVCTWVDQIAALNDSKTRKTTSETVRAVLDSLPGSVGGLSPSQASSAASSASSSPGSGISEALRAGAGSGTGYNKEFLLYLAGFVDGDGSIYARIEPRQTAKFKHYLRLTFHVSQKTQRRWFLDKLVDEIGVGYVVDQGSVSQYFLSQIKPLHNFLTQLQPFLKLKQKQANLVLKIIEQLPSAKESPDKFLEVCTWVDQIAALNDSKTRKTTSETVRAVLDSLSEKKKSSP

SEQ ID NO: 82 - protein, 354 aa, synthetic construct
  REGION 1..354: note = Synthetic Polypeptide
MNTKYNKEFLLYLAGFVDGDGSIYAAIMPTQSYKFKHRLRLAFSVSQKTQRRWFLDKLVDEIGVGYVTDAGSVSEYRLSQIKPLHNFLTQLQPFLKLKQKQANLVLKIIEQLPSAKESPDKFLEVCTWVDQIAALNDSKTRKTTSETVRAVLDSLPGSVGGLSPSQASSAASSASSSPGSGISEALRAGAGSGTGYNKEFLLYLAGFVDGDGSIYARIEPRQTAKFKHYLRLTFHVSQKTQRRWFLDKLVDEIGVGYVVDQGSVSQYFLSQIKPLHNFLTQLQPFLKLKQKQANLVLKIIEQLPSAKESPDKFLEVCTWVDQIAALNDSKTRKTTSETVRAVLDSLSEKKKSSP

SEQ ID NO: 83 - protein, 354 aa, synthetic construct
  REGION 1..354: note = Synthetic Polypeptide
MNTKYNKEFLLYLAGFVDGDGSIYATITPNQRTKFKHQLKLAFAVYQKTQRRWFLDKLVDEIGVGYVYDQGSVSCYRLSEIKPLHNFLTQLQPFLKLKQKQANLVLKIIEQLPSAKESPDKFLEVCTWVDQIAALNDSKTRKTTSETVRAVLDSLPGSVGGLSPSQASSAASSASSSPGSGISEALRAGAGSGTGYNKEFLLYLAGFVDGDGSIYARIEPRQTAKFKHYLRLTFHVSQKTQRRWFLDKLVDEIGVGYVVDQGSVSQYFLSQIKPLHNFLTQLQPFLKLKQKQANLVLKIIEQLPSAKESPDKFLEVCTWVDQIAALNDSKTRKTTSETVRAVLDSLSEKKKSSP

SEQ ID NO: 84 - protein, 354 aa, synthetic construct
  REGION 1..354: note = Synthetic Polypeptide
MNTKYNKEFLLYLAGFVDGDGSIYAAIVPVQSTKFKHRLRLYFTVHQKTQRRWFLDKLVDEIGVGYVYDQGSVSEYRLSQIKPLHNFLTQLQPFLKLKQKQANLVLKIIEQLPSAKESPDKFLEVCTWVDQIAALNDSKTRKTTSETVRAVLDSLPGSVGGLSPSQASSAASSASSSPGSGISEALRAGAGSGTGYNKEFLLYLAGFVDGDGSIYARIEPRQTAKFKHYLRLTFHVSQKTQRRWFLDKLVDEIGVGYVVDQGSVSQYFLSQIKPLHNFLTQLQPFLKLKQKQANLVLKIIEQLPSAKESPDKFLEVCTWVDQIAALNDSKTRKTTSETVRAVLDSLSEKKKSSP

SEQ ID NO: 85 - protein, 354 aa, synthetic construct
  REGION 1..354: note = Synthetic Polypeptide
MNTKYNKEFLLYLAGFVDGDGSIYATICPVQSLKFKHRLRLFFAVCQKTQRRWFLDKLVDEIGVGYVVDHGSVSEYRLSEIKPLHNFLTQLQPFLKLKQKQANLVLKIIEQLPSAKESPDKFLEVCTWVDQIAALNDSKTRKTTSETVRAVLDSLPGSVGGLSPSQASSAASSASSSPGSGVSEALRAGAGSGTGYNKEFLLYLAGFVDGDGSIYARIEPRQTAKFKHYLRLTFHVSQKTQRRWFLDKLVDEIGVGYVVDQGSVSQYFLSQIKPLHNFLTQLQPFLKLKQKQANLVLKIIEQLPSAKESPDKFLEVCTWVDQIAALNDSKTRKTTSETVRAVLDSLSEKKKSSP

SEQ ID NO: 86 - protein, 354 aa, synthetic construct
  REGION 1..354: note = Synthetic Polypeptide
MNTKYNKEFLLYLAGFVDGDGSIWASILPEQRNKFKHRLKLGFSVSQKTQRRWFLDKLVDEIGVGYVVDQGSVSEYRLSQIKPLHNFLTQLQPFLKLKQKQANLVLKIIEQLPSAKESPDKFLEVCTWVDQIAALNDSKTRKTTSETVRAVLDSLPGSVGGLSPSQASSAASSASSSPGSGISEALRAGAGSGTGYNKEFLLYLAGFVDGDGSIYARIEPRQTAKFKHYLRLTFHVSQKTQRRWFLDKLVDEIGVGYVVDQGSVSQYFLSQIKPLHNFLTQLQPFLKLKQKQANLVLKIIEQLPSAKESPDKFLEVCTWVDQIAALNDSKTRKTTSETVRAVLDSLSEKKKSSP

SEQ ID NO: 87 - protein, 354 aa, synthetic construct
  REGION 1..354: note = Synthetic Polypeptide
MNTKYNKEFLLYLAGFVDGDGSIYATIHPCQCTKFKHRLRLYFEVYQKTQRRWFLDKLVDEIGVGYVYDQGSVSSYRLSQIKPLHNFLTQLQPFLKLKQKQANLVLKIIEQLPSAKESPDKFLEVCTWVDQIAALNDSKTRKTTSETVRAVLDSLPGSVGGLSPSQASSAASSASSSPGSGISEALRAGAGSGTGYNKEFLLYLAGFVDGDGSIYARIEPRQTAKFKHYLRLTFHVSQKTQRRWFLDKLVDEIGVGYVTDWGSVSGYYLSEIKPLHNFLTQLQPFLKLKQKQANLVLKIIEQLPSAKESPDKFLEVCTWVDQIAALNDSKTRKTTSETVRAVLDSLSEKKKSSP

SEQ ID NO: 88 - protein, 354 aa, synthetic construct
  REGION 1..354: note = Synthetic Polypeptide
MNTKYNKEFLLYLAGFVDGDGSIYATIDPDQRQKFKHRLRLKFSVSQKTQRRWFLDKLVDEIGVGYVVDGGSVSEYRLSEIKPLHNFLTQLQPFLKLKQKQANLVLKIIEQLPSAKESPDKFLEVCTWVDQIAALNDSKTRKTTSETVRAVLDSLPGSVGGLSPSQASSAASSASSSPGSGISEALRAGAGSGTGYNKEFLLYLAGFVDGDGSIYACIEPKQTSKFKHRLCLRFHVSQKTQRRWFLDKLVDEIGVGYVHDNGSVSQYYLSEIKPLHNFLTQLQPFLKLKQKQANLVLKIIEQLPSAKESPDKFLEVCTWVDQIAALNDSKTRKTTSETVRAVLDSLSEKKKSSP

SEQ ID NO: 89 - protein, 354 aa, synthetic construct
  REGION 1..354: note = Synthetic Polypeptide
MNTKYNKEFLLYLAGFVDGDGSIYAAIVPDQAPKFKHRLRLFFAVSQKTQRRWFLDKLVDEIGVGYVADQGSVSEYRLSQIKPLHNFLTQLQPFLKLKQKQANLVLKIIEQLPSAKESPDKFLEVCTWVDQIAALNDSKTRKTTSETVRAVLDSLPGSVGGLSPSQASSAASSASSSPGSGISEALRAGAGSGTGYNKEFLLYLAGFVDGDGSIYARIYPGQHYKFKHYLRLTFHVSQKTQRRWFLDKLVDEIGVGYVTDAGSVSQYFLSQIKPLHNFLTQLQPFLKLKQKQANLVLKIIEQLPSAKESPDKFLEVCTWVDQIAALNDSKTRKTTSETVRAVLDSLSEKKKSSP

SEQ ID NO: 90 - protein, 354 aa, synthetic construct
  REGION 1..354: note = Synthetic Polypeptide
MNTKYNKEFLLYLAGFVDGDGSIYASILPEQRNKFKHRLKLSFSVCQKTQRRWFLDKLVDEIGVGYVVDQGSVSEYRLSEIKPLHNFLTQLQPFLKLKQKQANLVLKIIEQLPSAKESPDKFLEVCTWVDQIAALNDSKTRKTTSETVRAVLDSLPGSVGGLSPSQASSAASSASSSPGSGISEALRAGAGSGTGYNKEFLLYLAGFVDGDGSIYARIEPRQTAKFKHYLRLTFHVSQKTQRRWFLDKLVDEIGVGYVIDAGSVSGYYLSEIKPLHNFLTQLQPFLKLKQKQANLVLKIIEQLPSAKESPDKFLEVCTWVDQIAALNDSKTRKTTSETVRAVLDSLSEKKKSSP

SEQ ID NO: 91 - protein, 354 aa, synthetic construct
  REGION 1..354: note = Synthetic Polypeptide
MNTKYNKEFLLYLAGFVDGDGSIYAAIVPDQAPKFKHRLRLFFAVSQKTQRRWFLDKLVDEIGVGYVADQGSVSEYRLSEIKPLHNFLTQLQPFLKLKQKQANLVLKIIEQLPSAKESPDKFLEVCTWVDQIAALNDSKTRKTTSETVRAVLDSLPGSVGGLSPSQASSAASSASSSPGSGISEALRAGAGSGTGYNKEFLLYLAGFVDGDGSIYACIEPKQTSKFKHRLCLRFHVSQKTQRRWFLDKLVDEIGVGYVHDNGSVSQYYLSQIKPLHNFLTQLQPFLKLKQKQANLVLKIIEQLPSAKESPDKFLEVCTWVDQIAALNDSKTRKTTSETVRAVLDSLSEKKKSSP

SEQ ID NO: 92 - protein, 354 aa, synthetic construct
  REGION 1..354: note = Synthetic Polypeptide
MNTKYNKEFLLYLAGFVDGDGSIYACICPDQGYKFKHRLTLKFSVAQKTQRRWFLDKLVDEIGVGYVLDQGSVSEYRLSEIKPLHNFLTQLQPFLKLKQKQANLVLKIIEQLPSAKESPDKFLEVCTWVDQIAALNDSKTRKTTSETVRAVLDSLPGSVGGLSPSQASSAASSASSSPGSGISEALRAGAGSGTGYNKEFLLYLAGFVDGDGSIYARIEPRQTAKFKHQLRLTFHVSQKTQRRWFLDKLVDEIGVGYVTDWGSVSGYYLSQIKPLHNFLTQLQPFLKLKQKQANLVLKIIEQLPSAKESPDKFLEVCTWVDQIAALNDSKTRKTTSETVRAVLDSLSEKKKSSP

SEQ ID NO: 93 - protein, 354 aa, synthetic construct
  REGION 1..354: note = Synthetic Polypeptide
MNTKYNKEFLLYLAGFVDGDGSIYACILPEQKTKFKHRLKLSFTVCQKTQRRWFLDKLVDEIGVGYVVDQGSVSEYRLSQIKPLHNFLTQLQPFLKLKQKQANLVLKIIEQLPSAKESPDKFLEVCTWVDQIAALNDSKTRKTTSETVRAVLDSLPGSVGGLSPSQASSAASSASSSPGSGISEALRAGAGSGTGYNKEFLLYLAGFVDGDGSIYARIEPRQTVKFKHMLRLTFHVSQKTQRRWFLDKLVDEIGVGYVHDNGSVSQYYLSQIKPLHNFLTQLQPFLKLKQKQANLVLKIIEQLPSAKESPDKFLEVCTWVDQIAALNDSKTRKTTSETVRAVLDSLSEKKKSSP

SEQ ID NO: 94 - protein, 163 aa, synthetic construct
  REGION 1..163: note = Synthetic Polypeptide
MNTKYNKEFLLYLAGFVDGDGSIIAQIKPNQSYKFKHQLSLAFQVTQKTQRRWFLDKLVDEIGVGYVRDRGSVSDYILSEIKPLHNFLTQLQPFLKLKQKQANLVLKIIWRLPSAKESPDKFLEVCTWVDQIAALNDSKTRKTTSETVRAVLDSLSEKKKSSP

SEQ ID NO: 95 - protein, 9 aa, synthetic construct
  REGION 1..9: note = Synthetic Polypeptide
LAGLIDADG

SEQ ID NO: 96 - DNA, 1047 bp, synthetic construct
  misc_feature 1..1047: note = Synthetic Polynucleotide
  source 1..1047: mol_type = other DNA
atgaatggcacagaaggccctaacttctacgtgcccttctccaatgcgacgggtgtggtacgcagccccttcgagtacccacagtactacctggctgagccatggcagttctccatgctggccgcctacatgtttctgctgatcgtgctgggcttccccatcaacttcctcacgctctacgtcaccgtccagcacaagaagctgcgcacgcctctcaactacatcctgctcaacctagccgtggctgacctcttcatggtcctaggtggcttcaccagcaccctctacacctctctgcatggatacttcgtcttcgggcccacaggatgcaatttggagggcttctttgccaccctgggcggtgaaattgccctgtggtccttggtggtcctggccatcgagcggtacgtggtggtgtgtaagcccatgagcaacttccgcttcggggagaaccatgccatcatgggcgttgccttcacctgggtcatggcgctggcctgcgccgcacccccactcgccggctggtccaggtacatccccgagggcctgcagtgctcgtgtggaatcgactactacacgctcaagccggaggtcaacaacgagtcttttgtcatctacatgttcgtggtccacttcaccatccccatgattatcatctttttctgctatgggcagctcgtcttcaccgtcaaggaggccgctgcccagcagcaggagtcagccaccacacagaaggcagagaaggaggtcacccgcatggtcatcatcatggtcatcgctttcctgatctgctgggtgccctacgccagcgtggcattctacatcttcacccaccagggctccaacttcggtcccatcttcatgaccatcccagcgttctttgccaagagcgccgccatctacaaccctgtcatctatatcatgatgaacaagcagttccggaactgcatgctcaccaccatctgctgcggcaagaacccactgggtgacgatgaggcctctgctaccgtgtccaagacggagacgagccaggtggccccggcctaa

SEQ ID NO: 97 - DNA, 1047 bp, synthetic construct
  misc_feature 1..1047: note = Synthetic Polynucleotide
  source 1..1047: mol_type = other DNA
atgaatggcacagaaggccctaacttctacgtgcccttctccaatgcgacgggtgtggtacgcagccacttcgagtacccacagtactacctggctgagccatggcagttctccatgctggccgcctacatgtttctgctgatcgtgctgggcttccccatcaacttcctcacgctctacgtcaccgtccagcacaagaagctgcgcacgcctctcaactacatcctgctcaacctagccgtggctgacctcttcatggtcctaggtggcttcaccagcaccctctacacctctctgcatggatacttcgtcttcgggcccacaggatgcaatttggagggcttctttgccaccctgggcggtgaaattgccctgtggtccttggtggtcctggccatcgagcggtacgtggtggtgtgtaagcccatgagcaacttccgcttcggggagaaccatgccatcatgggcgttgccttcacctgggtcatggcgctggcctgcgccgcacccccactcgccggctggtccaggtacatccccgagggcctgcagtgctcgtgtggaatcgactactacacgctcaagccggaggtcaacaacgagtcttttgtcatctacatgttcgtggtccacttcaccatccccatgattatcatctttttctgctatgggcagctcgtcttcaccgtcaaggaggccgctgcccagcagcaggagtcagccaccacacagaaggcagagaaggaggtcacccgcatggtcatcatcatggtcatcgctttcctgatctgctgggtgccctacgccagcgtggcattctacatcttcacccaccagggctccaacttcggtcccatcttcatgaccatcccagcgttctttgccaagagcgccgccatctacaaccctgtcatctatatcatgatgaacaagcagttccggaactgcatgctcaccaccatctgctgcggcaagaacccactgggtgacgatgaggcctctgctaccgtgtccaagacggagacgagccaggtggccccggcctaa

SEQ ID NO: 98 - DNA, 13706 bp, synthetic construct
  misc_feature 1..13706: note = Synthetic Polynucleotide
  source 1..13706: mol_type = other DNA
gtgggggaccaggagaaagaaagccaaggaagaggaggaggaggaggagaaggaggagaaggatgctgacctagcagctcctctcacagcagctcctctcttgcagaggctgaagagcgatttgtgccctgcaagctaagcccctaatccaccgaggcaaaggcaaagcccctagccgggctcccgagggctgggactcgggtgccccaagatggctgcatccagccatcttggcttagaaagccccccacatgccagcttggccaacacccacaccatgggtttctctggactgcccgacacaaggtgtgggtgctggccaggcctgtgttcaaatcccagctctgcagaggaactttgaccctgcataccccagattcctcagtggtcagtggggagttagaccctcttcatagggggcaggaggagttgttcattcattcaacaaatgtttattgaacacctcctatgggttgtgagctcagaggcagcgatgaacaggccaggctggtcctgcattctagaaatagatgggaagtcagtcaataagtagacaaatgaggccaggtgtggtggcatgcctgtagacccagttactcgggatgctgaggtaggaggatcacttgagcctaggacaggaattcaaggctgcagtaagctatgattgcgccactgcactccagcctgggcaacagagcaagactcatctctaaaaaacatttaaaaattgttttaagaagacaaatgagatagtcgctgatggtaatgactgtgtaaaaactgaacatggctgggtgtggttgctcacacctataatctcagcactttgggaggctgagattacagcctcccaagtggctcccaaggcaggaggatcacttgagcctgggagttagagaacagcttggacaatatagggagagcccaactctacaaaaatgaaaataaattagccaggcatggtggcacacaccaatggtcccagctactcaggggttgaggtggtggaccgcttgagcccaggaggttgaggctgcagtgagccatgatcatgccgctgcactccaacctgagtcacagagtgataccctgtctcaaaaaacaataggccaggtgtggtggctcacgcctgtaaccccagcactttgggaggccgaggcggatggatcacttgagatcaggagttagagaccagcctggctaacatggcaaaatcctgtctgtactaaaaatataaaaattagccaggcatggcagtacatgcctgtagtcctggttacttgggaggctaaggcaggagaatcgcttgaacccaggaagaggaggttgcagtgagccaagatcacaccactgcactccagcttgggtgacagagtgagaccctgtctcaaaacagctaaacctggtgggggtgcctggtgtgtaggatggtcaggggtggtctctccaaggacatgagtgtgagcggagacctgaaggagactcaggaagagattaatactgtcagcaacaaatatattgatcacttacaagcactcccaataatcctattaggtaggcactattatcattcccattttacagagtggagaaccgaagcacactctcgggagggcggggtagctggctgcacccaggctgtgtagcctcagtccagatgtaagggtgggtggaaaagagccttgcccaatgagggagaacagtgaaaccaaggccatagggtctaaagattcacgaaccaggctctcatggagaaagcaggtgaggtttactgtatagatgggtgtgcccctaccccacactgaggcttcctcgtctgagcaaactgaggcccagagaggggaaggaagcaggactaccatggtgactcaaagaccagctagaatccagcctcctctcctcgaggcttccactgccccacgccaggcctgtgtgactcagtctagggcctttccattaccccagctaaacctttctttagtcatttataccatggtgtgaatggctggctggtctttcctgagagctatctttgatgaggggagggaggcatagccaggtttgggaagctgataccccaggaagcccagttgactgtgtgggttatagcccaggctgtcactgatttgtaacgggacctgagcaactctgcagagctaggcctcagtcttttcatctgcaaaatggatatagcagagatggtcagagtaggtgacttcgaatgacccttccagctcactatgagtctgttttcctgaacaaagagcattttttgtttaaaaaaaaatttcttgggccggacacggtggttcactcctataatcctggcactttgggaggccgaggagggtggatcgcttgagccaggagttcaggaccagcctgggcaacatagcgagactccacccctacaaaaaatacaaaaactagtggtgtgcacttgtggtcccagctactcaggaggctgaggtgagaggatcgcttgagcccaggaggcagaggctacagtgagctatgattgtggcactgcactccagcctgggcgacagagaccttgtctcaaaactttttttttcttcgtcaagctttacagaataaagagcactgtcacctcagtgatggctgttagttccccatcaccagggctccatgaggttgcaattgtgaaactcacaaaggaggaacctgagacagagaggggaagtactgagatcatctaggtccattcccccactcactcgttcattcaacaaatattcaggagcaccttctaggtgccaggccctggagacacatcagtgaacaaaacagacatcatcccacctctttccactacaggccaagcaccatgctggtctctgggaaccctgttgtgagcaagacagacccaggcttacccttgtggactcatgttacaggcagggagacgggcacaaaacacaaataaaaagcttccatgctgtcagaagcactatgcaaaaagcaagatgctgaggtactgctaagctgtgtgggatgggggctcagcccggccagggaggggccagttgtgggtcagtcttgacccaaggcatccaggacaccctccttctggccatgagggtccacgtcagaatcaaaccctcaccttaacctcattagcgttgggcataatcaccaggccaagcgccttaaactacgagaggccccatcccacccgccctgccttagccctgccacgtgtgccaaacgctgttagacccaacaccacccaggccaggtagggggctggagcccaggtgggctgcagggaagggggcactcttctgagcagacagatctgggaatcctgggtgggaagagagacagtgagagagagattaagggatatttcccaggcatcagggctttgcactctcaggggtccttccgcctggatgtccttcccctgaagcttcctcctgttgttccgttctcagctcaagctccagcttctcagagaagcctcctgtgttgggagtggctgcgactgaactgtccctactgttattcgctcttctatttgtttgtggtccctgtgccccctcaccccacaaaaacactggcttcttgtgagcaggagcttgctctttcgtgtaccctgtgtgtccccaaggaccaagcaccttgtctgggccacagtaggtgctcaatacacatgttggctggacagtggtcactgagcggccgcacgtcgggcactctcagcacttgcacaggccgccccagacaccccacttcattcctgggaggtgtcatcatgttgcttggacgacggggagagggggacctgccagtgttggcctccattttcccccagtcatctgcccccaaggctctgactactttctttctcacggtacatcctgctattctggaatcggccctcgtggggccacctggtacatggcatttgaggccctcgtggctgattaggcctcccccaacagtgccctgtctgctgcctccagggccagcctccccttcagactggagtcccctgaagggttctgcccctcccctgctctggtagccccctccatcctccctccctccactccatctttgggggcatttgagtcacctttctacaccagtgatctgcccaagccactgctcactttcctctggataaagccaggttccccggcctagcgttcaagacccattacaactgcccccagcccagatcttccccacctagccacctggcaaactgctccttctctcaaaggcccaaacatggcctcccagactgcaacccccaggcagtcaggccctgtctccacaacctcacagccaccctggacggaatctgcttcttcccacatttgagtcctcctcagcccctgagctcctctgggcagggctgtttctttccatctttgtattcccaggggcctgcaaataaatgtttaatgaacgaacaagagagtgaattccaattccatgcaacaaggattgggctcctgggccctaggctatgtgtctggcaccagaaacggaagctgcaggttgcagcccctgccctcatggagctcctcctgtcagaggagtgtggggactggatgactccagaggtaacttgtgggggaacgaacaggtaaggggctgtgtgacgagatgagagactgggagaataaaccagaaagtctctagctgtccagaggacatagcacagaggcccatggtccctatttcaaacccaggccaccagactgagctgggaccttgggacagacaagtcatgcagaagttaggggaccttctcctcccttttcctggatcctgagtacctctcctccctgacctcaggcttcctcctagtgtcaccttggcccctcttagaagccaattaggccctcagtttctgcagcggggattaatatgattatgaacacccccaatctcccagatgctgattcagccaggagcttaggagggggaggtcactttataagggtctgggggggtcagaacccagagtcatccagctggagccctgagtggctgagctcaggccttcgcagcattcttgggtgggagcagccacgggtcagccacaagggccacagccatgaatggcacagaaggccctaacttctacgtgcccttctccaatgcgacgggtgtggtacgcagccccttcgagtacccacagtactacctggctgagccatggcagttctccatgctggccgcctacatgtttctgctgatcgtgctgggcttccccatcaacttcctcacgctctacgtcaccgtccagcacaagaagctgcgcacgcctctcaactacatcctgctcaacctagccgtggctgacctcttcatggtcctaggtggcttcaccagcaccctctacacctctctgcatggatacttcgtcttcgggcccacaggatgcaatttggagggcttctttgccaccctgggcggtatgagccgggtgtgggtggggtgtgcaggagcccgggagcatggaggggtctgggagagtcccgggcttggcggtggtggctgagaggccttctcccttctcctgtcctgtcaatgttatccaaagccctcatatattcagtcaacaaacaccattcatggtgatagccgggctgctgtttgtgcagggctggcactgaacactgccttgatcttatttggagcaatatgcgcttgtctaatttcacagcaagaaaactgagctgaggctcaaagaagtcaagcgccctgctggggcgtcacacagggacgggtgcagagttgagttggaagcccgcatctatctcgggccatgtttgcagcaccaagcctctgtttcccttggagcagctgtgctgagtcagacccaggctgggcactgagggagagctgggcaagccagacccctcctctctgggggcccaagctcagggtgggaagtggattttccattctccagtcattgggtcttccctgtgctgggcaatgggctcggtcccctctggcatcctctgcctcccctctcagcccctgtcctcaggtgcccctccagcctccctgccgcgttccaagtctcctggtgttgagaaccgcaagcagccgctctgaagcagttcctttttgctttagaataatgtcttgcatttaacaggaaaacagatggggtgctgcagggataacagatcccacttaacagagaggaaaactgaggcagggagaggggaagagactcatttagggatgtggccaggcagcaacaagagcctaggtctcctggctgtgatccaggaatatctctgctgagatgcaggaggagacgctagaagcagccattgcaaagctgggtgacggggagagcttaccgccagccacaagcgtctctctgccagccttgccctgtctcccccatgtccaggctgctgcctcggtcccattctcagggaatctctggccattgttgggtgtttgttgcattcaataatcacagatcactcagttctggccagaaggtgggtgtgccacttacgggtggttgttctctgcagggtcagtcccagtttacaaatattgtccctttcactgttaggaatgtcccagtttggttgattaactatatggccactctccctatggaacttcatggggtggtgagcaggacagatgtctgaattccatcatttccttcttcttcctctgggcaaaacattgcacattgcttcatggctcctaggagaggcccccacatgtccgggttatttcatttcccgagaagggagagggaggaaggactgccaattctgggtttccaccacctctgcattccttcccaacaaggaactctgccccacattaggatgcattcttctgctaaacacacacacacacacacacacacacaacacacacacacacacacacacacacacacacacaaaactccctaccgggttcccagttcaatcctgaccccctgatctgattcgtgtcccttatgggcccagagcgctaagcaaataacttcccccattccctggaatttctttgcccagctctcctcagcgtgtggtccctctgccccttccccctcctcccagcaccaagctctctccttccccaaggcctcctcaaatccctctcccactcctggttgccttcctagctaccctctccctgtctaggggggagtgcaccctccttaggcagtggggtctgtgctgaccgcctgctgactgccttgcaggtgaaattgccctgtggtccttggtggtcctggccatcgagcggtacgtggtggtgtgtaagcccatgagcaacttccgcttcggggagaaccatgccatcatgggcgttgccttcacctgggtcatggcgctggcctgcgccgcacccccactcgccggctggtccaggtaatggcactgagcagaagggaagaagctccgggggctctttgtagggtcctccagtcaggactcaaacccagtagtgtctggttccaggcactgaccttgtatgtctcctggcccaaatgcccactcagggtaggggtgtagggcagaagaagaaacagactctaatgttgctacaagggctggtcccatctcctgagccccatgtcaaacagaatccaagacatcccaacccttcaccttggctgtgcccctaatcctcaactaagctaggcgcaaattccaatcctctttggtctagtaccccgggggcagccccctctaaccttgggcctcagcagcaggggaggccacaccttcctagtgcaggtggccatattgtggccccttggaactgggtcccactcagcctctaggcgattgtctcctaatggggctgagatgagacacagtggggacagtggtttggacaataggactggtgactctggtccccagaggcctcatgtccctctgtctccagaaaattcccactctcacttccctttcctcctcagtcttgctagggtccatttcttaccccttgctgaatttgagcccaccccctggactttttccccatcttctccaatctggcctagttctatcctctggaagcagagccgctggacgctctgggtttcctgaggcccgtccactgtcaccaatatcaggaaccattgccacgtcctaatgacgtgcgctggaagcctctagtttccagaagctgcacaaagatcccttagatactctgtgtgtccatctttggcctggaaaatactctcaccctggggctaggaagacctcggtttgtacaaacttcctcaaatgcagagcctgagggctctccccacctcctcaccaaccctctgcgtggcatagccctagcctcagcgggcagtggatgctggggctgggcatgcagggagaggctgggtggtgtcatctggtaacgcagccaccaaacaatgaagcgacactgattccacaaggtgcatctgcatccccatctgatccattccatcctgtcacccagccatgcagacgtttatgatccccttttccagggagggaatgtgaagccccagaaagggccagcgctcggcagccaccttggctgttcccaagtccctcacaggcagggtctccctacctgcctgtcctcaggtacatccccgagggcctgcagtgctcgtgtggaatcgactactacacgctcaagccggaggtcaacaacgagtcttttgtcatctacatgttcgtggtccacttcaccatccccatgattatcatctttttctgctatgggcagctcgtcttcaccgtcaaggaggtacgggccggggggtgggcggcctcacggctctgagggtccagcccccagcatgcatctgcggctcctgctccctggaggagccatggtctggacccgggtcccgtgtcctgcaggccgctgcccagcagcaggagtcagccaccacacagaaggcagagaaggaggtcacccgcatggtcatcatcatggtcatcgctttcctgatctgctgggtgccctacgccagcgtggcattctacatcttcacccaccagggctccaacttcggtcccatcttcatgaccatcccagcgttctttgccaagagcgccgccatctacaaccctgtcatctatatcatgatgaacaagcaggtgcctactgcgggtgggagggccccagtgccccaggccacaggcgctgcctgccaaggacaagctacttcccagggcaggggagggggctccatcagggttactggcagcagtcttgggtcagcagtcccaatggggagtgtgtgagaaatgcagattcctggccccactcagaactgctgaatctcagggtgggcccaggaacctgcatttccagcaagccctccacaggtggctcagatgctcactcaggtgggagaagctccagtcagctagttctggaagcccaatgtcaaagtcagaaggacccaagtcgggaatgggatgggccagtctccataaagctgaataaggagctaaaaagtcttattctgaggggtaaaggggtaaagggttcctcggagaggtacctccgaggggtaaacagttgggtaaacagtctctgaagtcagctctgccattttctagctgtatggccctgggcaagtcaatttccttctctgtgctttggtttcctcatccatagaaaggtagaaagggcaaaacaccaaactcttggattacaagagataatttacagaacacccttggcacacagagggcaccatgaaatgtcacgggtgacacagcccccttgtgctcagtccctggcatctctaggggtgaggagcgtctgcctagcaggttccctccaggaagctggatttgagtggatggggcgctggaatcgtgaggggcagaagcaggcaaagggtcggggcgaacctcactaacgtgccagttccaagcacactgtgggcagccctggccctgactcaagcctcttgccttccagttccggaactgcatgctcaccaccatctgctgcggcaagaacccactgggtgacgatgaggcctctgctaccgtgtccaagacggagacgagccaggtggccccggcctaagacctgcctaggactctgtggccgactataggcgtctcccatcccctacaccttcccccagccacagccatcccaccaggagcagcgcctgtgcagaatgaacgaagtcacataggctccttaattttttttttttttttaagaaataattaatgaggctcctcactcacctgggacagcctgagaagggacatccaccaagacctactgatctggagtcccacgttccccaaggccagcgggatgtgtgcccctcctcctcccaactcatctttcaggaacacgaggattcttgctttctggaaaagtgtcccagcttagggataagtgtctagcacagaatggggcacacagtaggtgcttaataaatgctggatggatgcaggaaggaatggaggaatgaatgggaagggagaacatatctatcctctcagaccctcgcagcagcagcaactcatacttggctaatgatatggagcagttgtttttccctccctgggcctcactttcttctcctataaaatggaaatcccagatccctggtcctgccgacacgcagctactgagaagaccaaaagaggtgtgtgtgtgtctatgtgtgtgtttcagcactttgtaaatagcaagaagctgtacagattctagttaatgttgtgaataacatcaattaatgtaactagttaattactatgattatcacctcctgatagtgaacattttgagattgggcattcagatgatggggtttcacccaaccttggggcaggtttttaaaaattagctaggcatcaaggccagaccagggctgggggttgggctgtaggcagggacagtcacaggaatgcagaatgcagtcatcagacctgaaaaaacaacactgggggagggggacggtgaaggccaagttcccaatgagggtgagattgggcctggggtctcacccctagtgtggggccccaggtcccgtgcctccccttcccaatgtggcctatggagagacaggcctttctctcagcctctggaagccacctgctcttttgctctagcacctgggtcccagcatctagagcatggagcctctagaagccatgctcacccgcccacatttaattaacagctgagtccctgatgtcatccttatctcgaagagcttagaaacaaagagtgggaaattccactgggcctaccttccttggggatgttcatgggccccagtttccagtttcccttgccagacaagcccatcttcagcagttgctagtccattctccattctggagaatctgctccaaaaagctggccacatctctgaggtgtcagaattaagctgcctcagtaactgctcccccttctccatataagcaaagccagaagctctagctttacccagctctgcctggagactaaggcaaattgggccattaaaagctcagctcctatgttggtattaacggtggtgggttttgttgctttcacactctatccacaggatagattgaaactgccagcttccacctgatccctgaccctgggatggctggattgagcaatgagcagagccaagcagcacagagtcccctggggctagaggtggaggaggcagtcctgggaatgggaaaaaccccaactttggggtcatagaggcacaggtaacccataaaactgcaaacaagctttgtcacctctcagagcttccttatctgcaaaaaagaatcttaaaactgaccttggctgggcacagtggctcacacctctaatcccagcactttgggaggccaaggtgggcagatcacgaggtcaggagtttgagaccagcctgaccaacacggtgaaaccctgtctctactaaaaatacaaaaatcagctgggcatggtggcgcgtgcctgtaatcccagctattcagtgggctgaggcaggagaatcgcttgaacctgggaggtggaggttgcagtgagccgagattgcgccactgcactccagcctgagcaacagagggacagtctgtctccaaacaaaacaaaacaaacaaacaaacaaacaaacaaacaaaaaacaacaacaaaaaaaccacttgatcctaaggggattagatgcgactgtggactttaagtggccagcctactgcctggcatgcagcagatgagactatggcaatactgggcttcagctcagagctggccttactagagaccctgtcccaaaggggaaaaggatggagctaaagctcccgagagtcaccccctcctccgaggtgagaaaggagggcaggagcatgagatagccgatcctcggtgccttggtgaggctggggcaaatcatgctgggatctctatcattgtccctctttactgtgactcactagataatatcagtcaggatacttttggtcacaagtgataggaaatccaactcatttgggctgaagcaaaagggacacattgttggctcacatgaacaaaaagcccggggcttcaggcacagggtatcaccatgactgagatggggattaattctgtgattggccaagtctaggtcacctgatcatacgtaactcatttatgcctgaggttgcaattttttggatttttgcaatcagaccttggcgatgaccttgagcagtaggatataaataactcccacatgcttagcgttccaataatggaatactaggcatacgcaggtctaactgcatcaccatggctggaatggggattcatcctctgattggtcagacctaggtcacatgctcaccctgcagcccaagcaggctgaatggggagaggtaggtttcacaaaggaaagcccaggtgctgttacctgaagtaggagggcaggaggcagggtgagcagagccaacatcaacccagagggaatggaatctaagttggtgttttctgggcacgtggctggaccaggcctccctccctcatcatctcagggacatgagggagaagattcctatgggtggtcccgaaggtctcaccctttgttttggatgctgtgttgggccagggtggcagtgggtgggacagtggcatcttagctgccctgacttgcaggcagcccattccagctccccgccccaaccccaacccagcccactttttctgagaaatggtacatttgccccagcctcatgtccagaggaaaattttactctaacaccagaacattctctggtttgtcctgatagacaagaaagcctccacctccttaatttacaaatgacttgacagctgcttcgtgggcacttgcatacataaagagaaggagctgctgccttaagttgcagcaagtttggccccacctcatctccaggcagccagcagatgtacagagtgcctcttgggtacaatggcagctccattcaaccaaacctgagcaagctgaccccatgccagaatgcactggggactcggagatgaattggagcctagagaccaagtctctaggctatgacctgggctgcctcacggccacagagctctgtcacgccaagggagagatgcacccctgaaagcctgaggtgccccataaggagagagtgggtgcccttcccaactatgtagcttcagggcaagttctctttctttctttttctttctttctctttctttctttcttt

SEQ ID NO: 99 - DNA, 13706 bp, synthetic construct
  misc_feature 1..13706: note = Synthetic Polynucleotide
  source 1..13706: mol_type = other DNA
gtgggggaccaggagaaagaaagccaaggaagaggaggaggaggaggagaaggaggagaaggatgctgacctagcagctcctctcacagcagctcctctcttgcagaggctgaagagcgatttgtgccctgcaagctaagcccctaatccaccgaggcaaaggcaaagcccctagccgggctcccgagggctgggactcgggtgccccaagatggctgcatccagccatcttggcttagaaagccccccacatgccagcttggccaacacccacaccatgggtttctctggactgcccgacacaaggtgtgggtgctggccaggcctgtgttcaaatcccagctctgcagaggaactttgaccctgcataccccagattcctcagtggtcagtggggagttagaccctcttcatagggggcaggaggagttgttcattcattcaacaaatgtttattgaacacctcctatgggttgtgagctcagaggcagcgatgaacaggccaggctggtcctgcattctagaaatagatgggaagtcagtcaataagtagacaaatgaggccaggtgtggtggcatgcctgtagacccagttactcgggatgctgaggtaggaggatcacttgagcctaggacaggaattcaaggctgcagtaagctatgattgcgccactgcactccagcctgggcaacagagcaagactcatctctaaaaaacatttaaaaattgttttaagaagacaaatgagatagtcgctgatggtaatgactgtgtaaaaactgaacatggctgggtgtggttgctcacacctataatctcagcactttgggaggctgagattacagcctcccaagtggctcccaaggcaggaggatcacttgagcctgggagttagagaacagcttggacaatatagggagagcccaactctacaaaaatgaaaataaattagccaggcatggtggcacacaccaatggtcccagctactcaggggttgaggtggtggaccgcttgagcccaggaggttgaggctgcagtgagccatgatcatgccgctgcactccaacctgagtcacagagtgataccctgtctcaaaaaacaataggccaggtgtggtggctcacgcctgtaaccccagcactttgggaggccgaggcggatggatcacttgagatcaggagttagagaccagcctggctaacatggcaaaatcctgtctgtactaaaaatataaaaattagccaggcatggcagtacatgcctgtagtcctggttacttgggaggctaaggcaggagaatcgcttgaacccaggaagaggaggttgcagtgagccaagatcacaccactgcactccagcttgggtgacagagtgagaccctgtctcaaaacagctaaacctggtgggggtgcctggtgtgtaggatggtcaggggtggtctctccaaggacatgagtgtgagcggagacctgaaggagactcaggaagagattaatactgtcagcaacaaatatattgatcacttacaagcactcccaataatcctattaggtaggcactattatcattcccattttacagagtggagaaccgaagcacactctcgggagggcggggtagctggctgcacccaggctgtgtagcctcagtccagatgtaagggtgggtggaaaagagccttgcccaatgagggagaacagtgaaaccaaggccatagggtctaaagattcacgaaccaggctctcatggagaaagcaggtgaggtttactgtatagatgggtgtgcccctaccccacactgaggcttcctcgtctgagcaaactgaggcccagagaggggaaggaagcaggactaccatggtgactcaaagaccagctagaatccagcctcctctcctcgaggcttccactgccccacgccaggcctgtgtgactcagtctagggcctttccattaccccagctaaacctttctttagtcatttataccatggtgtgaatggctggctggtctttcctgagagctatctttgatgaggggagggaggcatagccaggtttgggaagctgataccccaggaagcccagttgactgtgtgggttatagcccaggctgtcactgatttgtaacgggacctgagcaactctgcagagctaggcctcagtcttttcatctgcaaaatggatatagcagagatggtcagagtaggtgacttcgaatgacccttccagctcactatgagtctgttttcctgaacaaagagcattttttgtttaaaaaaaaatttcttgggccggacacggtggttcactcctataatcctggcactttgggaggccgaggagggtggatcgcttgagccaggagttcaggaccagcctgggcaacatagcgagactccacccctacaaaaaatacaaaaactagtggtgtgcacttgtggtcccagctactcaggaggctgaggtgagaggatcgcttgagcccaggaggcagaggctacagtgagctatgattgtggcactgcactccagcctgggcgacagagaccttgtctcaaaactttttttttcttcgtcaagctttacagaataaagagcactgtcacctcagtgatggctgttagttccccatcaccagggctccatgaggttgcaattgtgaaactcacaaaggaggaacctgagacagagaggggaagtactgagatcatctaggtccattcccccactcactcgttcattcaacaaatattcaggagcaccttctaggtgccaggccctggagacacatcagtgaacaaaacagacatcatcccacctctttccactacaggccaagcaccatgctggtctctgggaaccctgttgtgagcaagacagacccaggcttacccttgtggactcatgttacaggcagggagacgggcacaaaacacaaataaaaagcttccatgctgtcagaagcactatgcaaaaagcaagatgctgaggtactgctaagctgtgtgggatgggggctcagcccggccagggaggggccagttgtgggtcagtcttgacccaaggcatccaggacaccctccttctggccatgagggtccacgtcagaatcaaaccctcaccttaacctcattagcgttgggcataatcaccaggccaagcgccttaaactacgagaggccccatcccacccgccctgccttagccctgccacgtgtgccaaacgctgttagacccaacaccacccaggccaggtagggggctggagcccaggtgggctgcagggaagggggcactcttctgagcagacagatctgggaatcctgggtgggaagagagacagtgagagagagattaagggatatttcccaggcatcagggctttgcactctcaggggtccttccgcctggatgtccttcccctgaagcttcctcctgttgttccgttctcagctcaagctccagcttctcagagaagcctcctgtgttgggagtggctgcgactgaactgtccctactgttattcgctcttctatttgtttgtggtccctgtgccccctcaccccacaaaaacactggcttcttgtgagcaggagcttgctctttcgtgtaccctgtgtgtccccaaggaccaagcaccttgtctgggccacagtaggtgctcaatacacatgttggctggacagtggtcactgagcggccgcacgtcgggcactctcagcacttgcacaggccgccccagacaccccacttcattcctgggaggtgtcatcatgttgcttggacgacggggagagggggacctgccagtgttggcctccattttcccccagtcatctgcccccaaggctctgactactttctttctcacggtacatcctgctattctggaatcggccctcgtggggccacctggtacatggcatttgaggccctcgtggctgattaggcctcccccaacagtgccctgtctgctgcctccagggccagcctccccttcagactggagtcccctgaagggttctgcccctcccctgctctggtagccccctccatcctccctccctccactccatctttgggggcatttgagtcacctttctacaccagtgatctgcccaagccactgctcactttcctctggataaagccaggttccccggcctagcgttcaagacccattacaactgcccccagcccagatcttccccacctagccacctggcaaactgctccttctctcaaaggcccaaacatggcctcccagactgcaacccccaggcagtcaggccctgtctccacaacctcacagccaccctggacggaatctgcttcttcccacatttgagtcctcctcagcccctgagctcctctgggcagggctgtttctttccatctttgtattcccaggggcctgcaaataaatgtttaatgaacgaacaagagagtgaattccaattccatgcaacaaggattgggctcctgggccctaggctatgtgtctggcaccagaaacggaagctgcaggttgcagcccctgccctcatggagctcctcctgtcagaggagtgtggggactggatgactccagaggtaacttgtgggggaacgaacaggtaaggggctgtgtgacgagatgagagactgggagaataaaccagaaagtctctagctgtccagaggacatagcacagaggcccatggtccctatttcaaacccaggccaccagactgagctgggaccttgggacagacaagtcatgcagaagttaggggaccttctcctcccttttcctggatcctgagtacctctcctccctgacctcaggcttcctcctagtgtcaccttggcccctcttagaagccaattaggccctcagtttctgcagcggggattaatatgattatgaacacccccaatctcccagatgctgattcagccaggagcttaggagggggaggtcactttataagggtctgggggggtcagaacccagagtcatccagctggagccctgagtggctgagctcaggccttcgcagcattcttgggtgggagcagccacgggtcagccacaagggccacagccatgaatggcacagaaggccctaacttctacgtgcccttctccaatgcgacgggtgtggtacgcagccacttcgagtacccacagtactacctggctgagccatggcagttctccatgctggccgcctacatgtttctgctgatcgtgctgggcttccccatcaacttcctcacgctctacgtcaccgtccagcacaagaagctgcgcacgcctctcaactacatcctgctcaacctagccgtggctgacctcttcatggtcctaggtggcttcaccagcaccctctacacctctctgcatggatacttcgtcttcgggcccacaggatgcaatttggagggcttctttgccaccctgggcggtatgagccgggtgtgggtggggtgtgcaggagcccgggagcatggaggggtctgggagagtcccgggcttggcggtggtggctgagaggccttctcccttctcctgtcctgtcaatgttatccaaagccctcatatattcagtcaacaaacaccattcatggtgatagccgggctgctgtttgtgcagggctggcactgaacactgccttgatcttatttggagcaatatgcgcttgtctaatttcacagcaagaaaactgagctgaggctcaaagaagtcaagcgccctgctggggcgtcacacagggacgggtgcagagttgagttggaagcccgcatctatctcgggccatgtttgcagcaccaagcctctgtttcccttggagcagctgtgctgagtcagacccaggctgggcactgagggagagctgggcaagccagacccctcctctctgggggcccaagctcagggtgggaagtggattttccattctccagtcattgggtcttccctgtgctgggcaatgggctcggtcccctctggcatcctctgcctcccctctcagcccctgtcctcaggtgcccctccagcctccctgccgcgttccaagtctcctggtgttgagaaccgcaagcagccgctctgaagcagttcctttttgctttagaataatgtcttgcatttaacaggaaaacagatggggtgctgcagggataacagatcccacttaacagagaggaaaactgaggcagggagaggggaagagactcatttagggatgtggccaggcagcaacaagagcctaggtctcctggctgtgatccaggaatatctctgctgagatgcaggaggagacgctagaagcagccattgcaaagctgggtgacggggagagcttaccgccagccacaagcgtctctctgccagccttgccctgtctcccccatgtccaggctgctgcctcggtcccattctcagggaatctctggccattgttgggtgtttgttgcattcaataatcacagatcactcagttctggccagaaggtgggtgtgccacttacgggtggttgttctctgcagggtcagtcccagtttacaaatattgtccctttcactgttaggaatgtcccagtttggttgattaactatatggccactctccctatggaacttcatggggtggtgagcaggacagatgtctgaattccatcatttccttcttcttcctctgggcaaaacattgcacattgcttcatggctcctaggagaggcccccacatgtccgggttatttcatttcccgagaagggagagggaggaaggactgccaattctgggtttccaccacctctgcattccttcccaacaaggaactctgccccacattaggatgcattcttctgctaaacacacacacacacacacacacacacaacacacacacacacacacacacacacacacacacaaaactccctaccgggttcccagttcaatcctgaccccctgatctgattcgtgtcccttatgggcccagagcgctaagcaaataacttcccccattccctggaatttctttgcccagctctcctcagcgtgtggtccctctgccccttccccctcctcccagcaccaagctctctccttccccaaggcctcctcaaatccctctcccactcctggttgccttcctagctaccctctccctgtctaggggggagtgcaccctccttaggcagtggggtctgtgctgaccgcctgctgactgccttgcaggtgaaattgccctgtggtccttggtggtcctggccatcgagcggtacgtggtggtgtgtaagcccatgagcaacttccgcttcggggagaaccatgccatcatgggcgttgccttcacctgggtcatggcgctggcctgcgccgcacccccactcgccggctggtccaggtaatggcactgagcagaagggaagaagctccgggggctctttgtagggtcctccagtcaggactcaaacccagtagtgtctggttccaggcactgaccttgtatgtctcctggcccaaatgcccactcagggtaggggtgtagggcagaagaagaaacagactctaatgttgctacaagggctggtcccatctcctgagccccatgtcaaacagaatccaagacatcccaacccttcaccttggctgtgcccctaatcctcaactaagctaggcgcaaattccaatcctctttggtctagtaccccgggggcagccccctctaaccttgggcctcagcagcaggggaggccacaccttcctagtgcaggtggccatattgtggccccttggaactgggtcccactcagcctctaggcgattgtctcctaatggggctgagatgagacacagtggggacagtggtttggacaataggactggtgactctggtccccagaggcctcatgtccctctgtctccagaaaattcccactctcacttccctttcctcctcagtcttgctagggtccatttcttaccccttgctgaatttgagcccaccccctggactttttccccatcttctccaatctggcctagttctatcctctggaagcagagccgctggacgctctgggtttcctgaggcccgtccactgtcaccaatatcaggaaccattgccacgtcctaatgacgtgcgctggaagcctctagtttccagaagctgcacaaagatcccttagatactctgtgtgtccatctttggcctggaaaatactctcaccctggggctaggaagacctcggtttgtacaaacttcctcaaatgcagagcctgagggctctccccacctcctcaccaaccctctgcgtggcatagccctagcctcagcgggcagtggatgctggggctgggcatgcagggagaggctgggtggtgtcatctggtaacgcagccaccaaacaatgaagcgacactgattccacaaggtgcatctgcatccccatctgatccattccatcctgtcacccagccatgcagacgtttatgatccccttttccagggagggaatgtgaagccccagaaagggccagcgctcggcagccaccttggctgttcccaagtccctcacaggcagggtctccctacctgcctgtcctcaggtacatccccgagggcctgcagtgctcgtgtggaatcgactactacacgctcaagccggaggtcaacaacgagtcttttgtcatctacatgttcgtggtccacttcaccatccccatgattatcatctttttctgctatgggcagctcgtcttcaccgtcaaggaggtacgggccggggggtgggcggcctcacggctctgagggtccagcccccagcatgcatctgcggctcctgctccctggaggagccatggtctggacccgggtcccgtgtcctgcaggccgctgcccagcagcaggagtcagccaccacacagaaggcagagaaggaggtcacccgcatggtcatcatcatggtcatcgctttcctgatctgctgggtgccctacgccagcgtggcattctacatcttcacccaccagggctccaacttcggtcccatcttcatgaccatcccagcgttctttgccaagagcgccgccatctacaaccctgtcatctatatcatgatgaacaagcaggtgcctactgcgggtgggagggccccagtgccccaggccacaggcgctgcctgccaaggacaagctacttcccagggcaggggagggggctccatcagggttactggcagcagtcttgggtcagcagtcccaatggggagtgtgtgagaaatgcagattcctggccccactcagaactgctgaatctcagggtgggcccaggaacctgcatttccagcaagccctccacaggtggctcagatgctcactcaggtgggagaagctccagtcagctagttctggaagcccaatgtcaaagtcagaaggacccaagtcgggaatgggatgggccagtctccataaagctgaataaggagctaaaaagtcttattctgaggggtaaaggggtaaagggttcctcggagaggtacctccgaggggtaaacagttgggtaaacagtctctgaagtcagctctgccattttctagctgtatggccctgggcaagtcaatttccttctctgtgctttggtttcctcatccatagaaaggtagaaagggcaaaacaccaaactcttggattacaagagataatttacagaacacccttggcacacagagggcaccatgaaatgtcacgggtgacacagcccccttgtgctcagtccctggcatctctaggggtgaggagcgtctgcctagcaggttccctccaggaagctggatttgagtggatggggcgctggaatcgtgaggggcagaagcaggcaaagggtcggggcgaacctcactaacgtgccagttccaagcacactgtgggcagccctggccctgactcaagcctcttgccttccagttccggaactgcatgctcaccaccatctgctgcggcaagaacccactgggtgacgatgaggcctctgctaccgtgtccaagacggagacgagccaggtggccccggcctaagacctgcctaggactctgtggccgactataggcgtctcccatcccctacaccttcccccagccacagccatcccaccaggagcagcgcctgtgcagaatgaacgaagtcacataggctccttaattttttttttttttttaagaaataattaatgaggctcctcactcacctgggacagcctgagaagggacatccaccaagacctactgatctggagtcccacgttccccaaggccagcgggatgtgtgcccctcctcctcccaactcatctttcaggaacacgaggattcttgctttctggaaaagtgtcccagcttagggataagtgtctagcacagaatggggcacacagtaggtgcttaataaatgctggatggatgcaggaaggaatggaggaatgaatgggaagggagaacatatctatcctctcagaccctcgcagcagcagcaactcatacttggctaatgatatggagcagttgtttttccctccctgggcctcactttcttctcctataaaatggaaatcccagatccctggtcctgccgacacgcagctactgagaagaccaaaagaggtgtgtgtgtgtctatgtgtgtgtttcagcactttgtaaatagcaagaagctgtacagattctagttaatgttgtgaataacatcaattaatgtaactagttaattactatgattatcacctcctgatagtgaacattttgagattgggcattcagatgatggggtttcacccaaccttggggcaggtttttaaaaattagctaggcatcaaggccagaccagggctgggggttgggctgtaggcagggacagtcacaggaatgcagaatgcagtcatcagacctgaaaaaacaacactgggggagggggacggtgaaggccaagttcccaatgagggtgagattgggcctggggtctcacccctagtgtggggccccaggtcccgtgcctccccttcccaatgtggcctatggagagacaggcctttctctcagcctctggaagccacctgctcttttgctctagcacctgggtcccagcatctagagcatggagcctctagaagccatgctcacccgcccacatttaattaacagctgagtccctgatgtcatccttatctcgaagagcttagaaacaaagagtgggaaattccactgggcctaccttccttggggatgttcatgggccccagtttccagtttcccttgccagacaagcccatcttcagcagttgctagtccattctccattctggagaatctgctccaaaaagctggccacatctctgaggtgtcagaattaagctgcctcagtaactgctcccccttctccatataagcaaagccagaagctctagctttacccagctctgcctggagactaaggcaaattgggccattaaaagctcagctcctatgttggtattaacggtggtgggttttgttgctttcacactctatccacaggatagattgaaactgccagcttccacctgatccctgaccctgggatggctggattgagcaatgagcagagccaagcagcacagagtcccctggggctagaggtggaggaggcagtcctgggaatgggaaaaaccccaactttggggtcatagaggcacaggtaacccataaaactgcaaacaagctttgtcacctctcagagcttccttatctgcaaaaaagaatcttaaaactgaccttggctgggcacagtggctcacacctctaatcccagcactttgggaggccaaggtgggcagatcacgaggtcaggagtttgagaccagcctgaccaacacggtgaaaccctgtctctactaaaaatacaaaaatcagctgggcatggtggcgcgtgcctgtaatcccagctattcagtgggctgaggcaggagaatcgcttgaacctgggaggtggaggttgcagtgagccgagattgcgccactgcactccagcctgagcaacagagggacagtctgtctccaaacaaaacaaaacaaacaaacaaacaaacaaacaaacaaaaaacaacaacaaaaaaaccacttgatcctaaggggattagatgcgactgtggactttaagtggccagcctactgcctggcatgcagcagatgagactatggcaatactgggcttcagctcagagctggccttactagagaccctgtcccaaaggggaaaaggatggagctaaagctcccgagagtcaccccctcctccgaggtgagaaaggagggcaggagcatgagatagccgatcctcggtgccttggtgaggctggggcaaatcatgctgggatctctatcattgtccctctttactgtgactcactagataatatcagtcaggatacttttggtcacaagtgataggaaatccaactcatttgggctgaagcaaaagggacacattgttggctcacatgaacaaaaagcccggggcttcaggcacagggtatcaccatgactgagatggggattaattctgtgattggccaagtctaggtcacctgatcatacgtaactcatttatgcctgaggttgcaattttttggatttttgcaatcagaccttggcgatgaccttgagcagtaggatataaataactcccacatgcttagcgttccaataatggaatactaggcatacgcaggtctaactgcatcaccatggctggaatggggattcatcctctgattggtcagacctaggtcacatgctcaccctgcagcccaagcaggctgaatggggagaggtaggtttcacaaaggaaagcccaggtgctgttacctgaagtaggagggcaggaggcagggtgagcagagccaacatcaacccagagggaatggaatctaagttggtgttttctgggcacgtggctggaccaggcctccctccctcatcatctcagggacatgagggagaagattcctatgggtggtcccgaaggtctcaccctttgttttggatgctgtgttgggccagggtggcagtgggtgggacagtggcatcttagctgccctgacttgcaggcagcccattccagctccccgccccaaccccaacccagcccactttttctgagaaatggtacatttgccccagcctcatgtccagaggaaaattttactctaacaccagaacattctctggtttgtcctgatagacaagaaagcctccacctccttaatttacaaatgacttgacagctgcttcgtgggcacttgcatacataaagagaaggagctgctgccttaagttgcagcaagtttggccccacctcatctccaggcagccagcagatgtacagagtgcctcttgggtacaatggcagctccattcaaccaaacctgagcaagctgaccccatgccagaatgcactggggactcggagatgaattggagcctagagaccaagtctctaggctatgacctgggctgcctcacggccacagagctctgtcacgccaagggagagatgcacccctgaaagcctgaggtgccccataaggagagagtgggtgcccttcccaactatgtagcttcagggcaagttctctttctttctttttctttctttctctttctttctttcttt

SEQ ID NO: 100 - protein, 348 aa, synthetic construct [sequence omitted]

SEQ ID NO: 101 - protein, 348 aa, synthetic construct
  REGION 1..348: note = Synthetic Polypeptide
MNGTEGPNFYVPFSNATGVVRSHFEYPQYYLAEPWQFSMLAAYMFLLIVLGFPINFLTLYVTVQHKKLRTPLNYILLNLAVADLFMVLGGFTSTLYTSLHGYFVFGPTGCNLEGFFATLGGEIALWSLVVLAIERYVVVCKPMSNFRFGENHAIMGVAFTWVMALACAAPPLAGWSRYIPEGLQCSCGIDYYTLKPEVNNESFVIYMFVVHFTIPMIIIFFCYGQLVFTVKEAAAQQQESATTQKAEKEVTRMVIIMVIAFLICWVPYASVAFYIFTHQGSNFGPIFMTIPAFFAKSAAIYNPVIYIMMNKQFRNCMLTTICCGKNPLGDDEASATVSKTETSQVAPA

SEQ ID NO: 102 - protein, 147 aa, synthetic construct
  REGION 1..147: note = Synthetic Polypeptide
KEFLLYLAGFVDGDGSIWASIIPEQGYKFKHRLRLSFTVAQKTQRRWFLDKLVDEIGVGYVVDQGSVSEYRLSEIKPLHNFLTQLQPFLKLKQKQANLVLKIIEQLPSAKESPDKFLEVCTWVDQIAALNDSKTRKTTSETVRAVLD

SEQ ID NO: 103 - protein, 147 aa, synthetic construct; identical to SEQ ID NO: 102
  REGION 1..147: note = Synthetic Polypeptide

SEQ ID NO: 104 - protein, 147 aa, synthetic construct; identical to SEQ ID NO: 102
  REGION 1..147: note = Synthetic Polypeptide

SEQ ID NO: 105 - protein, 147 aa, synthetic construct; identical to SEQ ID NO: 102
  REGION 1..147: note = Synthetic Polypeptide

SEQ ID NO: 106 - protein, 147 aa, synthetic construct
  REGION 1..147: note = Synthetic Polypeptide
KEFLLYLAGFVDGDGSIYATIMPEQRQKFKHRLRLYFEVCQKTQRRWFLDKLVDEIGVGYVYDQGSVSTYRLSQIKPLHNFLTQLQPFLKLKQKQANLVLKIIEQLPSAKESPDKFLEVCTWVDQIAALNDSKTRKTTSETVRAVLD

SEQ ID NO: 107 - protein, 147 aa, synthetic construct
  REGION 1..147: note = Synthetic Polypeptide
KEFLLYLAGFVDGDGSIYATIIPSQTDKFKHRLRLYFAVSQKTQRRWFLDKLVDEIGVGYVIDSGSVSEYRLSEIKPLHNFLTQLQPFLKLKQKQANLVLKIIEQLPSAKESPDKFLEVCTWVDQIAALNDSKTRKTTSETVRAVLD

SEQ ID NO: 108 - protein, 147 aa, synthetic construct
  REGION 1..147: note = Synthetic Polypeptide
KEFLLYLAGFVDGDGSIYASIQPDQVYKFKHRLRLRFAVFQKTQRRWFLDKLVDEIGVGYVYDHGSVSEYRLSQIKPLHNFLTQLQPFLKLKQKQANLVLKIIEQLPSAKESPDKFLEVCTWVDQIAALNDSKTRKTTSETVRAVLD

SEQ ID NO: 109 - protein, 147 aa, synthetic construct
  REGION 1..147: note = Synthetic Polypeptide
KEFLLYLAGFVDGDGSIYASIEPVQTYKFKHRLRLSFAVSQKTQRRWFLDKLVDEIGVGYVCDVGSVSEYRLSEIKPLHNFLTQLQPFLKLKQKQANLVLKIIEQLPSAKESPDKFLEVCTWVDQIAALNDSKTRKTTSETVRAVLD

SEQ ID NO: 110 - protein, 147 aa, synthetic construct
  REGION 1..147: note = Synthetic Polypeptide
KEFLLYLAGFVDGDGSIYASITPSQAGKFKHRLRLYFEVSQKTQRRWFLDKLVDEIGVGYVYDQGSVSCYRLSQIKPLHNFLTQLQPFLKLKQKQANLVLKIIEQLPSAKESPDKFLEVCTWVDQIAALNDSKTRKTTSETVRAVLD

SEQ ID NO: 111 - protein, 147 aa, synthetic construct
  REGION 1..147: note = Synthetic Polypeptide
KEFLLYLAGFVDGDGSIYATIEPAQRYKFKHRLRLKFAVSQKTQRRWFLDKLVDEIGVGYVADQGSVSEYRLSQIKPLHNFLTQLQPFLKLKQKQANLVLKIIEQLPSAKESPDKFLEVCTWVDQIAALNDSKTRKTTSETVRAVLD

SEQ ID NO: 112 - protein, 147 aa, synthetic construct
  REGION 1..147: note = Synthetic Polypeptide
KEFLLYLAGFVDGDGSIYATIEPQQPGKFKHRLSLRFAVYQKTQRRWFLDKLVDEIGVGYVYDPGSVSEYRLSQIKPLHNFLTQLQPFLKLKQKQANLVLKIIEQLPSAKESPDKFLEVCTWVDQIAALNDSKTRKTTSETVRAVLD

SEQ ID NO: 113 - protein, 147 aa, synthetic construct
  REGION 1..147: note = Synthetic Polypeptide
KEFLLYLAGFVDGDGSIYASIGPEQSSKFKHRLRLLFAVAQKTQRRWFLDKLVDEIGVGYVVDQGSVSEYRLSQIKPLHNFLTQLQPFLKLKQKQANLVLKIIEQLPSAKESPDKFLEVCTWVDQIAALNDSKTRKTTSETVRAVLD

SEQ ID NO: 114 - protein, 147 aa, synthetic construct
  REGION 1..147: note = Synthetic Polypeptide
KEFLLYLAGFVDGDGSIYATIQPDQNQKFKHRLRLYFAVYQKTQRRWFLDKLVDEIGVGYVYDTGSVSRYQLSQIKPLHNFLTQLQPFLKLKQKQANLVLKIIEQLPSAKESPDKFLEVCTWVDQIAALNDSKTRKTTSETVRAVLD

SEQ ID NO: 115 - protein, 147 aa, synthetic construct; identical to SEQ ID NO: 102
  REGION 1..147: note = Synthetic Polypeptide

SEQ ID NO: 116 - protein, 147 aa, synthetic construct; identical to SEQ ID NO: 102
  REGION 1..147: note = Synthetic Polypeptide

SEQ ID NO: 117 - protein, 147 aa, synthetic construct; identical to SEQ ID NO: 102
  REGION 1..147: note = Synthetic Polypeptide

SEQ ID NO: 118 - protein, 147 aa, synthetic construct; identical to SEQ ID NO: 102
  REGION 1..147: note = Synthetic Polypeptide

SEQ ID NO: 119 - protein, 147 aa, synthetic construct; identical to SEQ ID NO: 102
  REGION 1..147: note = Synthetic Polypeptide

SEQ ID NO: 120 - protein, 147 aa, synthetic construct; identical to SEQ ID NO: 102
  REGION 1..147: note = Synthetic Polypeptide

SEQ ID NO: 121 - protein, 147 aa, synthetic construct; identical to SEQ ID NO: 102
  REGION 1..147: note = Synthetic Polypeptide

SEQ ID NO: 122 - protein, 147 aa, synthetic construct; identical to SEQ ID NO: 102
  REGION 1..147: note = Synthetic Polypeptide

SEQ ID NO: 123 - protein, 147 aa, synthetic construct; identical to SEQ ID NO: 102
  REGION 1..147: note = Synthetic Polypeptide

SEQ ID NO: 124 - protein, 147 aa, synthetic construct; identical to SEQ ID NO: 102
  REGION 1..147: note = Synthetic Polypeptide

SEQ ID NO: 125 - protein, 147 aa, synthetic construct; identical to SEQ ID NO: 102
  REGION 1..147: note = Synthetic Polypeptide

SEQ ID NO: 126 - protein, 147 aa, synthetic construct; identical to SEQ ID NO: 102
  REGION 1..147: note = Synthetic Polypeptide

SEQ ID NO: 127 - protein, 147 aa, synthetic construct; identical to SEQ ID NO: 102
  REGION 1..147: note = Synthetic Polypeptide

SEQ ID NO: 128 - protein, 147 aa, synthetic construct; identical to SEQ ID NO: 102
  REGION 1..147: note = Synthetic Polypeptide

SEQ ID NO: 129 - protein, 147 aa, synthetic construct; identical to SEQ ID NO: 102
  REGION 1..147: note = Synthetic Polypeptide

SEQ ID NO: 130 - protein, 147 aa, synthetic construct; identical to SEQ ID NO: 102
  REGION 1..147: note = Synthetic Polypeptide

SEQ ID NO: 131 - protein, 147 aa, synthetic construct; identical to SEQ ID NO: 102
  REGION 1..147: note = Synthetic Polypeptide

SEQ ID NO: 132 - protein, 147 aa, synthetic construct; identical to SEQ ID NO: 102
  REGION 1..147: note = Synthetic Polypeptide

SEQ ID NO: 133 - protein, 147 aa, synthetic construct; identical to SEQ ID NO: 102
  REGION 1..147: note = Synthetic Polypeptide

SEQ ID NO: 134 - protein, 147 aa, synthetic construct; identical to SEQ ID NO: 102
  REGION 1..147: note = Synthetic Polypeptide

SEQ ID NO: 135 - protein, 147 aa, synthetic construct; identical to SEQ ID NO: 102
  REGION 1..147: note = Synthetic Polypeptide

SEQ ID NO: 136 - protein, 147 aa, synthetic construct; identical to SEQ ID NO: 102
  REGION 1..147: note = Synthetic Polypeptide

SEQ ID NO: 137 - protein, 147 aa, synthetic construct; identical to SEQ ID NO: 102
  REGION 1..147: note = Synthetic Polypeptide

SEQ ID NO: 138 - protein, 147 aa, synthetic construct; identical to SEQ ID NO: 102
  REGION 1..147: note = Synthetic Polypeptide

SEQ ID NO: 139 - protein, 147 aa, synthetic construct; identical to SEQ ID NO: 102
  REGION 1..147: note = Synthetic Polypeptide

SEQ ID NO: 140 - protein, 147 aa, synthetic construct; identical to SEQ ID NO: 102
  REGION 1..147: note = Synthetic Polypeptide

SEQ ID NO: 141 - protein, 147 aa, synthetic construct; identical to SEQ ID NO: 102
  REGION 1..147: note = Synthetic Polypeptide

SEQ ID NO: 142 - protein, 147 aa, synthetic construct; identical to SEQ ID NO: 102
  REGION 1..147: note = Synthetic Polypeptide

SEQ ID NO: 143 - protein, 147 aa, synthetic construct; identical to SEQ ID NO: 102
  REGION 1..147: note = Synthetic Polypeptide

SEQ ID NO: 144 - protein, 147 aa, synthetic construct; identical to SEQ ID NO: 102
  REGION 1..147: note = Synthetic Polypeptide

SEQ ID NO: 145 - protein, 147 aa, synthetic construct; identical to SEQ ID NO: 102
  REGION 1..147: note = Synthetic Polypeptide

SEQ ID NO: 146 - protein, 147 aa, synthetic construct; identical to SEQ ID NO: 102
  REGION 1..147: note = Synthetic Polypeptide

SEQ ID NO: 147 - protein, 147 aa, synthetic construct; identical to SEQ ID NO: 102
  REGION 1..147: note = Synthetic Polypeptide

SEQ ID NO: 148 - protein, 147 aa, synthetic construct; identical to SEQ ID NO: 102
  REGION 1..147: note = Synthetic Polypeptide

SEQ ID NO: 149 - protein, 147 aa, synthetic construct; identical to SEQ ID NO: 102
  REGION 1..147: note = Synthetic Polypeptide

SEQ ID NO: 150 - protein, 147 aa, synthetic construct
  REGION 1..147: note = Synthetic Polypeptide
KEFLLYLAGFVDGDGSIWASILPESRMKFKHRLRLGFTVAQKTQRRWFLDKLVDEIGVGYVVDQGSVSEYRLSEIKPLHNFLTQLQPFLKLKQKQANLVLKIIEQLPSAKESPDKFLEVCTWVDQIAALNDSKTRKTTSETVRAVLD

SEQ ID NO: 151 - protein, 147 aa, synthetic construct
  REGION 1..147: note = Synthetic Polypeptide
KEFLLYLAGFVDGDGSIWAQILPEKKCAFKHRLRLWFTVAQKTQRRWFLDKLVDEIGVGYVVDQGSVSEYRLSEIKPLHNFLTQLQPFLKLKQKQANLVLKIIEQLPSAKESPDKFLEVCTWVDQIAALNDSKTRKTTSETVRAVLD

SEQ ID NO: 152 - protein, 147 aa, synthetic construct
  REGION 1..147: note = Synthetic Polypeptide
KEFLLYLAGFVDGDGSIWACIVPEKASRFKHRLRLAFTVAQKTQRRWFLDKLVDEIGVGYVVDQGSVSEYRLSEIKPLHNFLTQLQPFLKLKQKQANLVLKIIEQLPSAKESPDKFLEVCTWVDQIAALNDSKTRKTTSETVRAVLD

SEQ ID NO: 153 - protein, 147 aa, synthetic construct
  REGION 1..147: note = Synthetic Polypeptide
KEFLLYLAGFVDGDGSIWATIVPEKSSIFKHRLRLYFTVAQKTQRRWFLDKLVDEIGVGYVVDQGSVSEYRLSEIKPLHNFLTQLQPFLKLKQKQANLVLKIIEQLPSAKESPDKFLEVCTWVDQIAALNDSKTRKTTSETVRAVLD

SEQ ID NO: 154 - protein, 147 aa, synthetic construct
  REGION 1..147: note = Synthetic Polypeptide
KEFLLYLAGFVDGDGSIWASIVPEERTRFKHRLRLYFTVAQKTQRRWFLDKLVDEIGVGYVVDQGSVSEYRLSEIKPLHNFLTQLQPFLKLKQKQANLVLKIIEQLPSAKESPDKFLEVCTWVDQIAALNDSKTRKTTSETVRAVLD

SEQ ID NO: 155 - protein, 147 aa, synthetic construct
  REGION 1..147: note = Synthetic Polypeptide
KEFLLYLAGFVDGDGSIWARIEPEKGGRFKHRLRLYFTVAQKTQRRWFLDKLVDEIGVGYVVDQGSVSEYRLSEIKPLHNFLTQLQPFLKLKQKQANLVLKIIEQLPSAKESPDKFLEVCTWVDQIAALNDSKTRKTTSETVRAVLD

SEQ ID NO: 156 - protein, 147 aa, synthetic construct
  REGION 1..147: note = Synthetic Polypeptide
KEFLLYLAGFVDGDGSIWASISPEVRAPFKHRLRLYFTVAQKTQRRWFLDKLVDEIGVGYVVDQGSVSEYRLSEIKPLHNFLTQLQPFLKLKQKQANLVLKIIEQLPSAKESPDKFLEVCTWVDQIAALNDSKTRKTTSETVRAVLD

SEQ ID NO: 157 - protein, 147 aa, synthetic construct
  REGION 1..147: note = Synthetic Polypeptide
KEFLLYLAGFVDGDGSIWASILPETSARFKHRLRLFFTVAQKTQRRWFLDKLVDEIGVGYVVDQGSVSEYRLSEIKPLHNFLTQLQPFLKLKQKQANLVLKIIEQLPSAKESPDKFLEVCTWVDQIAALNDSKTRKTTSETVRAVLD

SEQ ID NO: 158 - protein, 147 aa, synthetic construct
  REGION 1..147: note = Synthetic Polypeptide
KEFLLYLAGFVDGDGSIWAAILPEQSYRFKHRLRLAFTVAQKTQRRWFLDKLVDEIGVGYVVDQGSVSEYRLSEIKPLHNFLTQLQPFLKLKQKQANLVLKIIEQLPSAKESPDKFLEVCTWVDQIAALNDSKTRKTTSETVRAVLD

SEQ ID NO: 159 - protein, 147 aa, synthetic construct
  REGION 1..147: note = Synthetic Polypeptide
KEFLLYLAGFVDGDGSIWASILPERKTKFKHRLRLAFTVAQKTQRRWFLDKLVDEIGVGYVVDQGSVSEYRLSEIKPLHNFLTQLQPFLKLKQKQANLVLKIIEQLPSAKESPDKFLEVCTWVDQIAALNDSKTRKTTSETVRAVLD

SEQ ID NO: 160 - protein, 147 aa, synthetic construct
  REGION 1..147: note = Synthetic Polypeptide
KEFLLYLAGFVDGDGSIWACIEPERGYRFKHRLRLAFTVAQKTQRRWFLDKLVDEIGVGYVVDQGSVSEYRLSEIKPLHNFLTQLQPFLKLKQKQANLVLKIIEQLPSAKESPDKFLEVCTWVDQIAALNDSKTRKTTSETVRAVLD

SEQ ID NO: 161 - protein, 147 aa, synthetic construct
  REGION 1..147: note = Synthetic Polypeptide
KEFLLYLAGFVDGDGSIWARIEPELRLRFKHRLRLFFTVAQKTQRRWFLDKLVDEIGVGYVVDQGSVSEYRLSEIKPLHNFLTQLQPFLKLKQKQANLVLKIIEQLPSAKESPDKFLEVCTWVDQIAALNDSKTRKTTSETVRAVLD

SEQ ID NO: 162 - protein, 147 aa, synthetic construct
  REGION 1..147: note = Synthetic Polypeptide
KEFLLYLAGFVDGDGSIWAQIVPERAGRFKHRLRLYFTVAQKTQRRWFLDKLVDEIGVGYVVDQGSVSEYRLSEIKPLHNFLTQLQPFLKLKQKQANLVLKIIEQLPSAKESPDKFLEVCTWVDQIAALNDSKTRKTTSETVRAVLD

SEQ ID NO: 163 - protein, 147 aa, synthetic construct
  REGION 1..147: note = Synthetic Polypeptide
KEFLLYLAGFVDGDGSIWASITPEPTASFKHRLRLYFTVAQKTQRRWFLDKLVDEIGVGYVVDQGSVSEYRLSEIKPLHNFLTQLQPFLKLKQKQANLVLKIIEQLPSAKESPDKFLEVCTWVDQIAALNDSKTRKTTSETVRAVLD

SEQ ID NO: 164 - protein, 147 aa, synthetic construct
  REGION 1..147: note = Synthetic Polypeptide
KEFLLYLAGFVDGDGSIWASINPEPSYRFKHRLRLSFTVAQKTQRRWFLDKLVDEIGVGYVVDQGSVSEYRLSEIKPLHNFLTQLQPFLKLKQKQANLVLKIIEQLPSAKESPDKFLEVCTWVDQIAALNDSKTRKTTSETVRAVLD

SEQ ID NO: 165 - protein, 147 aa, synthetic construct
  REGION 1..147: note = Synthetic Polypeptide
KEFLLYLAGFVDGDGSIWASILPEHQYRFKHRLRLGFTVAQKTQRRWFLDKLVDEIGVGYVVDQGSVSEYRLSEIKPLHNFLTQLQPFLKLKQKQANLVLKIIEQLPSAKESPDKFLEVCTWVDQIAALNDSKTRKTTSETVRAVLD

SEQ ID NO: 166 - protein, 147 aa, synthetic construct
  REGION 1..147: note = Synthetic Polypeptide
KEFLLYLAGFVDGDGSIYAAIDPDQKYKFKHRLRLIFAVCQKTQRRWFLDKLVDEIGVGYVVDHGSVSEYRLSQIKPLHNFLTQLQPFLKLKQKQANLVLKIIEQLPSAKESPDKFLEVCTWVDQIAALNDSKTRKTTSETVRAVLD

SEQ ID NO: 167 - protein, 147 aa, synthetic construct
  REGION 1..147: note = Synthetic Polypeptide
KEFLLYLAGFVDGDGSIYATIEPAQRYKFKHRLRLKFAVSQKTQRRWFLDKLVDEIGVGYVADQGSVSEYRLSEIKPLHNFLTQLQPFLKLKQKQANLVLKIIEQLPSAKESPDKFLEVCTWVDQIAALNDSKTRKTTSETVRAVLD

SEQ ID NO: 168 - protein, 147 aa, synthetic construct
  REGION 1..147: note = Synthetic Polypeptide
KEFLLYLAGFVDGDGSIYATINPDQTNKFKHRLRLWFAVCQKTQRRWFLDKLVDEIGVGYVADTGSVSEYRLSQIKPLHNFLTQLQPFLKLKQKQANLVLKIIEQLPSAKESPDKFLEVCTWVDQIAALNDSKTRKTTSETVRAVLD

SEQ ID NO: 169 - protein, 147 aa, synthetic construct
  REGION 1..147: note = Synthetic Polypeptide
KEFLLYLAGFVDGDGSIYACIEPAQNSKFKHYLRLRFEVSQKTQRRWFLDKLVDEIGVGYVYDQGSVSSYRLSQIKPLHNFLTQLQPFLKLKQKQANLVLKIIEQLPSAKESPDKFLEVCTWVDQIAALNDSKTRKTTSETVRAVLD

SEQ ID NO: 170 - protein, 147 aa, synthetic construct
  REGION 1..147: note = Synthetic Polypeptide
KEFLLYLAGFVDGDGSIYASITPCQSYKFKHRLLLKFSVAQKTQRRWFLDKLVDEIGVGYVTDSGSVSEYRLSQIKPLHNFLTQLQPFLKLKQKQANLVLKIIEQLPSAKESPDKFLEVCTWVDQIAALNDSKTRKTTSETVRAVLD

SEQ ID NO: 171 - protein, 147 aa, synthetic construct
  REGION 1..147: note = Synthetic Polypeptide
KEFLLYLAGFVDGDGSIYATIMPEQTVKFKHRLRLFFEVAQKTQRRWFLDKLVDEIGVGYVYDQGSVSSYRLSQIKPLHNFLTQLQPFLKLKQKQANLVLKIIEQLPSAKESPDKFLEVCTWVDQIAALNDSKTRKTTSETVRAVLD

SEQ ID NO: 172 - protein, 147 aa, synthetic construct
  REGION 1..147: note = Synthetic Polypeptide
KEFLLYLAGFVDGDGSIYATIQPEQAPKFKHRLRLHFTVHQKTQRRWFLDKLVDEIGVGYVYDQGSVSEYRLSQIKPLHNFLTQLQPFLKLKQKQANLVLKIIEQLPSAKESPDKFLEVCTWVDQIAALNDSKTRKTTSETVRAVLD

SEQ ID NO: 173 - protein, 147 aa, synthetic construct
  REGION 1..147: note = Synthetic Polypeptide
KEFLLYLAGFVDGDGSIWATIEPSQTLKFKHRLRLHFSVYQKTQRRWFLDKLVDEIGVGYVYDDGSVSRYQLSQIKPLHNFLTQLQPFLKLKQKQANLVLKIIEQLPSAKESPDKFLEVCTWVDQIAALNDSKTRKTTSETVRAVLD

SEQ ID NO: 174 - protein, 147 aa, synthetic construct
  REGION 1..147: note = Synthetic Polypeptide
KEFLLYLAGFVDGDGSIYASITPCQSYKFKHRLLLKFSVAQKTQRRWFLDKLVDEIGVGYVTDSGSVSEYRLSEIKPLHNFLTQLQPFLKLKQKQANLVLKIIEQLPSAKESPDKFLEVCTWVDQIAALNDSKTRKTTSETVRAVLD

SEQ ID NO: 175 - protein, 147 aa, synthetic construct
  REGION 1..147: note = Synthetic Polypeptide
KEFLLYLAGFVDGDGSIYATIIPSQNLKFKHRLRLYFEVCQKTQRRWFLDKLVDEIGVGYVYDQGSVSSYRLSEIKPLHNFLTQLQPFLKLKQKQANLVLKIIEQLPSAKESPDKFLEVCTWVDQIAALNDSKTRKTTSETVRAVLD

SEQ ID NO: 176 - protein, 147 aa, synthetic construct
  REGION 1..147: note = Synthetic Polypeptide
KEFLLYLAGFVDGDGSIYASICPTQAAKFKHRLRLHFAVFQKTQRRWFLDKLVDEIGVGYVTDCGSVSEYRLSQIKPLHNFLTQLQPFLKLKQKQANLVLKIIEQLPSAKESPDKFLEVCTWVDQIAALNDSKTRKTTSETVRAVLD

SEQ ID NO: 177 - protein, 147 aa, synthetic construct
  REGION 1..147: note = Synthetic Polypeptide
KEFLLYLAGFVDGDGSIYASIEPAQSYKFKHRLQLKFAVAQKTQRRWFLDKLVDEIGVGYVCDIGSVSEYRLSQIKPLHNFLTQLQPFLKLKQKQANLVLKIIEQLPSAKESPDKFLEVCTWVDQIAALNDSKTRKTTSETVRAVLD

SEQ ID NO: 178 - protein, 147 aa, synthetic construct
  REGION 1..147: note = Synthetic Polypeptide
KEFLLYLAGFVDGDGSIYAAIMPTQSYKFKHRLRLAFSVSQKTQRRWFLDKLVDEIGVGYVTDAGSVSEYRLSQIKPLHNFLTQLQPFLKLKQKQANLVLKIIEQLPSAKESPDKFLEVCTWVDQIAALNDSKTRKTTSETVRAVLD

SEQ ID NO: 179 - protein, 147 aa, synthetic construct
  REGION 1..147: note = Synthetic Polypeptide
KEFLLYLAGFVDGDGSIYATITPNQRTKFKHQLKLAFAVYQKTQRRWFLDKLVDEIGVGYVYDQGSVSCYRLSEIKPLHNFLTQLQPFLKLKQKQANLVLKIIEQLPSAKESPDKFLEVCTWVDQIAALNDSKTRKTTSETVRAVLD

SEQ ID NO: 180 - protein, 147 aa, synthetic construct
  REGION 1..147: note = Synthetic Polypeptide
KEFLLYLAGFVDGDGSIYAAIVPVQSTKFKHRLRLYFTVHQKTQRRWFLDKLVDEIGVGYVYDQGSVSEYRLSQIKPLHNFLTQLQPFLKLKQKQANLVLKIIEQLPSAKESPDKFLEVCTWVDQIAALNDSKTRKTTSETVRAVLD

SEQ ID NO: 181 - protein, 147 aa, synthetic construct
  REGION 1..147: note = Synthetic Polypeptide
KEFLLYLAGFVDGDGSIYATICPVQSLKFKHRLRLFFAVCQKTQRRWFLDKLVDEIGVGYVVDHGSVSEYRLSEIKPLHNFLTQLQPFLKLKQKQANLVLKIIEQLPSAKESPDKFLEVCTWVDQIAALNDSKTRKTTSETVRAVLD

SEQ ID NO: 182 - protein, 147 aa, synthetic construct
  REGION 1..147: note = Synthetic Polypeptide
KEFLLYLAGFVDGDGSIWASILPEQRNKFKHRLKLGFSVSQKTQRRWFLDKLVDEIGVGYVVDQGSVSEYRLSQIKPLHNFLTQLQPFLKLKQKQANLVLKIIEQLPSAKESPDKFLEVCTWVDQIAALNDSKTRKTTSETVRAVLD

SEQ ID NO: 183 - protein, 147 aa, synthetic construct
  REGION 1..147: note = Synthetic Polypeptide
KEFLLYLAGFVDGDGSIYATIHPCQCTKFKHRLRLYFEVYQKTQRRWFLDKLVDEIGVGYVYDQGSVSSYRLSQIKPLHNFLTQLQPFLKLKQKQANLVLKIIEQLPSAKESPDKFLEVCTWVDQIAALNDSKTRKTTSETVRAVLD

SEQ ID NO: 184 - protein, 147 aa, synthetic construct
  REGION 1..147: note = Synthetic Polypeptide
KEFLLYLAGFVDGDGSIYATIDPDQRQKFKHRLRLKFSVSQKTQRRWFLDKLVDEIGVGYVVDGGSVSEYRLSEIKPLHNFLTQLQPFLKLKQKQANLVLKIIEQLPSAKESPDKFLEVCTWVDQIAALNDSKTRKTTSETVRAVLD

SEQ ID NO: 185 - protein, 147 aa, synthetic construct
  REGION 1..147: note = Synthetic Polypeptide
KEFLLYLAGFVDGDGSIYAAIVPDQAPKFKHRLRLFFAVSQKTQRRWFLDKLVDEIGVGYVADQGSVSEYRLSQIKPLHNFLTQLQPFLKLKQKQANLVLKIIEQLPSAKESPDKFLEVCTWVDQIAALNDSKTRKTTSETVRAVLD

SEQ ID NO: 186 - protein, 147 aa, synthetic construct
  REGION 1..147: note = Synthetic Polypeptide
KEFLLYLAGFVDGDGSIYASILPEQRNKFKHRLKLSFSVCQKTQRRWFLDKLVDEIGVGYVVDQGSVSEYRLSEIKPLHNFLTQLQPFLKLKQKQANLVLKIIEQLPSAKESPDKFLEVCTWVDQIAALNDSKTRKTTSETVRAVLD

SEQ ID NO: 187 - protein, 147 aa, synthetic construct
  REGION 1..147: note = Synthetic Polypeptide
KEFLLYLAGFVDGDGSIYAAIVPDQAPKFKHRLRLFFAVSQKTQRRWFLDKLVDEIGVGYVADQGSVSEYRLSEIKPLHNFLTQLQPFLKLKQKQANLVLKIIEQLPSAKESPDKFLEVCTWVDQIAALNDSKTRKTTSETVRAVLD

SEQ ID NO: 188 - protein, 147 aa, synthetic construct
  REGION 1..147: note = Synthetic Polypeptide
KEFLLYLAGFVDGDGSIYACICPDQGYKFKHRLTLKFSVAQKTQRRWFLDKLVDEIGVGYVLDQGSVSEYRLSEIKPLHNFLTQLQPFLKLKQKQANLVLKIIEQLPSAKESPDKFLEVCTWVDQIAALNDSKTRKTTSETVRAVLD

SEQ ID NO: 189 - protein, 147 aa, synthetic construct
  REGION 1..147: note = Synthetic Polypeptide
KEFLLYLAGFVDGDGSIYACILPEQKTKFKHRLKLSFTVCQKTQRRWFLDKLVDEIGVGYVVDQGSVSEYRLSQIKPLHNFLTQLQPFLKLKQKQANLVLKIIEQLPSAKESPDKFLEVCTWVDQIAALNDSKTRKTTSETVRAVLD

SEQ ID NO: 190 - protein, 147 aa, synthetic construct
  REGION 1..147: note = Synthetic Polypeptide
KEFLLYLAGFVDGDGSIFARIFKGQHWKFKHYIRLTFTVAQKTQRRWFLDKLVDEIGVGYVTDWGSVSHYYLSEIKPLHNFLTQLQPFLKLKQKQANLVLKIIEQLPSAKESPDKFLEVCTWVDQIAALNDSKTRKTTSETVRAVLD

SEQ ID NO: 191 - protein, 147 aa, synthetic construct
  REGION 1..147: note = Synthetic Polypeptide
KEFLLYLAGFVDGDGSIYARIFKGQHWKFKHYIRLTFCVRQKTQRRWFLDKLVDEIGVGYVTDSGSVSAYYLSEIKPLHNFLTQLQPFLKLKQKQANLVLKIIEQLPSAKESPDKFLEVCTWVDQIAALNDSKTRKTTSETVRAVLD

SEQ ID NO: 192 - protein, 147 aa, synthetic construct
  REGION 1..147: note = Synthetic Polypeptide
KEFLLYLAGFVDGDGSIYARIFKGQHWKFKHHIRLTFHVSQKTQRRWFLDKLVDEIGVGYVTDWGSVSGYYLSEIKPLHNFLTQLQPFLKLKQKQANLVLKIIEQLPSAKESPDKFLEVCTWVDQIAALNDSKTRKTTSETVRAVLD

SEQ ID NO: 193 - protein, 147 aa, synthetic construct
  REGION 1..147: note = Synthetic Polypeptide
KEFLLYLAGFVDGDGSIYARIEPRQTAKFKHYLRLTFHVSQKTQRRWFLDKLVDEIGVGYVTDWGSVSGYYLSEIKPLHNFLTQLQPFLKLKQKQANLVLKIIEQLPSAKESPDKFLEVCTWVDQIAALNDSKTRKTTSETVRAVLD

SEQ ID NO: 194 - protein, 147 aa, synthetic construct
  REGION 1..147: note = Synthetic Polypeptide
KEFLLYLAGFVDGDGSIYARIEPRQTAKFKHYLRLTFHVSQKTQRRWFLDKLVDEIGVGYVVDQGSVSQYFLSEIKPLHNFLTQLQPFLKLKQKQANLVLKIIEQLPSAKESPDKFLEVCTWVDQIAALNDSKTRKTTSETVRAVLD

SEQ ID NO: 195 - protein, 147 aa, synthetic construct
  REGION 1..147: note = Synthetic Polypeptide
KEFLLYLAGFVDGDGSIYARIEPRQNFKFKHTLRLTFFVSQKTQRRWFLDKLVDEIGVGYVTDWGSVSGYYLSQIKPLHNFLTQLQPFLKLKQKQANLVLKIIEQLPSAKESPDKFLEVCTWVDQIAALNDSKTRKTTSETVRAVLD

SEQ ID NO: 196 - protein, 147 aa, synthetic construct
  REGION 1..147: note = Synthetic Polypeptide
KEFLLYLAGFVDGDGSIYARIEPRQGNKFKHYLRLTFNVCQKTQRRWFLDKLVDEIGVGYVIDRGSVSDYYLSEIKPLHNFLTQLQPFLKLKQKQANLVLKIIEQLPSAKESPDKFLEVCTWVDQIAALNDSKTRKTTSETVRAVLD

SEQ ID NO: 197 - protein, 147 aa, synthetic construct
  REGION 1..147: note = Synthetic Polypeptide
KEFLLYLAGFVDGDGSIYARIEPRQTAKFKHYLRLTFHVSQKTQRRWFLDKLVDEIGVGYVVDQGSVSQYFLSQIKPLHNFLTQLQPFLKLKQKQANLVLKIIEQLPSAKESPDKFLEVCTWVDQIAALNDSKTRKTTSETVRAVLD

SEQ ID NO: 198 - protein, 147 aa, synthetic construct
  REGION 1..147: note = Synthetic Polypeptide
KEFLLYLAGFVDGDGSIYARIEPRQTAKFKHYLRLTFHVSQKTQRRWFLDKLVDEIGVGYVVDQGSVSQYYLSQIKPLHNFLTQLQPFLKLKQKQANLVLKIIEQLPSAKESPDKFLEVCTWVDQIAALNDSKTRKTTSETVRAVLD

SEQ ID NO: 199 - protein, 147 aa, synthetic construct
  REGION 1..147: note = Synthetic Polypeptide
KEFLLYLAGFVDGDGSIYARIYPKQSSKFKHHLRLTFHVSQKTQRRWFLDKLVDEIGVGYVYDSGSVSQYYLSEIKPLHNFLTQLQPFLKLKQKQANLVLKIIEQLPSAKESPDKFLEVCTWVDQIAALNDSKTRKTTSETVRAVLD

SEQ ID NO: 200 - protein, 147 aa, synthetic construct
  REGION 1..147: note = Synthetic Polypeptide
KEFLLYLAGFVDGDGSIYARIEPEQTAKFKHMLRLTFRVSQKTQRRWFLDKLVDEIGVGYVNDSGSVSGYYLSQIKPLHNFLTQLQPFLKLKQKQANLVLKIIEQLPSAKESPDKFLEVCTWVDQIAALNDSKTRKTTSETVRAVLD

SEQ ID NO: 201 - protein, 147 aa, synthetic construct; identical to SEQ ID NO: 197
  REGION 1..147: note = Synthetic Polypeptide

SEQ ID NO: 202 - protein, 147 aa, synthetic construct
  REGION 1..147: note = Synthetic Polypeptide
KEFLLYLAGFVDGDGSIYARIEPKQTAKFKHHLCLRFHVSQKTQRRWFLDKLVDEIGVGYVVDHGSVSQYFLSQIKPLHNFLTQLQPFLKLKQKQANLVLKIIEQLPSAKESPDKFLEVCTWVDQIAALNDSKTRKTTSETVRAVLD

SEQ ID NO: 203 - protein, 147 aa, synthetic construct; identical to SEQ ID NO: 193
  REGION 1..147: note = Synthetic Polypeptide

SEQ ID NO: 204 - protein, 147 aa, synthetic construct
  REGION 1..147: note = Synthetic Polypeptide
KEFLLYLAGFVDGDGSIYARIEPRQRVKFKHFLRLTFHVSQKTQRRWFLDKLVDEIGVGYVTDWGSVSGYYLSEIKPLHNFLTQLQPFLKLKQKQANLVLKIIEQLPSAKESPDKFLEVCTWVDQIAALNDSKTRKTTSETVRAVLD

SEQ ID NO: 205 - protein, 147 aa, synthetic construct
  REGION 1..147: note = Synthetic Polypeptide
KEFLLYLAGFVDGDGSIYARIEPRQGCKFKHVLRLTFHVSQKTQRRWFLDKLVDEIGVGYVTDWGSVSGYYLSEIKPLHNFLTQLQPFLKLKQKQANLVLKIIEQLPSAKESPDKFLEVCTWVDQIAALNDSKTRKTTSETVRAVLD

SEQ ID NO: 206 - protein, 147 aa, synthetic construct
  REGION 1..147: note = Synthetic Polypeptide
KEFLLYLAGFVDGDGSIYARIEPRQVCKFKHILRLTFHVSQKTQRRWFLDKLVDEIGVGYVTDWGSVSGYYLSEIKPLHNFLTQLQPFLKLKQKQANLVLKIIEQLPSAKESPDKFLEVCTWVDQIAALNDSKTRKTTSETVRAVLD

SEQ ID NO: 207 - protein, 147 aa, synthetic construct
  REGION 1..147: note = Synthetic Polypeptide
KEFLLYLAGFVDGDGSIYARIEPRQCFKFKHCLRLTFHVSQKTQRRWFLDKLVDEIGVGYVTDWGSVSGYYLSEIKPLHNFLTQLQPFLKLKQKQANLVLKIIEQLPSAKESPDKFLEVCTWVDQIAALNDSKTRKTTSETVRAVLD

SEQ ID NO: 208 - protein, 147 aa, synthetic construct
  REGION 1..147: note = Synthetic Polypeptide
KEFLLYLAGFVDGDGSIYARIEPRQRFKFKHCLRLTFHVSQKTQRRWFLDKLVDEIGVGYVTDWGSVSGYYLSEIKPLHNFLTQLQPFLKLKQKQANLVLKIIEQLPSAKESPDKFLEVCTWVDQIAALNDSKTRKTTSETVRAVLD

SEQ ID NO: 209 - protein, 147 aa, synthetic construct
  REGION 1..147: note = Synthetic Polypeptide
KEFLLYLAGFVDGDGSIYARIEPRQFCKFKHILRLTFHVSQKTQRRWFLDKLVDEIGVGYVTDWGSVSGYYLSEIKPLHNFLTQLQPFLKLKQKQANLVLKIIEQLPSAKESPDKFLEVCTWVDQIAALNDSKTRKTTSETVRAVLD

SEQ ID NO: 210 - protein, 147 aa, synthetic construct
  REGION 1..147: note = Synthetic Polypeptide
KEFLLYLAGFVDGDGSIYARIEPRQAFKFKHALRLTFHVSQKTQRRWFLDKLVDEIGVGYVTDWGSVSGYYLSEIKPLHNFLTQLQPFLKLKQKQANLVLKIIEQLPSAKESPDKFLEVCTWVDQIAALNDSKTRKTTSETVRAVLD

SEQ ID NO: 211 - protein, 147 aa, synthetic construct
  REGION 1..147: note = Synthetic Polypeptide
KEFLLYLAGFVDGDGSIYARIEPRQTCKFKHILRLTFHVSQKTQRRWFLDKLVDEIGVGYVTDWGSVSGYYLSEIKPLHNFLTQLQPFLKLKQKQANLVLKIIEQLPSAKESPDKFLEVCTWVDQIAALNDSKTRKTTSETVRAVLD

SEQ ID NO: 212 - protein, 147 aa, synthetic construct
  REGION 1..147: note = Synthetic Polypeptide
KEFLLYLAGFVDGDGSIYARIEPRQCFKFKHGLRLTFHVSQKTQRRWFLDKLVDEIGVGYVTDWGSVSGYYLSEIKPLHNFLTQLQPFLKLKQKQANLVLKIIEQLPSAKESPDKFLEVCTWVDQIAALNDSKTRKTTSETVRAVLD

SEQ ID NO: 213 - protein, 147 aa, synthetic construct
  REGION 1..147: note = Synthetic Polypeptide
KEFLLYLAGFVDGDGSIYARIEPRQSSKFKHLLRLTFHVSQKTQRRWFLDKLVDEIGVGYVTDWGSVSGYYLSEIKPLHNFLTQLQPFLKLKQKQANLVLKIIEQLPSAKESPDKFLEVCTWVDQIAALNDSKTRKTTSETVRAVLD

SEQ ID NO: 214 - protein, 147 aa, synthetic construct
  REGION 1..147: note = Synthetic Polypeptide
KEFLLYLAGFVDGDGSIYARIYLGQHWKFKHYVRLTFHVSQKTQRRWFLDKLVDEIGVGYVTDWGSVSGYYLSEIKPLHNFLTQLQPFLKLKQKQANLVLKIIEQLPSAKESPDKFLEVCTWVDQIAALNDSKTRKTTSETVRAVLD

SEQ ID NO: 215 - protein, 147 aa, synthetic construct
  REGION 1..147: note = Synthetic Polypeptide
KEFLLYLAGFVDGDGSIYARIYLGQHYKFKHYIRLTFHVSQKTQRRWFLDKLVDEIGVGYVTDWGSVSGYYLSEIKPLHNFLTQLQPFLKLKQKQANLVLKIIEQLPSAKESPDKFLEVCTWVDQIAALNDSKTRKTTSETVRAVLD

SEQ ID NO: 216 - protein, 147 aa, synthetic construct
  REGION 1..147: note = Synthetic Polypeptide
KEFLLYLAGFVDGDGSIYARIYNAQYYKFKHYIRLTFHVSQKTQRRWFLDKLVDEIGVGYVTDWGSVSGYYLSEIKPLHNFLTQLQPFLKLKQKQANLVLKIIEQLPSAKESPDKFLEVCTWVDQIAALNDSKTRKTTSETVRAVLD

SEQ ID NO: 217 - protein, 147 aa, synthetic construct
  REGION 1..147: note = Synthetic Polypeptide
KEFLLYLAGFVDGDGSIYARIERRQNFKFKHHIRLTFHVSQKTQRRWFLDKLVDEIGVGYVTDWGSVSGYYLSEIKPLHNFLTQLQPFLKLKQKQANLVLKIIEQLPSAKESPDKFLEVCTWVDQIAALNDSKTRKTTSETVRAVLD

SEQ ID NO: 218 - protein, 147 aa, synthetic construct
  REGION 1..147: note = Synthetic Polypeptide
KEFLLYLAGFVDGDGSIYARIERRQCVKFKHYLRLTFHVSQKTQRRWFLDKLVDEIGVGYVTDWGSVSGYYLSEIKPLHNFLTQLQPFLKLKQKQANLVLKIIEQLPSAKESPDKFLEVCTWVDQIAALNDSKTRKTTSETVRAVLD

SEQ ID NO: 219 - protein, 147 aa, synthetic construct
  REGION 1..147: note = Synthetic Polypeptide
KEFLLYLAGFVDGDGSIYARIEYRQGAKFKHYLRLTFHVSQKTQRRWFLDKLVDEIGVGYVTDWGSVSGYYLSEIKPLHNFLTQLQPFLKLKQKQANLVLKIIEQLPSAKESPDKFLEVCTWVDQIAALNDSKTRKTTSETVRAVLD

SEQ ID NO: 220 - protein, 147 aa, synthetic construct
  REGION 1..147: note = Synthetic Polypeptide
KEFLLYLAGFVDGDGSIYARIEPRQSGKFKHYIRLTFHVSQKTQRRWFLDKLVDEIGVGYVTDWGSVSGYYLSEIKPLHNFLTQLQPFLKLKQKQANLVLKIIEQLPSAKESPDKFLEVCTWVDQIAALNDSKTRKTTSETVRAVLD

SEQ ID NO: 221 - protein, 147 aa, synthetic construct
  REGION 1..147: note = Synthetic Polypeptide
KEFLLYLAGFVDGDGSIYARIFKGQHWKFKHHIRLTFNVSQKTQRRWFLDKLVDEIGVGYVSDTGSQSNYYLSEIKPLHNFLTQLQPFLKLKQKQANLVLKIIEQLPSAKESPDKFLEVCTWVDQIAALNDSKTRKTTSETVRAVLD

SEQ ID NO: 222 - protein, 147 aa, synthetic construct
  REGION 1..147: note = Synthetic Polypeptide
KEFLLYLAGFVDGDGSIFARIFKGQHWKFKHHIRLTFNVSQKTQRRWFLDKLVDEIGVGYVNDYGSTSNYYLSEIKPLHNFLTQLQPFLKLKQKQANLVLKIIEQLPSAKESPDKFLEVCTWVDQIAALNDSKTRKTTSETVRAVLD

SEQ ID NO: 223 - protein, 147 aa, synthetic construct
  REGION 1..147: note = Synthetic Polypeptide
KEFLLYLAGFVDGDGSIFARIFKGQHWKFKHHIRLTFNVAQKTQRRWFLDKLVDEIGVGYVTDHGSNSNYYLSEIKPLHNFLTQLQPFLKLKQKQANLVLKIIEQLPSAKESPDKFLEVCTWVDQIAALNDSKTRKTTSETVRAVLD

SEQ ID NO: 224 - protein, 147 aa, synthetic construct
  REGION 1..147: note = Synthetic Polypeptide
KEFLLYLAGFVDGDGSIYARIFKGQHWKFKHHIRLTFNVTQKTQRRWFLDKLVDEIGVGYVSDYGSMSNYYLSEIKPLHNFLTQLQPFLKLKQKQANLVLKIIEQLPSAKESPDKFLEVCTWVDQIAALNDSKTRKTTSETVRAVLD

SEQ ID NO: 225 - protein, 147 aa, synthetic construct
  REGION 1..147: note = Synthetic Polypeptide
KEFLLYLAGFVDGDGSIYARIFKGQHWKFKHHIRLTFAVTQKTQRRWFLDKLVDEIGVGYVTDHGSCSNYYLSEIKPLHNFLTQLQPFLKLKQKQANLVLKIIEQLPSAKESPDKFLEVCTWVDQIAALNDSKTRKTTSETVRAVLD

SEQ ID NO: 226 - protein, 147 aa, synthetic construct
  REGION 1..147: note = Synthetic Polypeptide
KEFLLYLAGFVDGDGSIYARIFKGQHWKFKHHIRLTFNVSQKTQRRWFLDKLVDEIGVGYVGDYGSMSHYYLSEIKPLHNFLTQLQPFLKLKQKQANLVLKIIEQLPSAKESPDKFLEVCTWVDQIAALNDSKTRKTTSETVRAVLD

SEQ ID NO: 227 - protein, 147 aa, synthetic construct
  REGION 1..147: note = Synthetic Polypeptide
KEFLLYLAGFVDGDGSIYARIFKGQHWKFKHHIRLTFNVSQKTQRRWFLDKLVDEIGVGYVTDFGSQSQYYLSEIKPLHNFLTQLQPFLKLKQKQANLVLKIIEQLPSAKESPDKFLEVCTWVDQIAALNDSKTRKTTSETVRAVLD

SEQ ID NO: 228 - protein, 147 aa, synthetic construct
  REGION 1..147: note = Synthetic Polypeptide
KEFLLYLAGFVDGDGSIFARIFKGQHWKFKHHIRLTFNVTQKTQRRWFLDKLVDEIGVGYVSDYGSISNYYLSEIKPLHNFLTQLQPFLKLKQKQANLVLKIIEQLPSAKESPDKFLEVCTWVDQIAALNDSKTRKTTSETVRAVLD

SEQ ID NO: 229 - protein, 147 aa, synthetic construct
  REGION 1..147: note = Synthetic Polypeptide
KEFLLYLAGFVDGDGSIYARIFKGQHWKFKHHIRLTFNVTQKTQRRWFLDKLVDEIGVGYVIDYGSISNYYLSEIKPLHNFLTQLQPFLKLKQKQANLVLKIIEQLPSAKESPDKFLEVCTWVDQIAALNDSKTRKTTSETVRAVLD

SEQ ID NO: 230 - protein, 147 aa, synthetic construct
  REGION 1..147: note = Synthetic Polypeptide
KEFLLYLAGFVDGDGSIYARIFKGQHWKFKHHIRLTFNVTQKTQRRWFLDKLVDEIGVGYVTDYGSSSNYYLSEIKPLHNFLTQLQPFLKLKQKQANLVLKIIEQLPSAKESPDKFLEVCTWVDQIAALNDSKTRKTTSETVRAVLD

SEQ ID NO: 231 - protein, 147 aa, synthetic construct
  REGION 1..147: note = Synthetic Polypeptide
KEFLLYLAGFVDGDGSIFARIFKGQHWKFKHHIRLTFNVSQKTQRRWFLDKLVDEIGVGYVTDGGSSSNYYLSEIKPLHNFLTQLQPFLKLKQKQANLVLKIIEQLPSAKESPDKFLEVCTWVDQIAALNDSKTRKTTSETVRAVLD

SEQ ID NO: 232 - protein, 147 aa, synthetic construct
  REGION 1..147: note = Synthetic Polypeptide
KEFLLYLAGFVDGDGSIFARIFKGQHWKFKHHIRLTFNVSQKTQRRWFLDKLVDEIGVGYVYDHGSQSNYYLSEIKPLHNFLTQLQPFLKLKQKQANLVLKIIEQLPSAKESPDKFLEVCTWVDQIAALNDSKTRKTTSETVRAVLD

SEQ ID NO: 233 - protein, 147 aa, synthetic construct
  REGION 1..147: note = Synthetic Polypeptide
KEFLLYLAGFVDGDGSIYARIFKGQHWKFKHHIRLTFNVSQKTQRRWFLDKLVDEIGVGYVCDNGSNSNYYLSEIKPLHNFLTQLQPFLKLKQKQANLVLKIIEQLPSAKESPDKFLEVCTWVDQIAALNDSKTRKTTSETVRAVLD

SEQ ID NO: 234 - protein, 147 aa, synthetic construct
  REGION 1..147: note = Synthetic Polypeptide
KEFLLYLAGFVDGDGSIFARIFKGQHWKFKHHIRLTFNVSQKTQRRWFLDKLVDEIGVGYVADYGSTSNYYLSEIKPLHNFLTQLQPFLKLKQKQANLVLKIIEQLPSAKESPDKFLEVCTWVDQIAALNDSKTRKTTSETVRAVLD

SEQ ID NO: 235 - protein, 147 aa, synthetic construct
  REGION 1..147: note = Synthetic Polypeptide
KEFLLYLAGFVDGDGSIYARIFKGQHWKFKHHIRLTFCVSQKTQRRWFLDKLVDEIGVGYVADYGSMSNYYLSEIKPLHNFLTQLQPFLKLKQKQANLVLKIIEQLPSAKESPDKFLEVCTWVDQIAALNDSKTRKTTSETVRAVLD

SEQ ID NO: 236 - protein, 147 aa, synthetic construct
  REGION 1..147: note = Synthetic Polypeptide
KEFLLYLAGFVDGDGSIMARIFKGQHWKFKHYIRLTLCVRQKTQRRWFLDKLVDEIGVGYVCDSGSMSAYYLSEIKPLHNFLTQLQPFLKLKQKQANLVLKIIEQLPSAKESPDKFLEVCTWVDQIAALNDSKTRKTTSETVRAVLD

SEQ ID NO: 237 - protein, 147 aa, synthetic construct; identical to SEQ ID NO: 231
  REGION 1..147: note = Synthetic Polypeptide

SEQ ID NO: 238 - protein, 147 aa, synthetic construct; identical to SEQ ID NO: 192
  REGION 1..147: note = Synthetic Polypeptide

SEQ ID NO: 239 - protein, 147 aa, synthetic construct; identical to SEQ ID NO: 192
  REGION 1..147: note = Synthetic Polypeptide

SEQ ID NO: 240 - protein, 147 aa, synthetic construct; identical to SEQ ID NO: 192
  REGION 1..147: note = Synthetic Polypeptide

SEQ ID NO: 241 - protein, 147 aa, synthetic construct; identical to SEQ ID NO: 192
  REGION 1..147: note = Synthetic Polypeptide

SEQ ID NO: 242 - protein, 147 aa, synthetic construct; identical to SEQ ID NO: 192
  REGION 1..147: note = Synthetic Polypeptide

SEQ ID NO: 243 - protein, 147 aa, synthetic construct; identical to SEQ ID NO: 192
  REGION 1..147: note = Synthetic Polypeptide

SEQ ID NO: 244 - protein, 147 aa, synthetic construct; identical to SEQ ID NO: 192
  REGION 1..147: note = Synthetic Polypeptide

SEQ ID NO: 245 - protein, 147 aa, synthetic construct; identical to SEQ ID NO: 192
  REGION 1..147: note = Synthetic Polypeptide

SEQ ID NO: 246 - protein, 147 aa, synthetic construct; identical to SEQ ID NO: 192
  REGION 1..147: note = Synthetic Polypeptide

SEQ ID NO: 247 - protein, 147 aa, synthetic construct; identical to SEQ ID NO: 192
  REGION 1..147: note = Synthetic Polypeptide

SEQ ID NO: 248 - protein, 147 aa, synthetic construct; identical to SEQ ID NO: 192
  REGION 1..147: note = Synthetic Polypeptide

SEQ ID NO: 249 - protein, 147 aa, synthetic construct
  REGION 1..147: note = Synthetic Polypeptide
KEFLLYLAGFVDGDGSIYARIFKGQHWKFKHYIRLTFCVSQKTQRRWFLDKLVDEIGVGYVNDSGSCSNYYLSEIKPLHNFLTQLQPFLKLKQKQANLVLKIIEQLPSAKESPDKFLEVCTWVDQIAALNDSKTRKTTSETVRAVLD

SEQ ID NO: 250 - protein, 147 aa, synthetic construct; identical to SEQ ID NO: 249
  REGION 1..147: note = Synthetic Polypeptide

SEQ ID NO: 251 - protein, 147 aa, synthetic construct
  REGION 1..147: note = Synthetic Polypeptide
KEFLLYLAGFVDGDGSIYARIFKGQHWKFKHHIRLTFNVSQKTQRRWFLDKLVDEIGVGYVCDSGSQSNYYLSEIKPLHNFLTQLQPFLKLKQKQANLVLKIIEQLPSAKESPDKFLEVCTWVDQIAALNDSKTRKTTSETVRAVLD

SEQ ID NO: 252 - protein, 147 aa, synthetic construct
  REGION 1..147: note = Synthetic Polypeptide
KEFLLYLAGFVDGDGSIFARIFKGQHWKFKHHIRLTFCVSQKTQRRWFLDKLVDEIGVGYVVDNGSMSNYYLSEIKPLHNFLTQLQPFLKLKQKQANLVLKIIEQLPSAKESPDKFLEVCTWVDQIAALNDSKTRKTTSETVRAVLD

SEQ ID NO: 253 - protein, 147 aa, synthetic construct
  REGION 1..147: note = Synthetic Polypeptide
KEFLLYLAGFVDGDGSIYARIFKGQHWKFKHHIRLTFCVTQKTQRRWFLDKLVDEIGVGYVHDYGSCSNYYLSEIKPLHNFLTQLQPFLKLKQKQANLVLKIIEQLPSAKESPDKFLEVCTWVDQIAALNDSKTRKTTSETVRAVLD

SEQ ID NO: 254 - protein, 147 aa, synthetic construct; identical to SEQ ID NO: 194
  REGION 1..147: note = Synthetic Polypeptide

SEQ ID NO: 255 - protein, 147 aa, synthetic construct; identical to SEQ ID NO: 194
  REGION 1..147: note = Synthetic Polypeptide

SEQ ID NO: 256 - protein, 147 aa, synthetic construct; identical to SEQ ID NO: 194
  REGION 1..147: note = Synthetic Polypeptide

SEQ ID NO: 257 - protein, 147 aa, synthetic construct; identical to SEQ ID NO: 194
  REGION 1..147: note = Synthetic Polypeptide

SEQ ID NO: 258 - protein, 147 aa, synthetic construct; identical to SEQ ID NO: 197
  REGION 1..147: note = Synthetic Polypeptide

SEQ ID NO: 259 - protein, 147 aa, synthetic construct; identical to SEQ ID NO: 197
  REGION 1..147: note = Synthetic Polypeptide

SEQ ID NO: 260 - protein, 147 aa, synthetic construct; identical to SEQ ID NO: 197
  REGION 1..147: note = Synthetic Polypeptide

SEQ ID NO: 261 - protein, 147 aa, synthetic construct; identical to SEQ ID NO: 197
  REGION 1..147: note = Synthetic Polypeptide

SEQ ID NO: 262 - protein, 147 aa, synthetic construct; identical to SEQ ID NO: 197
  REGION 1..147: note = Synthetic Polypeptide

SEQ ID NO: 263 - protein, 147 aa, synthetic construct; identical to SEQ ID NO: 197
  REGION 1..147: note = Synthetic Polypeptide

SEQ ID NO: 264 - protein, 147 aa, synthetic construct; identical to SEQ ID NO: 197
  REGION 1..147: note = Synthetic Polypeptide

SEQ ID NO: 265 - protein, 147 aa, synthetic construct; identical to SEQ ID NO: 197
  REGION 1..147: note = Synthetic Polypeptide

SEQ ID NO: 266 - protein, 147 aa, synthetic construct; identical to SEQ ID NO: 197
  REGION 1..147: note = Synthetic Polypeptide

SEQ ID NO: 267 - protein, 147 aa, synthetic construct; identical to SEQ ID NO: 197
  REGION 1..147: note = Synthetic Polypeptide

SEQ ID NO: 268 - protein, 147 aa, synthetic construct; identical to SEQ ID NO: 197
  REGION 1..147: note = Synthetic Polypeptide

SEQ ID NO: 269 - protein, 147 aa, synthetic construct; identical to SEQ ID NO: 197
  REGION 1..147: note = Synthetic Polypeptide

SEQ ID NO: 270 - protein, 147 aa, synthetic construct; identical to SEQ ID NO: 197
  REGION 1..147: note = Synthetic Polypeptide

SEQ ID NO: 271 - protein, 147 aa, synthetic construct; identical to SEQ ID NO: 193
  REGION 1..147: note = Synthetic Polypeptide

SEQ ID NO: 272 - protein, 147 aa, synthetic construct
  REGION 1..147: note = Synthetic Polypeptide
KEFLLYLAGFVDGDGSIYACIEPKQTSKFKHRLCLRFHVSQKTQRRWFLDKLVDEIGVGYVHDNGSVSQYYLSEIKPLHNFLTQLQPFLKLKQKQANLVLKIIEQLPSAKESPDKFLEVCTWVDQIAALNDSKTRKTTSETVRAVLD

SEQ ID NO: 273 - protein, 147 aa, synthetic construct
  REGION 1..147: note = Synthetic Polypeptide
KEFLLYLAGFVDGDGSIYARIYPGQHYKFKHYLRLTFHVSQKTQRRWFLDKLVDEIGVGYVTDAGSVSQYFLSQIKPLHNFLTQLQPFLKLKQKQANLVLKIIEQLPSAKESPDKFLEVCTWVDQIAALNDSKTRKTTSETVRAVLD

SEQ ID NO: 274 - protein, 147 aa, synthetic construct
  REGION 1..147: note = Synthetic Polypeptide
KEFLLYLAGFVDGDGSIYARIEPRQTAKFKHYLRLTFHVSQKTQRRWFLDKLVDEIGVGYVIDAGSVSGYYLSEIKPLHNFLTQLQPFLKLKQKQANLVLKIIEQLPSAKESPDKFLEVCTWVDQIAALNDSKTRKTTSETVRAVLD

SEQ ID NO: 275 - protein, 147 aa, synthetic construct
  REGION 1..147: note = Synthetic Polypeptide
KEFLLYLAGFVDGDGSIYACIEPKQTSKFKHRLCLRFHVSQKTQRRWFLDKLVDEIGVGYVHDNGSVSQYYLSQIKPLHNFLTQLQPFLKLKQKQANLVLKIIEQLPSAKESPDKFLEVCTWVDQIAALNDSKTRKTTSETVRAVLD

SEQ ID NO: 276 - protein, 147 aa, synthetic construct
  REGION 1..147: note = Synthetic Polypeptide
KEFLLYLAGFVDGDGSIYARIEPRQTAKFKHQLRLTFHVSQKTQRRWFLDKLVDEIGVGYVTDWGSVSGYYLSQIKPLHNFLTQLQPFLKLKQKQANLVLKIIEQLPSAKESPDKFLEVCTWVDQIAALNDSKTRKTTSETVRAVLD

SEQ ID NO: 277 - protein, 147 aa, synthetic construct
  REGION 1..147: note = Synthetic Polypeptide
KEFLLYLAGFVDGDGSIYARIEPRQTVKFKHMLRLTFHVSQKTQRRWFLDKLVDEIGVGYVHDNGSVSQYYLSQIKPLHNFLTQLQPFLKLKQKQANLVLKIIEQLPSAKESPDKFLEVCTWVDQIAALNDSKTRKTTSETVRAVLD

SEQ ID NO: 278 - DNA, 6214 bp, synthetic construct
  misc_feature 1..6214: note = Synthetic Polynucleotide
  source 1..6214: mol_type = other DNA
cagcagctggcgtaatagcgaagaggcccgcaccgatcgcccttcccaacagttgcgcagcctgaatggcgaatggaattccagacgattgagcgtcaaaatgtaggtatttccatgagcgtttttcctgttgcaatggctggcggtaatattgttctggatattaccagcaaggccgatagtttgagttcttctactcaggcaagtgatgttattactaatcaaagaagtattgcgacaacggttaatttgcgtgatggacagactcttttactcggtggcctcactgattataaaaacacttctcaggattctggcgtaccgttcctgtctaaaatccctttaatcggcctcctgtttagctcccgctctgattctaacgaggaaagcacgttatacgtgctcgtcaaagcaaccatagtacgcgccctgtagcggcgcattaagcgcggcgggtgtggtggttacgcgcagcgtgaccgctacacttgccagcgccctagcgcccgctcctttcgctttcttcccttcctttctcgccacgttcgccggctttccccgtcaagctctaaatcgggggctccctttagggttccgatttagtgctttacggcacctcgaccccaaaaaacttgattagggtgatggttcacgtagtgggccatcgccctgatagacggtttttcgccctttgacgttggagtccacgttctttaatagtggactcttgttccaaactggaacaacactcaaccctatctcggtctattcttttgatttataagggattttgccgatttcggcctattggttaaaaaatgagctgatttaacaaaaatttaacgcgaattttaacaaaatattaacgcttacaatttaaatatttgcttatacaatcttcctgtttttggggcttttctgattatcaaccggggtacatatgattgacatgctagttttacgattaccgttcatcgccctgcgcgctcgctcgctcactgaggccgcccgggcaaagcccgggcgtcgggcgacctttggtcgcccggcctcagtgagcgagcgagcgcgcagagagggagtggaattcacgcgtggatctaatagtaatcaattacggggtcattagttcatagcccatatatggagttccgcgttacataacttacggtaaatggcccgcctggctgaccgcccaacgacccccgcccattgacgtcaataatgacgtatgttcccatagtaacgccaatagggactttccattgacgtcaatgggtggagtatttacggtaaactgcccacttggcagtacatcaagtgtatcatatgccaagtccgccccctattgacgtcaatgacggtaaatggcccgcctggcattatgcccagtacatgaccttacgggactttcctacttggcagtacatctacgtattagtcatcgctattaccatgttgatgcggttttggcagtacaccaatgggcgtggatagcggtttgactcacggggatttccaagtctccaccccattgacgtcaatgggagtttgtttggcaccaaaatcaacgggactttccaaaatgtcgtaataaccccgccccgttgacgcaaatgggcggtaggcgtgtacggtgggaggtctatataagcagagctcgtttagtgaaccgtcagatcactagaagctttattgcggtagtttatcacagttaaattgctaacgcagtcagtgcttctgacacaacagtctcgaacttaagctgcagaagttggtcgtgaggcactgggcaggtaagtatcaaggttacaagacaggtttaaggagaccaatagaaactgggcttgtcgagacagagaagactcttgcgtttctgataggcacctattggtcttactgacatccactttgcctttctctccacaggtgtccactcccagttcaattacagctcttaaggctagagtacttaatacgactcactataggctagccaccatggcaccgaagaagaagcgcaaggtgcatatgaatacaaaatataataaagagttcttactctacttagcagggtttgtagacggtgacggttccatctttgcccgtatctttaagggtcaacattggaagttcaagcactatattcgtttgaccttcacggtggctcagaagacacagcgccgttggttcctcgacaagctggtggacgagatcggtgtgggttacgtgactgactggggcagcgtgtcccattactatctgtccgagatcaagcctttgcataattttttaacacaactacaaccttttctaaaactaaaacaaaaacaagcaaatttagttttaaaaattattgaacaacttccgtcagcaaaagaatccccggacaaattcttagaagtttgtacatgggtggatcaaattgcagctctgaatgattcgaagacgcgtaaaacaacttctgaaaccgttcgtgctgtgctagacagtttaccaggatccgtgggaggtctatcgccatctcaggcatccagcgccgcatcctcggcttcctcaagcccgggttcagggatctccgaagcactcagagctggagcaggttccggcactggatacaacaaggaattcctgctctacctggcgggcttcgtcgacggggacggctccatctgggcctcgatcattcctgagcaaggttataagttcaagcacaggctgcgtctctctttcactgtcgctcagaagacacagcgccgttggttcctcgacaagctggtggacgagatcggtgtgggttacgtggttgaccagggcagcgtctccgagtacaggctgtccgagatcaagcctctgcacaacttcctgacccagctccagcccttcctgaagctcaagcagaagcaggccaacctcgtgctgaagatcatcgagcagctgccctccgccaaggaatccccggacaagttcctggaggtgtgcacctgggtggaccagatcgccgctctgaacgactccaagacccgcaagaccacttccgaaaccgtccgcgccgttctagacagtctctccgagaagaagaagtcgtccccctaaggtaccagcggccgcgactctagatcataatcagccataccacatttgtagaggttttacttgctttaaaaaacctcccacacctccccctgaacctgaaacataaaatgaatgcaattgttgttgttaacttgtttattgcagcttataatggttacaaataaagcaatagcatcacaaatttcacaaataaagcatttttttcactgcattctagttgtggtttgtccaaactcatcaatgtatcttaaggcgggaattgatctgaggaacccctagtgatggagttggccactccctctctgcgcgctcgctcgctcactgaggccgggcgaccaaaggtcgcccgacgcccgggcaaagcccgggcgtcgggcgacctttggtcgcccggcctcagtgagcgagcgagcgcgcagagagggagtggccaaccccccccccccccccccggcgattctcttgtttgctccagactctcaggcaatgacctgatagcctttgtagagacctctcaaaaatagctaccctctccggcatgaatttatcagctagaacggttgaatatcatattgatggtgatttgactgtctccggcctttctcacccgtttgaatctttacctacacattactcaggcattgcatttaaaatatatgagggttctaaaaatttttatccttgcgttgaaataaaggcttctcccgcaaaagtattacagggtcataatgtttttggtacaaccgatttagctttatgctctgaggctttattgcttaattttgctaattctttgccttgcctgtatgatttattggatgttggaattcctgatgcggtattttctccttacgcatctgtgcggtatttcacaccgcatatggtgcactctcagtacaatctgctctgatgccgcatagttaagccagccccgacacccgccaacacccgctgacgcgccctgacgggcttgtctgctcccggcatccgcttacagacaagctgtgaccgtctccgggagctgcatgtgtcagaggttttcaccgtcatcaccgaaacgcgcgagacgaaagggcctcgtgatacgcctatttttataggttaatgtcatgataataatggtttcttagacgtcaggtggcacttttcggggaaatgtgcgcggaacccctatttgtttatttttctaaatacattcaaatatgtatccgctcatgagacaataaccctgataaatgcttcaataatattgaaaaaggaagagtatgagtattcaacatttccgtgtcgcccttattcccttttttgcggcattttgccttcctgtttttgctcacccagaaacgctggtgaaagtaaaagatgctgaagatcagttgggtgcacgagtgggttacatcgaactggatctcaacagcggtaagatccttgagagttttcgccccgaagaacgttttccaatgatgagcacttttaaagttctgctatgtggcgcggtattatcccgtattgacgccgggcaagagcaactcggtcgccgcatacactattctcagaatgacttggttgagtactcaccagtcacagaaaagcatcttacggatggcatgacagtaagagaattatgcagtgctgccataaccatgagtgataacactgcggccaacttacttctgacaacgatcggaggaccgaaggagctaaccgcttttttgcacaacatgggggatcatgtaactcgccttgatcgttgggaaccggagctgaatgaagccataccaaacgacgagcgtgacaccacgatgcctgtagcaatggcaacaacgttgcgcaaactattaactggcgaactacttactctagcttcccggcaacaattaatagactggatggaggcggataaagttgcaggaccacttctgcgctcggcccttccggctggctggtttattgctgataaatctggagccggtgagcgtgggtctcgcggtatcattgcagcactggggccagatggtaagccctcccgtatcgtagttatctacacgacggggagtcaggcaactatggatgaacgaaatagacagatcgctgagataggtgcctcactgattaagcattggtaactgtcagaccaagtttactcatatatactttagattgatttaaaacttcatttttaatttaaaaggatctaggtgaagatcctttttgataatctcatgaccaaaatcccttaacgtgagttttcgttccactgagcgtcagaccccgtagaaaagatcaaaggatcttcttgagatcctttttttctgcgcgtaatctgctgcttgcaaacaaaaaaaccaccgctaccagcggtggtttgtttgccggatcaagagctaccaactctttttccgaaggtaactggcttcagcagagcgcagataccaaatactgtccttctagtgtagccgtagttaggccaccacttcaagaactctgtagcaccgcctacatacctcgctctgctaatcctgttaccagtggctgctgccagtggcgataagtcgtgtcttaccgggttggactcaagacgatagttaccggataaggcgcagcggtcgggctgaacggggggttcgtgcacacagcccagcttggagcgaacgacctacaccgaactgagatacctacagcgtgagctatgagaaagcgccacgcttcccgaagggagaaaggcggacaggtatccggtaagcggcagggtcggaacaggagagcgcacgagggagcttccagggggaaacgcctggtatctttatagtcctgtcgggtttcgccacctctgacttgagcgtcgatttttgtgatgctcgtcaggggggcggagcctatggaaaaacgccagcaacgcggcctttttacggttcctggccttttgctggccttttgctcacatgttctttcctgcgttatcccctgattctgtggataaccgtattaccgcctttgagtgagctgataccgctcgccgcagccgaacgaccgagcgcagcgagtcagtgagcgaggaagcggaagagcgcccaatacgcaaaccgcctctccccgcgcgttggccgattcattaatg

SEQ ID NO: 279 - DNA, 6214 bp, synthetic construct
  misc_feature 1..6214: note = Synthetic Polynucleotide
  source 1..6214: mol_type = other DNA
cagcagctggcgtaatagcgaagaggcccgcaccgatcgcccttcccaacagttgcgcagcctgaatggcgaatggaattccagacgattgagcgtcaaaatgtaggtatttccatgagcgtttttcctgttgcaatggctggcggtaatattgttctggatattaccagcaaggccgatagtttgagttcttctactcaggcaagtgatgttattactaatcaaagaagtattgcgacaacggttaatttgcgtgatggacagactcttttactcggtggcctcactgattataaaaacacttctcaggattctggcgtaccgttcctgtctaaaatccctttaatcggcctcctgtttagctcccgctctgattctaacgaggaaagcacgttatacgtgctcgtcaaagcaaccatagtacgcgccctgtagcggcgcattaagcgcggcgggtgtggtggttacgcgcagcgtgaccgctacacttgccagcgccctagcgcccgctcctttcgctttcttcccttcctttctcgccacgttcgccggctttccccgtcaagctctaaatcgggggctccctttagggttccgatttagtgctttacggcacctcgaccccaaaaaacttgattagggtgatggttcacgtagtgggccatcgccctgatagacggtttttcgccctttgacgttggagtccacgttctttaatagtggactcttgttccaaactggaacaacactcaaccctatctcggtctattcttttgatttataagggattttgccgatttcggcctattggttaaaaaatgagctgatttaacaaaaatttaacgcgaattttaacaaaatattaacgcttacaatttaaatatttgcttatacaatcttcctgtttttggggcttttctgattatcaaccggggtacatatgattgacatgctagttttacgattaccgttcatcgccctgcgcgctcgctcgctcactgaggccgcccgggcaaagcccgggcgtcgggcgacctttggtcgcccggcctcagtgagcgagcgagcgcgcagagagggagtggaattcacgcgtggatctaatagtaatcaattacggggtcattagttcatagcccatatatggagttccgcgttacataacttacggtaaatggcccgcctggctgaccgcccaacgacccccgcccattgacgtcaataatgacgtatgttcccatagtaacgccaatagggactttccattgacgtcaatgggtggagtatttacggtaaactgcccacttggcagtacatcaagtgtatcatatgccaagtccgccccctattgacgtcaatgacggtaaatggcccgcctggcattatgcccagtacatgaccttacgggactttcctacttggcagtacatctacgtattagtcatcgctattaccatgttgatgcggttttggcagtacaccaatgggcgtggatagcggtttgactcacggggatttccaagtctccaccccattgacgtcaatgggagtttgtttggcaccaaaatcaacgggactttccaaaatgtcgtaataaccccgccccgttgacgcaaatgggcggtaggcgtgtacggtgggaggtctatataagcagagctcgtttagtgaaccgtcagatcactagaagctttattgcggtagtttatcacagttaaattgctaacgcagtcagtgcttctgacacaacagtctcgaacttaagctgcagaagttggtcgtgaggcactgggcaggtaagtatcaaggttacaagacaggtttaaggagaccaatagaaactgggcttgtcgagacagagaagactcttgcgtttctgataggcacctattggtcttactgacatccactttgcctttctctccacaggtgtccactcccagttcaattacagctcttaaggctagagtacttaatacgactcactataggctagccaccatggcaccgaagaagaagcgcaaggtgcatatgaatacaaaatataataaagagttcttactctacttagcagggtttgtagacggtgacggttccatctatgcccgtatctttaagggtcaacattggaagttcaagcactatattcgtttgaccttctgtgtgcggcagaagacacagcgccgttggttcctcgacaagctggtggacgagatcggtgtgggttacgtgactgactctggcagcgtttccgcttactatctgtccgagatcaagcctttgcataattttttaacacaactacaaccttttctaaaactaaaacaaaaacaagcaaatttagttttaaaaattattgaacaacttccgtcagcaaaagaatccccggacaaattcttagaagtttgtacatgggtggatcaaattgcagctctgaatgattcgaagacgcgtaaaacaacttctgaaaccgttcgtgctgtgctagacagtttaccaggatccgtgggaggtctatcgccatctcaggcatccagcgccgcatcctcggcttcctcaagcccgggttcagggatctccgaagcactcagagctggagcaggttccggcactggatacaacaaggaattcctgctctacctggcgggcttcgtcgacggggacggctccatctgggcctcgatcattcctgagcaaggttataagttcaagcacaggctgcgtctctctttcactgtcgctcagaagacacagcgccgttggttcctcgacaagctggtggacgagatcggtgtgggttacgtggttgaccagggcagcgtctccgagtacaggctgtccgagatcaagcctctgcacaacttcctgacccagctccagcccttcctgaagctcaagcagaagcaggccaacctcgtgctgaagatcatcgagcagctgccctccgccaaggaatccccggacaagttcctggaggtgtgcacctgggtggaccagatcgccgctctgaacgactccaagacccgcaagaccacttccgaaaccgtccgcgccgttctagacagtctctccgagaagaagaagtcgtccccctaaggtaccagcggccgcgactctagatcataatcagccataccacatttgtagaggttttacttgctttaaaaaacctcccacacctccccctgaacctgaaacataaaatgaatgcaattgttgttgttaacttgtttattgcagcttataatggttacaaataaagcaatagcatcacaaatttcacaaataaagcatttttttcactgcattctagttgtggtttgtccaaactcatcaatgtatcttaaggcgggaattgatctgaggaacccctagtgatggagttggccactccctctctgcgcgctcgctcgctcactgaggccgggcgaccaaaggtcgcccgacgcccgggcaaagcccgggcgtcgggcgacctttggtcgcccggcctcagtgagcgagcgagcgcgcagagagggagtggccaaccccccccccccccccccggcgattctcttgtttgctccagactctcaggcaatgacctgatagcctttgtagagacctctcaaaaatagctaccctctccggcatgaatttatcagctagaacggttgaatatcatattgatggtgatttgactgtctccggcctttctcacccgtttgaatctttacctacacattactcaggcattgcatttaaaatatatgagggttctaaaaatttttatccttgcgttgaaataaaggcttctcccgcaaaagtattacagggtcataatgtttttggtacaaccgatttagctttatgctctgaggctttattgcttaattttgctaattctttgccttgcctgtatgatttattggatgttggaattcctgatgcggtattttctccttacgcatctgtgcggtatttcacaccgcatatggtgcactctcagtacaatctgctctgatgccgcatagttaagccagccccgacacccgccaacacccgctgacgcgccctgacgggcttgtctgctcccggcatccgcttacagacaagctgtgaccgtctccgggagctgcatgtgtcagaggttttcaccgtcatcaccgaaacgcgcgagacgaaagggcctcgtgatacgcctatttttataggttaatgtcatgataataatggtttcttagacgtcaggtggcacttttcggggaaatgtgcgcggaacccctatttgtttatttttctaaatacattcaaatatgtatccgctcatgagacaataaccctgataaatgcttcaataatattgaaaaaggaagagtatgagtattcaacatttccgtgtcgcccttattcccttttttgcggcattttgccttcctgtttttgctcacccagaaacgctggtgaaagtaaaagatgctgaagatcagttgggtgcacgagtgggttacatcgaactggatctcaacagcggtaagatccttgagagttttcgccccgaagaacgttttccaatgatgagcacttttaaagttctgctatgtggcgcggtattatcccgtattgacgccgggcaagagcaactcggtcgccgcatacactattctcagaatgacttggttgagtactcaccagtcacagaaaagcatcttacggatggcatgacagtaagagaattatgcagtgctgccataaccatgagtgataacactgcggccaacttacttctgacaacgatcggaggaccgaaggagctaaccgcttttttgcacaacatgggggatcatgtaactcgccttgatcgttgggaaccggagctgaatgaagccataccaaacgacgagcgtgacaccacgatgcctgtagcaatggcaacaacgttgcgcaaactattaactggcgaactacttactctagcttcccggcaacaattaatagactggatggaggcggataaagttgcaggaccacttctgcgctcggcccttccggctggctggtttattgctgataaatctggagccggtgagcgtgggtctcgcggtatcattgcagcactggggccagatggtaagccctcccgtatcgtagttatctacacgacggggagtcaggcaactatggatgaacgaaatagacagatcgctgagataggtgcctcactgattaagcattggtaactgtcagaccaagtttactcatatatactttagattgatttaaaacttcatttttaatttaaaaggatctaggtgaagatcctttttgataatctcatgaccaaaatcccttaacgtgagttttcgttccactgagcgtcagaccccgtagaaaagatcaaaggatcttcttgagatcctttttttctgcgcgtaatctgctgcttgcaaacaaaaaaaccaccgctaccagcggtggtttgtttgccggatcaagagctaccaactctttttccgaaggtaactggcttcagcagagcgcagataccaaatactgtccttctagtgtagccgtagttaggccaccacttcaagaactctgtagcaccgcctacatacctcgctctgctaatcctgttaccagtggctgctgccagtggcgataagtcgtgtcttaccgggttggactcaagacgatagttaccggataaggcgcagcggtcgggctgaacggggggttcgtgcacacagcccagcttggagcgaacgacctacaccgaactgagatacctacagcgtgagctatgagaaagcgccacgcttcccgaagggagaaaggcggacaggtatccggtaagcggcagggtcggaacaggagagcgcacgagggagcttccagggggaaacgcctggtatctttatagtcctgtcgggtttcgccacctctgacttgagcgtcgatttttgtgatgctcgtcaggggggcggagcctatggaaaaacgccagcaacgcggcctttttacggttcctggccttttgctggccttttgctcacatgttctttcctgcgttatcccctgattctgtggataaccgtattaccgcctttgagtgagctgataccgctcgccgcagccgaacgaccgagcgcagcgagtcagtgagcgaggaagcggaagagcgcccaatacgcaaaccgcctctccccgcgcgttggccgattcattaatg

SEQ ID NO: 280 - DNA, 5888 bp, synthetic construct
  misc_feature 1..5888: note = Synthetic Polynucleotide
  source 1..5888: mol_type = other DNA
cagcagctggcgtaatagcgaagaggcccgcaccgatcgcccttcccaacagttgcgcagcctgaatggcgaatggaattccagacgattgagcgtcaaaatgtaggtatttccatgagcgtttttcctgttgcaatggctggcggtaatattgttctggatattaccagcaaggccgatagtttgagttcttctactcaggcaagtgatgttattactaatcaaagaagtattgcgacaacggttaatttgcgtgatggacagactcttttactcggtggcctcactgattataaaaacacttctcaggattctggcgtaccgttcctgtctaaaatccctttaatcggcctcctgtttagctcccgctctgattctaacgaggaaagcacgttatacgtgctcgtcaaagcaaccatagtacgcgccctgtagcggcgcattaagcgcggcgggtgtggtggttacgcgcagcgtgaccgctacacttgccagcgccctagcgcccgctcctttcgctttcttcccttcctttctcgccacgttcgccggctttccccgtcaagctctaaatcgggggctccctttagggttccgatttagtgctttacggcacctcgaccccaaaaaacttgattagggtgatggttcacgtagtgggccatcgccctgatagacggtttttcgccctttgacgttggagtccacgttctttaatagtggactcttgttccaaactggaacaacactcaaccctatctcggtctattcttttgatttataagggattttgccgatttcggcctattggttaaaaaatgagctgatttaacaaaaatttaacgcgaattttaacaaaatattaacgtttacaatttaaatatttgcttatacaatcttcctgtttttggggcttttctgattatcaaccggggtacatatgattgacatgctagttttacgattaccgttcatcgccctgcgcgctcgctcgctcactgaggccgcccgggcaaagcccgggcgtcgggcgacctttggtcgcccggcctcagtgagcgagcgagcgcgcagagagggagtggaattcacgcgtgggccccagaagcctggtggttgtttgtccttctcaggggaaaagtgaggcggccccttggaggaaggggccgggcagaatgatctaatcggattccaagcagctcaggggattgtctttttctagcaccttcttgccactcctaagcgtcctccgtgaccccggctgggatttagcctggtgctgtgtcagccccgggctcccaggggcttcccagtggtccccaggaaccctcgacagggccagggcgtctctctcgtccagcaagggcagggacgggccacaggccaagggcaagctttattgcggtagtttatcacagttaaattgctaacgcagtcagtgcttctgacacaacagtctcgaacttaagctgcagaagttggtcgtgaggcactgggcaggtaagtatcaaggttacaagacaggtttaaggagaccaatagaaactgggcttgtcgagacagagaagactcttgcgtttctgataggcacctattggtcttactgacatccactttgcctttctctccacaggtgtccactcccagttcaattacagctcttaaggctagagtacttaatacgactcactataggctagccaccatggcaccgaagaagaagcgcaaggtgcatatgaatacaaaatataataaagagttcttactctacttagcagggtttgtagacggtgacggttccatctttgcccgtatctttaagggtcaacattggaagttcaagcactatattcgtttgaccttcacggtggctcagaagacacagcgccgttggttcctcgacaagctggtggacgagatcggtgtgggttacgtgactgactggggcagcgtgtcccattactatctgtccgagatcaagcctttgcataattttttaacacaactacaaccttttctaaaactaaaacaaaaacaagcaaatttagttttaaaaattattgaacaacttccgtcagcaaaagaatccccggacaaattcttagaagtttgtacatgggtggatcaaattgcagctctgaatgattcgaagacgcgtaaaacaacttctgaaaccgttcgtgctgtgctagacagtttaccaggatccgtgggaggtctatcgccatctcaggcatccagcgccgcatcctcggcttcctcaagcccgggttcagggatctccgaagcactcagagctggagcaggttccggcactggatacaacaaggaattcctgctctacctggcgggcttcgtcgacggggacggctccatctgggcctcgatcattcctgagcaaggttataagttcaagcacaggctgcgtctctctttcactgtcgctcagaagacacagcgccgttggttcctcgacaagctggtggacgagatcggtgtgggttacgtggttgaccagggcagcgtctccgagtacaggctgtccgagatcaagcctctgcacaacttcctgacccagctccagcccttcctgaagctcaagcagaagcaggccaacctcgtgctgaagatcatcgagcagctgccctccgccaaggaatccccggacaagttcctggaggtgtgcacctgggtggaccagatcgccgctctgaacgactccaagacccgcaagaccacttccgaaaccgtccgcgccgttctagacagtctctccgagaagaagaagtcgtccccctaagcggccgcgactctagatcataatcagccataccacatttgtagaggttttacttgctttaaaaaacctcccacacctccccctgaacctgaaacataaaatgaatgcaattgttgttgttaacttgtttattgcagcttataatggttacaaataaagcaatagcatcacaaatttcacaaataaagcatttttttcactgcattctagttgtggtttgtccaaactcatcaatgtatcttaaggcgggaattgatctaggaacccctagtgatggagttggccactccctctctgcgcgctcgctcgctcactgaggccgcccgggcaaagcccgggcgtcgggcgacctttggtcgcccggcctcagtgagcgagcgagcgcgcagagagggagtggccaaccccccccccccccccccggcgattctcttgtttgctccagactctcaggcaatgacctgatagcctttgtagagacctctcaaaaatagctaccctctccggcatgaatttatcagctagaacggttgaatatcatattgatggtgatttgactgtctccggcctttctcacccgtttgaatctttacctacacattactcaggcattgcatttaaaatatatgagggttctaaaaatttttatccttgcgttgaaataaaggcttctcccgcaaaagtattacagggtcataatgtttttggtacaaccgatttagctttatgctctgaggctttattgcttaattttgctaattctttgccttgcctgtatgatttattggatgttggaattcctgatgcggtattttctccttacgcatctgtgcggtatttcacaccgcatatggtgcactctcagtacaatctgctctgatgccgcatagttaagccagccccgacacccgccaacacccgctgacgcgccctgacgggcttgtctgctcccggcatccgcttacagacaagctgtgaccgtctccgggagctgcatgtgtcagaggttttcaccgtcatcaccgaaacgcgcgagacgaaagggcctcgtgatacgcctatttttataggttaatgtcatgataataatggtttcttagacgtcaggtggcacttttcggggaaatgtgcgcggaacccctatttgtttatttttctaaatacattcaaatatgtatccgctcatgagacaataaccctgataaatgcttcaataatattgaaaaaggaagagtatgagtattcaacatttccgtgtcgcccttattcccttttttgcggcattttgccttcctgtttttgctcacccagaaacgctggtgaaagtaaaagatgctgaagatcagttgggtgcacgagtgggttacatcgaactggatctcaacagcggtaagatccttgagagttttcgccccgaagaacgttttccaatgatgagcacttttaaagttctgctatgtggcgcggtattatcccgtattgacgccgggcaagagcaactcggtcgccgcatacactattctcagaatgacttggttgagtactcaccagtcacagaaaagcatcttacggatggcatgacagtaagagaattatgcagtgctgccataaccatgagtgataacactgcggccaacttacttctgacaacgatcggaggaccgaaggagctaaccgcttttttgcacaacatgggggatcatgtaactcgccttgatcgttgggaaccggagctgaatgaagccataccaaacgacgagcgtgacaccacgatgcctgtagcaatggcaacaacgttgcgcaaactattaactggcgaactacttactctagcttcccggcaacaattaatagactggatggaggcggataaagttgcaggaccacttctgcgctcggcccttccggctggctggtttattgctgataaatctggagccggtgagcgtgggtctcgcggtatcattgcagcactggggccagatggtaagccctcccgtatcgtagttatctacacgacggggagtcaggcaactatggatgaacgaaatagacagatcgctgagataggtgcctcactgattaagcattggtaactgtcagaccaagtttactcatatatactttagattgatttaaaacttcatttttaatttaaaaggatctaggtgaagatcctttttgataatctcatgaccaaaatcccttaacgtgagttttcgttccactgagcgtcagaccccgtagaaaagatcaaaggatcttcttgagatcctttttttctgcgcgtaatctgctgcttgcaaacaaaaaaaccaccgctaccagcggtggtttgtttgccggatcaagagctaccaactctttttccgaaggtaactggcttcagcagagcgcagataccaaatactgtccttctagtgtagccgtagttaggccaccacttcaagaactctgtagcaccgcctacatacctcgctctgctaatcctgttaccagtggctgctgccagtggcgataagtcgtgtcttaccgggttggactcaagacgatagttaccggataaggcgcagcggtcgggctgaacggggggttcgtgcacacagcccagcttggagcgaacgacctacaccgaactgagatacctacagcgtgagctatgagaaagcgccacgcttcccgaagggagaaaggcggacaggtatccggtaagcggcagggtcggaacaggagagcgcacgagggagcttccagggggaaacgcctggtatctttatagtcctgtcgggtttcgccacctctgacttgagcgtcgatttttgtgatgctcgtcaggggggcggagcctatggaaaaacgccagcaacgcggcctttttacggttcctggccttttgctggccttttgctcacatgttctttcctgcgttatcccctgattctgtggataaccgtattaccgcctttgagtgagctgataccgctcgccgcagccgaacgaccgagcgcagcgagtcagtgagcgaggaagcggaagagcgcccaatacgcaaaccgcctctccccgcgcgttggccgattcattaatg

SEQ ID NO: 281 - DNA, 5888 bp, synthetic construct
  misc_feature 1..5888: note = Synthetic Polynucleotide
  source 1..5888: mol_type = other DNA
cagcagctggcgtaatagcgaagaggcccgcaccgatcgcccttcccaacagttgcgcagcctgaatggcgaatggaattccagacgattgagcgtcaaaatgtaggtatttccatgagcgtttttcctgttgcaatggctggcggtaatattgttctggatattaccagcaaggccgatagtttgagttcttctactcaggcaagtgatgttattactaatcaaagaagtattgcgacaacggttaatttgcgtgatggacagactcttttactcggtggcctcactgattataaaaacacttctcaggattctggcgtaccgttcctgtctaaaatccctttaatcggcctcctgtttagctcccgctctgattctaacgaggaaagcacgttatacgtgctcgtcaaagcaaccatagtacgcgccctgtagcggcgcattaagcgcggcgggtgtggtggttacgcgcagcgtgaccgctacacttgccagcgccctagcgcccgctcctttcgctttcttcccttcctttctcgccacgttcgccggctttccccgtcaagctctaaatcgggggctccctttagggttccgatttagtgctttacggcacctcgaccccaaaaaacttgattagggtgatggttcacgtagtgggccatcgccctgatagacggtttttcgccctttgacgttggagtccacgttctttaatagtggactcttgttccaaactggaacaacactcaaccctatctcggtctattcttttgatttataagggattttgccgatttcggcctattggttaaaaaatgagctgatttaacaaaaatttaacgcgaattttaacaaaatattaacgtttacaatttaaatatttgcttatacaatcttcctgtttttggggcttttctgattatcaaccggggtacatatgattgacatgctagttttacgattaccgttcatcgccctgcgcgctcgctcgctcactgaggccgcccgggcaaagcccgggcgtcgggcgacctttggtcgcccggcctcagtgagcgagcgagcgcgcagagagggagtggaattcacgcgtgggccccagaagcctggtggttgtttgtccttctcaggggaaaagtgaggcggccccttggaggaaggggccgggcagaatgatctaatcggattccaagcagctcaggggattgtctttttctagcaccttcttgccactcctaagcgtcctccgtgaccccggctgggatttagcctggtgctgtgtcagccccgggctcccaggggcttcccagtggtccccaggaaccctcgacagggccagggcgtctctctcgtccagcaagggcagggacgggccacaggccaagggcaagctttattgcggtagtttatcacagttaaattgctaacgcagtcagtgcttctgacacaacagtctcgaacttaagctgcagaagttggtcgtgaggcactgggcaggtaagtatcaaggttacaagacaggtttaaggagaccaatagaaactgggcttgtcgagacagagaagactcttgcgtttctgataggcacctattggtcttactgacatccactttgcctttctctccacaggtgtccactcccagttcaattacagctcttaaggctagagtacttaatacgactcactataggctagccaccatggcaccgaagaagaagcgcaaggtgcatatgaatacaaaatataataaagagttcttactctacttagcagggtttgtagacggtgacggttccatctatgcccgtatctttaagggtcaacattggaagttcaagcactatattcgtttgaccttctgtgtgcggcagaagacacagcgccgttggttcctcgacaagctggtggacgagatcggtgtgggttacgtgactgactctggcagcgtttccgcttactatctgtccgagatcaagcctttgcataattttttaacacaactacaaccttttctaaaactaaaacaaaaacaagcaaatttagttttaaaaattattgaacaacttccgtcagcaaaagaatccccggacaaattcttagaagtttgtacatgggtggatcaaattgcagctctgaatgattcgaagacgcgtaaaacaacttctgaaaccgttcgtgctgtgctagacagtttaccaggatccgtgggaggtctatcgccatctcaggcatccagcgccgcatcctcggcttcctcaagcccgggttcagggatctccgaagcactcagagctggagcaggttccggcactggatacaacaaggaattcctgctctacctggcgggcttcgtcgacggggacggctccatctgggcctcgatcattcctgagcaaggttataagttcaagcacaggctgcgtctctctttcactgtcgctcagaagacacagcgccgttggttcctcgacaagctggtggacgagatcggtgtgggttacgtggttgaccagggcagcgtctccgagtacaggctgtccgagatcaagcctctgcacaacttcctgacccagctccagcccttcctgaagctcaagcagaagcaggccaacctcgtgctgaagatcatcgagcagctgccctccgccaaggaatccccggacaagttcctggaggtgtgcacctgggtggaccagatcgccgctctgaacgactccaagacccgcaagaccacttccgaaaccgtccgcgccgttctagacagtctctccgagaagaagaagtcgtccccctaagcggccgcgactctagatcataatcagccataccacatttgtagaggttttacttgctttaaaaaacctcccacacctccccctgaacctgaaacataaaatgaatgcaattgttgttgttaacttgtttattgcagcttataatggttacaaataaagcaatagcatcacaaatttcacaaataaagcatttttttcactgcattctagttgtggtttgtccaaactcatcaatgtatcttaaggcgggaattgatctaggaacccctagtgatggagttggccactccctctctgcgcgctcgctcgctcactgaggccgcccgggcaaagcccgggcgtcgggcgacctttggtcgcccggcctcagtgagcgagcgagcgcgcagagagggagtggccaaccccccccccccccccccggcgattctcttgtttgctccagactctcaggcaatgacctgatagcctttgtagagacctctcaaaaatagctaccctctccggcatgaatttatcagctagaacggttgaatatcatattgatggtgatttgactgtctccggcctttctcacccgtttgaatctttacctacacattactcaggcattgcatttaaaatatatgagggttctaaaaatttttatccttgcgttgaaataaaggcttctcccgcaaaagtattacagggtcataatgtttttggtacaaccgatttagctttatgctctgaggctttattgcttaattttgctaattctttgccttgcctgtatgatttattggatgttggaattcctgatgcggtattttctccttacgcatctgtgcggtatttcacaccgcatatggtgcactctcagtacaatctgctctgatgccgcatagttaagccagccccgacacccgccaacacccgctgacgcgccctgacgggcttgtctgctcccggcatccgcttacagacaagctgtgaccgtctccgggagctgcatgtgtcagaggttttcaccgtcatcaccgaaacgcgcgagacgaaagggcctcgtgatacgcctatttttataggttaatgtcatgataataatggtttcttagacgtcaggtggcacttttcggggaaatgtgcgcggaacccctatttgtttatttttctaaatacattcaaatatgtatccgctcatgagacaataaccctgataaatgcttcaataatattgaaaaaggaagagtatgagtattcaacatttccgtgtcgcccttattcccttttttgcggcattttgccttcctgtttttgctcacccagaaacgctggtgaaagtaaaagatgctgaagatcagttgggtgcacgagtgggttacatcgaactggatctcaacagcggtaagatccttgagagttttcgccccgaagaacgttttccaatgatgagcacttttaaagttctgctatgtggcgcggtattatcccgtattgacgccgggcaagagcaactcggtcgccgcatacactattctcagaatgacttggttgagtactcaccagtcacagaaaagcatcttacggatggcatgacagtaagagaattatgcagtgctgccataaccatgagtgataacactgcggccaacttacttctgacaacgatcggaggaccgaaggagctaaccgcttttttgcacaacatgggggatcatgtaactcgccttgatcgttgggaaccggagctgaatgaagccataccaaacgacgagcgtgacaccacgatgcctgtagcaatggcaacaacgttgcgcaaactattaactggcgaactacttactctagcttcccggcaacaattaatagactggatggaggcggataaagttgcaggaccacttctgcgctcggcccttccggctggctggtttattgctgataaatctggagccggtgagcgtgggtctcgcggtatcattgcagcactggggccagatggtaagccctcccgtatcgtagttatctacacgacggggagtcaggcaactatggatgaacgaaatagacagatcgctgagataggtgcctcactgattaagcattggtaactgtcagaccaagtttactcatatatactttagattgatttaaaacttcatttttaatttaaaaggatctaggtgaagatcctttttgataatctcatgaccaaaatcccttaacgtgagttttcgttccactgagcgtcagaccccgtagaaaagatcaaaggatcttcttgagatcctttttttctgcgcgtaatctgctgcttgcaaacaaaaaaaccaccgctaccagcggtggtttgtttgccggatcaagagctaccaactctttttccgaaggtaactggcttcagcagagcgcagataccaaatactgtccttctagtgtagccgtagttaggccaccacttcaagaactctgtagcaccgcctacatacctcgctctgctaatcctgttaccagtggctgctgccagtggcgataagtcgtgtcttaccgggttggactcaagacgatagttaccggataaggcgcagcggtcgggctgaacggggggttcgtgcacacagcccagcttggagcgaacgacctacaccgaactgagatacctacagcgtgagctatgagaaagcgccacgcttcccgaagggagaaaggcggacaggtatccggtaagcggcagggtcggaacaggagagcgcacgagggagcttccagggggaaacgcctggtatctttatagtcctgtcgggtttcgccacctctgacttgagcgtcgatttttgtgatgctcgtcaggggggcggagcctatggaaaaacgccagcaacgcggcctttttacggttcctggccttttgctggccttttgctcacatgttctttcctgcgttatcccctgattctgtggataaccgtattaccgcctttgagtgagctgataccgctcgccgcagccgaacgaccgagcgcagcgagtcagtgagcgaggaagcggaagagcgcccaatacgcaaaccgcctctccccgcgcgttggccgattcattaatg